European Patent Application EP 4 137 506 A1, published February 22, 2023. Title: VACCINE COMPOSITION FOR AFRICAN SWINE FEVER. Applicant: Plumbline Life Sciences, Inc. The sequence listing filed with the application follows.

SEQUENCE LISTING (54 sequences)

SEQ ID NO: 1 - protein, 193 aa, Artificial Sequence
  ASFV p30
DFILNISMKMEVIFKTDLRSSSQVVFHAGSLYNWFSVEIINSGRIVTTAIKTLLSTVKYDIVKSARIYAGQGYTEHQAQEEWNMILHVLFEEETESSASSESIHEKNDNETNECTSSFETLFEQEPSSETPKDSKLYMLAQKTVQHIEQYGKAPDFNKVIRAHNFIQTIHGTPLKEEEKEVVRLMVIKLLKKK

SEQ ID NO: 2 - protein, 184 aa, Artificial Sequence
  ASFV P54_EP183L
DSEFFQPVYPRHYGECLSPVTTPSFFSTHMYTILIAIVVLVIIIIVLIYLFSSRKKKAAAAIEEEDIQFINPYQDQQWAEVTPQPGTSKPAGATTASVGKPVTGRPATNRPATNKPVTDNPVTDRLVMATGGPAAAPAAASAPAHPAEPYTTVTTQNTASQTMSAIENLRQRNTYTHKDLENSL

SEQ ID NO: 3 - protein, 157 aa, Artificial Sequence
  ASFV EP153R
FSKKKYIGLIDKKCELKKILDDYSILIIGILIGTNIITLIYNFIGWINYIKCYQNDDKMFYCPKDWVGYNNVCYYFSNEEKNYTNASNYCKQLNSTLANNNTNLVNLTKTLNLTKTYNHESNYWVNYSLIKNESVLLRNSGYYKKQKHVSLLYICSK

SEQ ID NO: 4 - protein, 364 aa, Artificial Sequence
  ASFV CD2v_EP402R
IILIFLIFSNIVLSIIYWVSFNKTIILDSNITNDNNDINGVSWNTYFNNSFNTLATCGKAGNFCECSNYSTSLYNITNNCSLTIFPHNTDIFNTTYQLVYLNQKINYTIKLLTPVDSPNITYNCTNSLITCKKNNGTNTNIYLNINDTIVNYTNESILNYYWNNSNINNFTATCIINNTISSSNETELINCTNPTLKYQNYFYTFFKLFYIIIFIVSGIIISILFISIITFLSLRKRKKHVEEIESPPPSESNEEEQCQHDDTTSIHEPSPREPLLPKPYSRYQYNTPIYYMRPSTQPLNPFPLPKPCPPPKPCPPPKPCPPPKPCPSAESYSPPKPLPSIPLLPNIPPLSTQNISLIHVDRII

SEQ ID NO: 5 - protein, 437 aa, Artificial Sequence
  ASFV p49_B438L
YHDYASKLLADYRSDPPLWESDLPRHNRYSDNILNSRYCGNKNGAAPVYNEYTNSPEKAEKGLQLSDLRNFSFMLNPQHKNIGYGDAQDLEPYSSIPKNKLFNHFKNHRPAFSTHTENLIRRNVVRTEKKTFPQVASLKGTQKNCLTQPSSLPSLKNPKNSSVPSTRFSEHTKFFSYEDLPKLRTKGTIKHEQHLGDQMPGQHYNGYIPHKDVYNILCLAHNLPASVEKGIAGRGIPLGNPHVKPNIEQELIKSTSTYTDVPMLGPLPPKDSQHGREYQEFSANRHMLQVSNILHSVFANHSIKPQILEDIPVLNAQLTSIKPVSPFLNKAYQTHYMENIVTLVPRFKSIANYSSPIPNYSKRNSGQAEYFDTSKQTISRHNNYIPKYTGGIGDSKLDSTFPKDFNASSVPLTSAEKDHSLRGDNSACCISSISPSL

SEQ ID NO: 6 - protein, 529 aa, Artificial Sequence
  ASFV pp62_CP530R
PSNMKQFCKISVWLQQHDPDLLEIINNLCMLGNLSAAKYKHGVTFIYPKQAKIRDEIKKHAYSNDPSQAIKTLESLILPFYIPTPAEFTGEIGSYTGVKLEVEKTEANKVILKNGEAVLVPAADFKPFPDRRLAVWIMESGSMPLEGPPYKRKKEGGGNDPPVPKHISPYTPRTRIAIEVEKAFDDCMRQNWCSVNNPYLAKSVSLLSFLSLNHPTEFIKVLPLIDFDPLVTFYLLLEPYKTHGDDFLIPETILFGPTGWNGTDLYQSAMLEFKKFFTQITRQTFMDIADSATKEVDVPICYSDPETVHSYANHVRTEILHHNAVNKVTTPNLVVQAYNELEQTNTIRHYGPIFPESTINALRFWKKLWQDEQRFVIHGLHRTLMDQPTYETSEFAEIVRNLRFSRPGNNYINELNITSPAMYGDKHTTGDIAPNDRFAMLVAFINSTDFLYTAIPEEKVGGNETQTSSLTDLVPTRLHSFLNHNLSKLKILNRAQQTVRNILSNDCLNQLKHYVKHTGKNEILKLLQE

SEQ ID NO: 7 - protein, 368 aa, Artificial Sequence
  ASFV EP364R
YFLVADHREHHVIPFLKTDFHHMHQNPIQKKQALLEIKQLFTGDYLICKSPSTILACIERKTYKDFAASLKDGRYKNRQKMLSLREQTNCQLYFFVEGPAFPNPQKKINHVAYASIITAMTHLMVRDHIFVIQTKNEAHSSQKLVQLFYAFSKEMVCVVPTSLTPTDEELCIKLWSSLSGISGVIGKILANTCSVAHLVSGKLSSQNIDQLKTPSNRPFPKKVKRMLISISKGNKELEIKLLSGVPNIGKKLAAEILKDHALLFFLNQPVECLANIQIVQKTRTIKLGMKRAEAIHYFLNWCGSAHVTDDSQNITEASRPTMQVATQSAATQPAATQPLHEVSDDASSDASSPVGHQTLSKEMLLNTA

SEQ ID NO: 8 - protein, 316 aa, Artificial Sequence
  ASFV F317L
VETQMDKLGFLLNHIGKQVTTKVLSNAHITQTMKEIILENHSVDGGAAKNVSKGKSSPKEKKHWTEFESWEQLSKSKRSFKEYWAERNEIVNTLLLNWDNVRGAIKKFLDDDREWCGRINMINGVPEIVEIIPSPYRAGENIYFGSEAMMPADIYSRVANKPAMFVFHTHPNLGSCCGGMPSICDISTTLRYLLMGWTAGHLIISSNQVGMLTVDKRIIVDLWANENPRWLMAQKILDIFMMLTSRRSLVNPWTLRDLKKILQDYGIEYIIFPSNDFFIYEDERLLMFSKKWTNFFTLHELLDDLETIETKASSTT

SEQ ID NO: 9 - protein, 103 aa, Artificial Sequence
  ASFV A104R
STKKKPTITKQELYSLVAADTQLNKALIERIFTSQQKIIQNALKHNQEVIIPPGIKFTVVTVKAKPARQGHNPATGEPIQIKAKPEHKAVKIRALKPVHDMLN

SEQ ID NO: 10 - protein, 204 aa, Artificial Sequence
  ASFV K205R
VEPREQFFQDLLSAVDQQMDTVKNDIKDIMKEKTSFMVSFENFIERYDTMEKNIQDLQNKYEEMAANLMTVMTDTKIQLGAIIAQLEILMINGTPLPAKKTTIKEAMPLPSSNTNNEQTSPPASGKTSETPKKNPTNAMFFTRSEWASSNTFREKFLTPEIQAILDEQFANKTGIERLHAEGLYMWRTQFSDEQKKMVKEMMKK

SEQ ID NO: 11 - DNA, 579 bp, Artificial Sequence
  ASFV p30_CP204L
gattttattttaaatatatccatgaaaatggaggtcatcttcaaaacggatttaagatcatcttcacaagttgtgtttcatgcgggtagcctgtataattggttttctgttgagattatcaatagcggtagaattgttacgaccgctataaaaacattgcttagtactgttaagtatgatattgtgaaatctgctcgtatatatgcagggcaagggtatactgaacatcaggctcaagaagaatggaatatgattctgcatgtgctgtttgaagaggagacggaatcctcagcatcttcggagtcaattcatgaaaaaaatgataatgaaaccaatgaatgcacatcctcctttgaaacgttgtttgagcaagagccctcatcggagacacctaaagactccaagctgtatatgcttgcacaaaagactgtgcaacatattgaacaatatggaaaggcacctgattttaacaaggttattagagcacataattttattcaaaccattcatggaacccctctaaaggaagaagaaaaagaggtggtaagactcatggttattaaacttttaaaaaaaaaa

SEQ ID NO: 12 - DNA, 552 bp, Artificial Sequence
  ASFV P54_EP183L
gattctgaattttttcaaccggtttatccgcggcattatggtgagtgtttgtcaccagtcactacaccaagcttcttctccacacatatgtatactattctcattgctatcgtggtcttagtcatcattatcatcgttctaatctatctattctcttcaagaaagaaaaaagctgctgctgctattgaggaggaagatatacagtttataaatccttatcaagatcagcagtgggcagaagtcactccacaaccaggtacctctaaaccagctggagcgactacagcaagtgtaggcaagccagtcacgggcagaccggcaacaaacagaccagcaacaaacaaaccagttacggacaacccagttacggacagactagtcatggcaactggcgggccggcggccgcacctgcggccgcgagtgctcctgctcatccggctgagccttacacgacagtcactactcagaacactgcttcacaaacaatgtcggctattgaaaatttacgacaaagaaacacctatacgcataaagacctagaaaactccttg

SEQ ID NO: 13 - DNA, 471 bp, Artificial Sequence
  ASFV C-type lectin_EP153R
ttttctaagaaaaagtacatcggtcttatcgataagaagtgtgaattgaaaaaaatactagatgattatagtatattaataattggaatattaattggaactaacatcataacccttatttataattttataggatggattaattatataaaatgttaccaaaatgatgataagatgttttattgccctaaagattgggttggatataataatgtttgttattattttagtaatgaagaaaaaaattatactaatgcaagtaattattgtaagcaattaaatagtacgcttgctaataataatactaatttagtaaatcttactaaaacattaaatcttactaaaacatataatcacgaatctaattattgggttaattattctttaattaaaaatgagtcagtactattacgtaatagtggatattacaaaaaacaaaaacatgtaagtttattatatatttgtagtaaa

SEQ ID NO: 14 - DNA, 1092 bp, Artificial Sequence
  ASFV CD2v_EP402R
ataatacttatttttttaatattttctaacatagttttaagtattatatattgggttagttttaataaaacaataattttagatagtaatattactaatgataataatgatataaatggagtatcatggaatacttattttaataattcttttaatacactagctacatgtggaaaagcaggtaacttttgtgaatgttctaattatagtacatcactatataatataacaaataattgtagcttaactatttttcctcataatactgatatatttaatacaacatatcaactagtatatctaaatcaaaaaattaattatacaataaaattattaacacctgtagattctccaaatatcacatataattgtactaattctttaataacatgtaaaaaaaataatggaacaaacactaatatatatttaaatataaatgatactatagttaattatactaatgaaagtatacttaattattattggaataatagtaacattaacaattttacagctacatgtataattaataatacaattagttcttctaatgaaacagaacttataaattgtactaatcccacattgaaatatcaaaactatttttatactttttttaaattattttatattataatatttatcgtatctgggataataataagtattctttttatatccatcataacttttttatctttacgaaaaagaaaaaaacatgttgaagaaatagaaagtccaccaccttctgaatctaatgaagaagaacaatgtcagcatgatgacaccacttccatacatgaaccatctcccagagaaccattacttcctaagccttacagtcgttatcagtataatacacctatttactacatgcgtccctcaacacaaccactcaacccatttcccttacctaaaccgtgtcctccacccaaaccatgtccgccacccaaaccatgtcctccacctaaaccatgtccttcagctgaatcctattctccacccaaaccactacctagtatcccgctactacccaatatcccgccattatctacccaaaatatttcgcttattcacgtagatagaattatt

SEQ ID NO: 15 - DNA, 1311 bp, Artificial Sequence
  ASFV p49_B438L
tatcatgattatgcttcaaagctgttagccgattataggtcagatccacctctttgggaaagcgatttgccgcgtcataaccggtattctgataatatactaaattcccggtactgcggcaacaaaaatggagctgcgcctgtatacaatgaatacactaatagtcctgaaaaggctgaaaagggattgcaactcagtgatctacgtaacttttcttttatgctgaaccctcagcacaaaaacattggttacggcgatgcgcaagatctggagccgtacagctccattccaaaaaataaactttttaatcattttaaaaatcatcgtcctgctttttcaacccatacggaaaacctaattaggcgcaatgttgttcgtacggaaaaaaaaacatttccgcaggtggctagcttaaagggcacacagaaaaattgtctgacccagccttcctcattgccttccttaaaaaacccaaaaaatagttcggttccttctacgaggttcagcgagcacacaaaatttttttcgtacgaggatcttcctaaactcagaacaaagggtaccattaagcatgagcagcaccttggcgatcagatgccgggccagcactataacggatatattccgcacaaagacgtgtacaatattttgtgtttagcgcacaatctacctgcgtcggtagaaaaagggattgcaggtagaggtattcctttaggaaatccacatgtcaaaccgaacatagagcaggaactcataaaatccaccagtacctacacggacgtgccgatgcttggtccccttccgcccaaagattcgcaacacggcagagaataccaggaattttccgcaaatagacatatgctacaagtatctaatatactacattctgtgtttgctaatcattctataaagccacaaatcctagaagacataccggtactcaatgcacaactaacaagcataaagccggtaagcccatttttaaacaaagcgtatcaaacccattatatggaaaatattgttaccttggtgccccggtttaagagtattgccaactactcaagccctataccgaattattctaaaagaaatagcggtcaggctgaatattttgatacctcaaagcaaacaatttctagacacaataattatatacctaaatatacgggaggaattggagattccaaactagacagcacctttcctaaagatttcaacgcctcctcggtaccgttaacaagcgcggaaaaggaccattccctgcggggagacaactcagcatgttgcatctcatctatatctccatcattg

SEQ ID NO: 16 - DNA, 1587 bp, Artificial Sequence
  ASFV pp62_CP530R
ccctctaatatgaaacagttttgcaagatttctgtatggctacagcagcacgatccagatttattagaaattatcaacaacttatgtatgcttggcaatttatccgcggcaaagtacaaacacggagttaccttcatttaccccaaacaggcaaagatccgcgatgaaataaaaaaacatgcctactccaatgacccttcacaagccataaagaccttagaatcactcatccttccattttacattcccactccagcggagttcaccggggaaatcggctcctacaccggagtgaaattagaggttgaaaaaacggaggcgaataaagttattttaaaaaatggagaagcggtcctagtaccggcggccgattttaagccctttcctgatcgccgactagcggtctggatcatggagtcaggctctatgcccctggagggtcccccctataagcggaaaaaggagggtggggggaatgacccgccggttcctaagcatatctcgccgtatactccgcgcacgcgtattgccattgaggtggaaaaggcctttgatgactgtatgcgtcaaaactggtgtagtgtcaataatccctatcttgccaagtcggtctccttgctgtctttcttgtcgctcaaccatcccaccgagtttattaaggtactgccgcttatagactttgaccccttggtgaccttttatctacttcttgagccctataaaacgcatggggatgactttttaattccggaaaccattttattcggccctaccggatggaatggtacagatctgtatcaaagtgccatgctggagtttaaaaagttttttacccagattactcgccaaacctttatggacatagccgattcggctactaaggaggtagatgttcccatatgttactcggatcccgaaaccgtacattcctatgccaatcacgtgcgtactgaaattttgcatcacaatgccgtcaataaggttacaacacctaacctcgtcgtgcaggcctataatgagctcgagcaaaccaataccatacgacattacggccctattttcccggaaagtaccatcaacgcactgcgtttttggaaaaagctgtggcaggatgaacagcgatttgttatccacggcctgcaccgcacgttgatggatcaacccacctatgaaacctctgagtttgcagagatcgttagaaatttacggttttcgcgtcccggcaataactatataaacgagcttaatattacaagtcccgctatgtacggcgacaagcataccaccggagatattgcgcccaatgatagatttgccatgttggtggcctttatcaacagtactgactttttatacaccgcgattcccgaggaaaaggtaggggggaatgaaacccaaaccagtagccttacagacctagttccaacacggctacactcttttttaaatcataatctaagcaaacttaaaatcttaaaccgcgcgcagcaaacggttagaaatattctttcaaatgattgtcttaatcaactgaaacattatgttaaacacacgggaaaaaatgaaatactaaagttacttcaagaa

SEQ ID NO: 17 - DNA, 1104 bp, Artificial Sequence
  ASFV EP364R
tattttctagtagcagatcatcgagaacatcatgtgattccttttcttaaaaccgatttccatcacatgcatcaaaatcctatacaaaaaaaacaagctctcctagaaatcaaacagctttttactggagattatctcatctgcaaaagcccttctaccattctggcctgtattgaacgaaaaacctacaaagactttgcggcttctttgaaagatggacgttataaaaatcgccaaaaaatgctgtcgctgcgagaacaaaccaactgtcaactttatttttttgtagaaggcccggcatttcctaaccctcaaaaaaaaattaatcacgttgcctatgcaagcattattactgctatgacgcatcttatggttagagatcatatttttgtcattcaaacgaaaaatgaggcccacagttcccaaaagcttgtgcagcttttttatgccttttctaaggaaatggtgtgcgtcgttcccacctccctcacccccacggatgaagagctatgcatcaagctatggtcttctctttctggtatttcaggcgtgataggtaaaatcttggcaaacacttgttccgtagctcatttggtttctggaaagctttcatcgcagaatattgatcagttaaaaactccctccaaccgaccattccccaaaaaagtaaaacgtatgcttataagcattagcaaaggaaataaggagttagaaataaaattgctctcgggggttcccaatatcgggaaaaaattagctgccgaaattttaaaagatcatgcgcttcttttttttctaaatcagcccgtagaatgcttggcaaatatacaaatcgttcaaaaaacccgtacgattaagttgggaatgaagcgagccgaagcgattcattattttttaaactggtgtggctctgcccatgtaaccgatgatagccaaaatatcacagaggcgtcgcggcctacaatgcaggtcgcgacgcagtccgccgcaactcagcccgctgcaacgcagccattgcacgaagtatcagatgatgcatcatcagatgcttcatcacccgtagggcatcaaacattatctaaagaaatgttattgaacacagcc

SEQ ID NO: 18 - DNA, 948 bp, Artificial Sequence
  ASFV F317L
gttgagacacaaatggacaaacttggttttctgctaaatcacataggtaaacaggttaccactaaggtgcttagcaatgcccatataactcaaacgatgaaggagattattttggaaaatcatagtgtagatggtggagccgcaaaaaatgtttcaaaagggaagtcttccccaaaagaaaaaaaacattggactgagttcgaatcctgggaacagctcagcaagtctaaaagaagttttaaggaatactgggcggagcgtaatgagattgtgaatactctgttgcttaactgggacaatgttcggggtgccatcaaaaaatttttggacgatgaccgtgaatggtgcggccgcattaatatgataaacggtgtacccgagatagtggaaatcattccaagcccctatagggcaggagagaacatttattttggcagcgaggctatgatgcctgctgatatttatagcagggtggccaacaagcctgctatgtttgtgtttcacacgcatcctaatttgggttcatgttgtggaggaatgccttccatatgtgacatttctacaacgctgcgttatctactcatggggtggactgctgggcatctaatcatttcttcgaatcaagtaggaatgctcacggttgataagagaattattgttgatttgtgggccaatgagaatccgcgctggcttatggcgcaaaaaatattagatatttttatgatgctcacttcgcgtagaagcctggtaaatccctggaccctgagagacctaaaaaaaatattacaagactatggtattgagtatatcatttttccttcgaatgacttttttatttatgaagacgaacgtcttttaatgttttcaaaaaaatggaccaacttttttacgttacatgagttattggatgacctcgaaactattgagacaaaggcatcgtccacaaca

SEQ ID NO: 19 - DNA, 309 bp, Artificial Sequence
  ASFV A104R
tcgacaaaaaaaaagcccacaattaccaagcaagagctttactccttagtagcggcagatacccagttaaataaagcattgattgaaagaatctttacaagtcagcaaaaaataatacaaaatgctttaaagcacaatcaagaagttattataccacccggaatcaagttcaccgtcgttacggtgaaagctaaacctgctcgccagggccataatcccgccacaggagagcctattcaaattaaagctaaacctgaacataaagccgtaaagatacgagcattgaaacctgtccatgatatgttaaac

SEQ ID NO: 20 - DNA, 612 bp, Artificial Sequence
  ASFV K205R
gttgagccacgcgaacagttttttcaagatctgctttcagcagtggatcaacaaatggacactgtaaaaaatgacataaaagacattatgaaagaaaaaacgtcttttatggtatcattcgaaaactttatagaacgttacgataccatggaaaaaaatattcaagaccttcagaataagtacgaagaaatggcggccaaccttatgaccgtcatgacggatacaaaaattcagcttggagccattatcgcccaacttgagattctaatgataaatggcactccacttccggcaaaaaagacaacaattaaggaggctatgcccttaccttcatcaaacacgaataatgaacaaacgagtcctcccgcctcaggcaaaacaagtgaaacacctaaaaaaaatcccacgaatgcgatgttcttcacgcgtagcgaatgggcatcctcgaatacttttcgagaaaagtttttaacaccagaaattcaagccatattggatgagcagtttgcaaacaagaccgggatcgaaagattgcatgccgagggtctttacatgtggagaacccaattctctgacgaacagaagaaaatggtcaaagagatgatgaagaag

SEQ ID NO: 21 - protein, 2855 aa, Artificial Sequence
  PLS-ASF fusion protein no. 1
DFILNISMKMEVIFKTDLRSSSQVVFHAGSLYNWFSVEIINSGRIVTTAIKTLLSTVKYDIVKSARIYAGQGYTEHQAQEEWNMILHVLFEEETESSASSESIHEKNDNETNECTSSFETLFEQEPSSETPKDSKLYMLAQKTVQHIEQYGKAPDFNKVIRAHNFIQTIHGTPLKEEEKEVVRLMVIKLLKKKDSEFFQPVYPRHYGECLSPVTTPSFFSTHMYTILIAIVVLVIIIIVLIYLFSSRKKKAAAAIEEEDIQFINPYQDQQWAEVTPQPGTSKPAGATTASVGKPVTGRPATNRPATNKPVTDNPVTDRLVMATGGPAAAPAAASAPAHPAEPYTTVTTQNTASQTMSAIENLRQRNTYTHKDLENSLFSKKKYIGLIDKKCELKKILDDYSILIIGILIGTNIITLIYNFIGWINYIKCYQNDDKMFYCPKDWVGYNNVCYYFSNEEKNYTNASNYCKQLNSTLANNNTNLVNLTKTLNLTKTYNHESNYWVNYSLIKNESVLLRNSGYYKKQKHVSLLYICSKIILIFLIFSNIVLSIIYWVSFNKTIILDSNITNDNNDINGVSWNTYFNNSFNTLATCGKAGNFCECSNYSTSLYNITNNCSLTIFPHNTDIFNTTYQLVYLNQKINYTIKLLTPVDSPNITYNCTNSLITCKKNNGTNTNIYLNINDTIVNYTNESILNYYWNNSNINNFTATCIINNTISSSNETELINCTNPTLKYQNYFYTFFKLFYIIIFIVSGIIISILFISIITFLSLRKRKKHVEEIESPPPSESNEEEQCQHDDTTSIHEPSPREPLLPKPYSRYQYNTPIYYMRPSTQPLNPFPLPKPCPPPKPCPPPKPCPPPKPCPSAESYSPPKPLPSIPLLPNIPPLSTQNISLIHVDRIIYHDYASKLLADYRSDPPLWESDLPRHNRYSDNILNSRYCGNKNGAAPVYNEYTNSPEKAEKGLQLSDLRNFSFMLNPQHKNIGYGDAQDLEPYSSIPKNKLFNHFKNHRPAFSTHTENLIRRNVVRTEKKTFPQVASLKGTQKNCLTQPSSLPSLKNPKNSSVPSTRFSEHTKFFSYEDLPKLRTKGTIKHEQHLGDQMPGQHYNGYIPHKDVYNILCLAHNLPASVEKGIAGRGIPLGNPHVKPNIEQELIKSTSTYTDVPMLGPLPPKDSQHGREYQEFSANRHMLQVSNILHSVFANHSIKPQILEDIPVLNAQLTSIKPVSPFLNKAYQTHYMENIVTLVPRFKSIANYSSPIPNYSKRNSGQAEYFDTSKQTISRHNNYIPKYTGGIGDSKLDSTFPKDFNASSVPLTSAEKDHSLRGDNSACCISSISPSLPSNMKQFCKISVWLQQHDPDLLEIINNLCMLGNLSAAKYKHGVTFIYPKQAKIRDEIKKHAYSNDPSQAIKTLESLILPFYIPTPAEFTGEIGSYTGVKLEVEKTEANKVILKNGEAVLVPAADFKPFPDRRLAVWIMESGSMPLEGPPYKRKKEGGGNDPPVPKHISPYTPRTRIAIEVEKAFDDCMRQNWCSVNNPYLAKSVSLLSFLSLNHPTEFIKVLPLIDFDPLVTFYLLLEPYKTHGDDFLIPETILFGPTGWNGTDLYQSAMLEFKKFFTQITRQTFMDIADSATKEVDVPICYSDPETVHSYANHVRTEILHHNAVNKVTTPNLVVQAYNELEQTNTIRHYGPIFPESTINALRFWKKLWQDEQRFVIHGLHRTLMDQPTYETSEFAEIVRNLRFSRPGNNYINELNITSPAMYGDKHTTGDIAPNDRFAMLVAFINSTDFLYTAIPEEKVGGNETQTSSLTDLVPTRLHSFLNHNLSKLKILNRAQQTVRNILSNDCLNQLKHYVKHTGKNEILKLLQEYFLVADHREHHVIPFLKTDFHHMHQNPIQKKQALLEIKQLFTGDYLICKSPSTILACIERKTYKDFAASLKDGRYKNRQKMLSLREQTNCQLYFFVEGPAFPNPQKKINHVAYASIITAMTHLMVRDHIFVIQTKNEAHSSQKLVQLFYAFSKEMVCVVPTSLTPTDEELCIKLWSSLSGISGVIGKILANTCSVAHLVSGKLSSQNIDQLKTPSNRPFPKKVKRMLISISKGNKELEIKLLSGVPNIGKKLAAEILKDHALLFFLNQPVECLANIQIVQKTRTIKLGMKRAEAIHYFLNWCGSAHVTDDSQNITEASRPTMQVATQSAATQPAATQPLHEVSDDASSDASSPVGHQTLSKEMLLNTAVETQMDKLGFLLNHIGKQVTTKVLSNAHITQTMKEIILENHSVDGGAAKNVSKGKSSPKEKKHWTEFESWEQLSKSKRSFKEYWAERNEIVNTLLLNWDNVRGAIKKFLDDDREWCGRINMINGVPEIVEIIPSPYRAGENIYFGSEAMMPADIYSRVANKPAMFVFHTHPNLGSCCGGMPSICDISTTLRYLLMGWTAGHLIISSNQVGMLTVDKRIIVDLWANENPRWLMAQKILDIFMMLTSRRSLVNPWTLRDLKKILQDYGIEYIIFPSNDFFIYEDERLLMFSKKWTNFFTLHELLDDLETIETKASSTTSTKKKPTITKQELYSLVAADTQLNKALIERIFTSQQKIIQNALKHNQEVIIPPGIKFTVVTVKAKPARQGHNPATGEPIQIKAKPEHKAVKIRALKPVHDMLNVEPREQFFQDLLSAVDQQMDTVKNDIKDIMKEKTSFMVSFENFIERYDTMEKNIQDLQNKYEEMAANLMTVMTDTKIQLGAIIAQLEILMINGTPLPAKKTTIKEAMPLPSSNTNNEQTSPPASGKTSETPKKNPTNAMFFTRSEWASSNTFREKFLTPEIQAILDEQFANKTGIERLHAEGLYMWRTQFSDEQKKMVKEMMKK

SEQ ID NO: 22 - protein, 898 aa, Artificial Sequence
  PLS-ASF fusion protein no. 2
DFILNISMKMEVIFKTDLRSSSQVVFHAGSLYNWFSVEIINSGRIVTTAIKTLLSTVKYDIVKSARIYAGQGYTEHQAQEEWNMILHVLFEEETESSASSESIHEKNDNETNECTSSFETLFEQEPSSETPKDSKLYMLAQKTVQHIEQYGKAPDFNKVIRAHNFIQTIHGTPLKEEEKEVVRLMVIKLLKKKDSEFFQPVYPRHYGECLSPVTTPSFFSTHMYTILIAIVVLVIIIIVLIYLFSSRKKKAAAAIEEEDIQFINPYQDQQWAEVTPQPGTSKPAGATTASVGKPVTGRPATNRPATNKPVTDNPVTDRLVMATGGPAAAPAAASAPAHPAEPYTTVTTQNTASQTMSAIENLRQRNTYTHKDLENSLFSKKKYIGLIDKKCELKKILDDYSILIIGILIGTNIITLIYNFIGWINYIKCYQNDDKMFYCPKDWVGYNNVCYYFSNEEKNYTNASNYCKQLNSTLANNNTNLVNLTKTLNLTKTYNHESNYWVNYSLIKNESVLLRNSGYYKKQKHVSLLYICSKIILIFLIFSNIVLSIIYWVSFNKTIILDSNITNDNNDINGVSWNTYFNNSFNTLATCGKAGNFCECSNYSTSLYNITNNCSLTIFPHNTDIFNTTYQLVYLNQKINYTIKLLTPVDSPNITYNCTNSLITCKKNNGTNTNIYLNINDTIVNYTNESILNYYWNNSNINNFTATCIINNTISSSNETELINCTNPTLKYQNYFYTFFKLFYIIIFIVSGIIISILFISIITFLSLRKRKKHVEEIESPPPSESNEEEQCQHDDTTSIHEPSPREPLLPKPYSRYQYNTPIYYMRPSTQPLNPFPLPKPCPPPKPCPPPKPCPPPKPCPSAESYSPPKPLPSIPLLPNIPPLSTQNISLIHVDRII

SEQ ID NO: 23 - protein, 1957 aa, Artificial Sequence
  PLS-ASF fusion protein no. 3
YHDYASKLLADYRSDPPLWESDLPRHNRYSDNILNSRYCGNKNGAAPVYNEYTNSPEKAEKGLQLSDLRNFSFMLNPQHKNIGYGDAQDLEPYSSIPKNKLFNHFKNHRPAFSTHTENLIRRNVVRTEKKTFPQVASLKGTQKNCLTQPSSLPSLKNPKNSSVPSTRFSEHTKFFSYEDLPKLRTKGTIKHEQHLGDQMPGQHYNGYIPHKDVYNILCLAHNLPASVEKGIAGRGIPLGNPHVKPNIEQELIKSTSTYTDVPMLGPLPPKDSQHGREYQEFSANRHMLQVSNILHSVFANHSIKPQILEDIPVLNAQLTSIKPVSPFLNKAYQTHYMENIVTLVPRFKSIANYSSPIPNYSKRNSGQAEYFDTSKQTISRHNNYIPKYTGGIGDSKLDSTFPKDFNASSVPLTSAEKDHSLRGDNSACCISSISPSLPSNMKQFCKISVWLQQHDPDLLEIINNLCMLGNLSAAKYKHGVTFIYPKQAKIRDEIKKHAYSNDPSQAIKTLESLILPFYIPTPAEFTGEIGSYTGVKLEVEKTEANKVILKNGEAVLVPAADFKPFPDRRLAVWIMESGSMPLEGPPYKRKKEGGGNDPPVPKHISPYTPRTRIAIEVEKAFDDCMRQNWCSVNNPYLAKSVSLLSFLSLNHPTEFIKVLPLIDFDPLVTFYLLLEPYKTHGDDFLIPETILFGPTGWNGTDLYQSAMLEFKKFFTQITRQTFMDIADSATKEVDVPICYSDPETVHSYANHVRTEILHHNAVNKVTTPNLVVQAYNELEQTNTIRHYGPIFPESTINALRFWKKLWQDEQRFVIHGLHRTLMDQPTYETSEFAEIVRNLRFSRPGNNYINELNITSPAMYGDKHTTGDIAPNDRFAMLVAFINSTDFLYTAIPEEKVGGNETQTSSLTDLVPTRLHSFLNHNLSKLKILNRAQQTVRNILSNDCLNQLKHYVKHTGKNEILKLLQEYFLVADHREHHVIPFLKTDFHHMHQNPIQKKQALLEIKQLFTGDYLICKSPSTILACIERKTYKDFAASLKDGRYKNRQKMLSLREQTNCQLYFFVEGPAFPNPQKKINHVAYASIITAMTHLMVRDHIFVIQTKNEAHSSQKLVQLFYAFSKEMVCVVPTSLTPTDEELCIKLWSSLSGISGVIGKILANTCSVAHLVSGKLSSQNIDQLKTPSNRPFPKKVKRMLISISKGNKELEIKLLSGVPNIGKKLAAEILKDHALLFFLNQPVECLANIQIVQKTRTIKLGMKRAEAIHYFLNWCGSAHVTDDSQNITEASRPTMQVATQSAATQPAATQPLHEVSDDASSDASSPVGHQTLSKEMLLNTAVETQMDKLGFLLNHIGKQVTTKVLSNAHITQTMKEIILENHSVDGGAAKNVSKGKSSPKEKKHWTEFESWEQLSKSKRSFKEYWAERNEIVNTLLLNWDNVRGAIKKFLDDDREWCGRINMINGVPEIVEIIPSPYRAGENIYFGSEAMMPADIYSRVANKPAMFVFHTHPNLGSCCGGMPSICDISTTLRYLLMGWTAGHLIISSNQVGMLTVDKRIIVDLWANENPRWLMAQKILDIFMMLTSRRSLVNPWTLRDLKKILQDYGIEYIIFPSNDFFIYEDERLLMFSKKWTNFFTLHELLDDLETIETKASSTTSTKKKPTITKQELYSLVAADTQLNKALIERIFTSQQKIIQNALKHNQEVIIPPGIKFTVVTVKAKPARQGHNPATGEPIQIKAKPEHKAVKIRALKPVHDMLNVEPREQFFQDLLSAVDQQMDTVKNDIKDIMKEKTSFMVSFENFIERYDTMEKNIQDLQNKYEEMAANLMTVMTDTKIQLGAIIAQLEILMINGTPLPAKKTTIKEAMPLPSSNTNNEQTSPPASGKTSETPKKNPTNAMFFTRSEWASSNTFREKFLTPEIQAILDEQFANKTGIERLHAEGLYMWRTQFSDEQKKMVKEMMKK

SEQ ID NO: 24 - protein, 1427 aa, Artificial Sequence
  PLS-ASF fusion protein no. 4
DFILNISMKMEVIFKTDLRSSSQVVFHAGSLYNWFSVEIINSGRIVTTAIKTLLSTVKYDIVKSARIYAGQGYTEHQAQEEWNMILHVLFEEETESSASSESIHEKNDNETNECTSSFETLFEQEPSSETPKDSKLYMLAQKTVQHIEQYGKAPDFNKVIRAHNFIQTIHGTPLKEEEKEVVRLMVIKLLKKKDSEFFQPVYPRHYGECLSPVTTPSFFSTHMYTILIAIVVLVIIIIVLIYLFSSRKKKAAAAIEEEDIQFINPYQDQQWAEVTPQPGTSKPAGATTASVGKPVTGRPATNRPATNKPVTDNPVTDRLVMATGGPAAAPAAASAPAHPAEPYTTVTTQNTASQTMSAIENLRQRNTYTHKDLENSLPSNMKQFCKISVWLQQHDPDLLEIINNLCMLGNLSAAKYKHGVTFIYPKQAKIRDEIKKHAYSNDPSQAIKTLESLILPFYIPTPAEFTGEIGSYTGVKLEVEKTEANKVILKNGEAVLVPAADFKPFPDRRLAVWIMESGSMPLEGPPYKRKKEGGGNDPPVPKHISPYTPRTRIAIEVEKAFDDCMRQNWCSVNNPYLAKSVSLLSFLSLNHPTEFIKVLPLIDFDPLVTFYLLLEPYKTHGDDFLIPETILFGPTGWNGTDLYQSAMLEFKKFFTQITRQTFMDIADSATKEVDVPICYSDPETVHSYANHVRTEILHHNAVNKVTTPNLVVQAYNELEQTNTIRHYGPIFPESTINALRFWKKLWQDEQRFVIHGLHRTLMDQPTYETSEFAEIVRNLRFSRPGNNYINELNITSPAMYGDKHTTGDIAPNDRFAMLVAFINSTDFLYTAIPEEKVGGNETQTSSLTDLVPTRLHSFLNHNLSKLKILNRAQQTVRNILSNDCLNQLKHYVKHTGKNEILKLLQEFSKKKYIGLIDKKCELKKILDDYSILIIGILIGTNIITLIYNFIGWINYIKCYQNDDKMFYCPKDWVGYNNVCYYFSNEEKNYTNASNYCKQLNSTLANNNTNLVNLTKTLNLTKTYNHESNYWVNYSLIKNESVLLRNSGYYKKQKHVSLLYICSKIILIFLIFSNIVLSIIYWVSFNKTIILDSNITNDNNDINGVSWNTYFNNSFNTLATCGKAGNFCECSNYSTSLYNITNNCSLTIFPHNTDIFNTTYQLVYLNQKINYTIKLLTPVDSPNITYNCTNSLITCKKNNGTNTNIYLNINDTIVNYTNESILNYYWNNSNINNFTATCIINNTISSSNETELINCTNPTLKYQNYFYTFFKLFYIIIFIVSGIIISILFISIITFLSLRKRKKHVEEIESPPPSESNEEEQCQHDDTTSIHEPSPREPLLPKPYSRYQYNTPIYYMRPSTQPLNPFPLPKPCPPPKPCPPPKPCPPPKPCPSAESYSPPKPLPSIPLLPNIPPLSTQNISLIHVDRII

SEQ ID NO: 25 - protein, 1428 aa, Artificial Sequence
  PLS-ASF fusion protein no. 5
YHDYASKLLADYRSDPPLWESDLPRHNRYSDNILNSRYCGNKNGAAPVYNEYTNSPEKAEKGLQLSDLRNFSFMLNPQHKNIGYGDAQDLEPYSSIPKNKLFNHFKNHRPAFSTHTENLIRRNVVRTEKKTFPQVASLKGTQKNCLTQPSSLPSLKNPKNSSVPSTRFSEHTKFFSYEDLPKLRTKGTIKHEQHLGDQMPGQHYNGYIPHKDVYNILCLAHNLPASVEKGIAGRGIPLGNPHVKPNIEQELIKSTSTYTDVPMLGPLPPKDSQHGREYQEFSANRHMLQVSNILHSVFANHSIKPQILEDIPVLNAQLTSIKPVSPFLNKAYQTHYMENIVTLVPRFKSIANYSSPIPNYSKRNSGQAEYFDTSKQTISRHNNYIPKYTGGIGDSKLDSTFPKDFNASSVPLTSAEKDHSLRGDNSACCISSISPSLYFLVADHREHHVIPFLKTDFHHMHQNPIQKKQALLEIKQLFTGDYLICKSPSTILACIERKTYKDFAASLKDGRYKNRQKMLSLREQTNCQLYFFVEGPAFPNPQKKINHVAYASIITAMTHLMVRDHIFVIQTKNEAHSSQKLVQLFYAFSKEMVCVVPTSLTPTDEELCIKLWSSLSGISGVIGKILANTCSVAHLVSGKLSSQNIDQLKTPSNRPFPKKVKRMLISISKGNKELEIKLLSGVPNIGKKLAAEILKDHALLFFLNQPVECLANIQIVQKTRTIKLGMKRAEAIHYFLNWCGSAHVTDDSQNITEASRPTMQVATQSAATQPAATQPLHEVSDDASSDASSPVGHQTLSKEMLLNTAVETQMDKLGFLLNHIGKQVTTKVLSNAHITQTMKEIILENHSVDGGAAKNVSKGKSSPKEKKHWTEFESWEQLSKSKRSFKEYWAERNEIVNTLLLNWDNVRGAIKKFLDDDREWCGRINMINGVPEIVEIIPSPYRAGENIYFGSEAMMPADIYSRVANKPAMFVFHTHPNLGSCCGGMPSICDISTTLRYLLMGWTAGHLIISSNQVGMLTVDKRIIVDLWANENPRWLMAQKILDIFMMLTSRRSLVNPWTLRDLKKILQDYGIEYIIFPSNDFFIYEDERLLMFSKKWTNFFTLHELLDDLETIETKASSTTSTKKKPTITKQELYSLVAADTQLNKALIERIFTSQQKIIQNALKHNQEVIIPPGIKFTVVTVKAKPARQGHNPATGEPIQIKAKPEHKAVKIRALKPVHDMLNVEPREQFFQDLLSAVDQQMDTVKNDIKDIMKEKTSFMVSFENFIERYDTMEKNIQDLQNKYEEMAANLMTVMTDTKIQLGAIIAQLEILMINGTPLPAKKTTIKEAMPLPSSNTNNEQTSPPASGKTSETPKKNPTNAMFFTRSEWASSNTFREKFLTPEIQAILDEQFANKTGIERLHAEGLYMWRTQFSDEQKKMVKEMMKK

SEQ ID NO: 26 - protein, 2930 aa, Artificial Sequence
  PLS-ASF fusion protein no. 1'
QIFVKTLTGKTITLEVEPSDTIENVKGKIQEKEGIPPDQQRLIFAGKQLEDGRTLSDYNIQKESTLHLVLRLRGADFILNISMKMEVIFKTDLRSSSQVVFHAGSLYNWFSVEIINSGRIVTTAIKTLLSTVKYDIVKSARIYAGQGYTEHQAQEEWNMILHVLFEEETESSASSESIHEKNDNETNECTSSFETLFEQEPSSETPKDSKLYMLAQKTVQHIEQYGKAPDFNKVIRAHNFIQTIHGTPLKEEEKEVVRLMVIKLLKKKDSEFFQPVYPRHYGECLSPVTTPSFFSTHMYTILIAIVVLVIIIIVLIYLFSSRKKKAAAAIEEEDIQFINPYQDQQWAEVTPQPGTSKPAGATTASVGKPVTGRPATNRPATNKPVTDNPVTDRLVMATGGPAAAPAAASAPAHPAEPYTTVTTQNTASQTMSAIENLRQRNTYTHKDLENSLFSKKKYIGLIDKKCELKKILDDYSILIIGILIGTNIITLIYNFIGWINYIKCYQNDDKMFYCPKDWVGYNNVCYYFSNEEKNYTNASNYCKQLNSTLANNNTNLVNLTKTLNLTKTYNHESNYWVNYSLIKNESVLLRNSGYYKKQKHVSLLYICSKIILIFLIFSNIVLSIIYWVSFNKTIILDSNITNDNNDINGVSWNTYFNNSFNTLATCGKAGNFCECSNYSTSLYNITNNCSLTIFPHNTDIFNTTYQLVYLNQKINYTIKLLTPVDSPNITYNCTNSLITCKKNNGTNTNIYLNINDTIVNYTNESILNYYWNNSNINNFTATCIINNTISSSNETELINCTNPTLKYQNYFYTFFKLFYIIIFIVSGIIISILFISIITFLSLRKRKKHVEEIESPPPSESNEEEQCQHDDTTSIHEPSPREPLLPKPYSRYQYNTPIYYMRPSTQPLNPFPLPKPCPPPKPCPPPKPCPPPKPCPSAESYSPPKPLPSIPLLPNIPPLSTQNISLIHVDRIIYHDYASKLLADYRSDPPLWESDLPRHNRYSDNILNSRYCGNKNGAAPVYNEYTNSPEKAEKGLQLSDLRNFSFMLNPQHKNIGYGDAQDLEPYSSIPKNKLFNHFKNHRPAFSTHTENLIRRNVVRTEKKTFPQVASLKGTQKNCLTQPSSLPSLKNPKNSSVPSTRFSEHTKFFSYEDLPKLRTKGTIKHEQHLGDQMPGQHYNGYIPHKDVYNILCLAHNLPASVEKGIAGRGIPLGNPHVKPNIEQELIKSTSTYTDVPMLGPLPPKDSQHGREYQEFSANRHMLQVSNILHSVFANHSIKPQILEDIPVLNAQLTSIKPVSPFLNKAYQTHYMENIVTLVPRFKSIANYSSPIPNYSKRNSGQAEYFDTSKQTISRHNNYIPKYTGGIGDSKLDSTFPKDFNASSVPLTSAEKDHSLRGDNSACCISSISPSLPSNMKQFCKISVWLQQHDPDLLEIINNLCMLGNLSAAKYKHGVTFIYPKQAKIRDEIKKHAYSNDPSQAIKTLESLILPFYIPTPAEFTGEIGSYTGVKLEVEKTEANKVILKNGEAVLVPAADFKPFPDRRLAVWIMESGSMPLEGPPYKRKKEGGGNDPPVPKHISPYTPRTRIAIEVEKAFDDCMRQNWCSVNNPYLAKSVSLLSFLSLNHPTEFIKVLPLIDFDPLVTFYLLLEPYKTHGDDFLIPETILFGPTGWNGTDLYQSAMLEFKKFFTQITRQTFMDIADSATKEVDVPICYSDPETVHSYANHVRTEILHHNAVNKVTTPNLVVQAYNELEQTNTIRHYGPIFPESTINALRFWKKLWQDEQRFVIHGLHRTLMDQPTYETSEFAEIVRNLRFSRPGNNYINELNITSPAMYGDKHTTGDIAPNDRFAMLVAFINSTDFLYTAIPEEKVGGNETQTSSLTDLVPTRLHSFLNHNLSKLKILNRAQQTVRNILSNDCLNQLKHYVKHTGKNEILKLLQEYFLVADHREHHVIPFLKTDFHHMHQNPIQKKQALLEIKQLFTGDYLICKSPSTILACIERKTYKDFAASLKDGRYKNRQKMLSLREQTNCQLYFFVEGPAFPNPQKKINHVAYASIITAMTHLMVRDHIFVIQTKNEAHSSQKLVQLFYAFSKEMVCVVPTSLTPTDEELCIKLWSSLSGISGVIGKILANTCSVAHLVSGKLSSQNIDQLKTPSNRPFPKKVKRMLISISKGNKELEIKLLSGVPNIGKKLAAEILKDHALLFFLNQPVECLANIQIVQKTRTIKLGMKRAEAIHYFLNWCGSAHVTDDSQNITEASRPTMQVATQSAATQPAATQPLHEVSDDASSDASSPVGHQTLSKEMLLNTAVETQMDKLGFLLNHIGKQVTTKVLSNAHITQTMKEIILENHSVDGGAAKNVSKGKSSPKEKKHWTEFESWEQLSKSKRSFKEYWAERNEIVNTLLLNWDNVRGAIKKFLDDDREWCGRINMINGVPEIVEIIPSPYRAGENIYFGSEAMMPADIYSRVANKPAMFVFHTHPNLGSCCGGMPSICDISTTLRYLLMGWTAGHLIISSNQVGMLTVDKRIIVDLWANENPRWLMAQKILDIFMMLTSRRSLVNPWTLRDLKKILQDYGIEYIIFPSNDFFIYEDERLLMFSKKWTNFFTLHELLDDLETIETKASSTTSTKKKPTITKQELYSLVAADTQLNKALIERIFTSQQKIIQNALKHNQEVIIPPGIKFTVVTVKAKPARQGHNPATGEPIQIKAKPEHKAVKIRALKPVHDMLNVEPREQFFQDLLSAVDQQMDTVKNDIKDIMKEKTSFMVSFENFIERYDTMEKNIQDLQNKYEEMAANLMTVMTDTKIQLGAIIAQLEILMINGTPLPAKKTTIKEAMPLPSSNTNNEQTSPPASGKTSETPKKNPTNAMFFTRSEWASSNTFREKFLTPEIQAILDEQFANKTGIERLHAEGLYMWRTQFSDEQKKMVKEMMKK

SEQ ID NO: 27 - protein, 973 aa, Artificial Sequence
  PLS-ASF fusion protein no. 2'
QIFVKTLTGKTITLEVEPSDTIENVKGKIQEKEGIPPDQQRLIFAGKQLEDGRTLSDYNIQKESTLHLVLRLRGADFILNISMKMEVIFKTDLRSSSQVVFHAGSLYNWFSVEIINSGRIVTTAIKTLLSTVKYDIVKSARIYAGQGYTEHQAQEEWNMILHVLFEEETESSASSESIHEKNDNETNECTSSFETLFEQEPSSETPKDSKLYMLAQKTVQHIEQYGKAPDFNKVIRAHNFIQTIHGTPLKEEEKEVVRLMVIKLLKKKDSEFFQPVYPRHYGECLSPVTTPSFFSTHMYTILIAIVVLVIIIIVLIYLFSSRKKKAAAAIEEEDIQFINPYQDQQWAEVTPQPGTSKPAGATTASVGKPVTGRPATNRPATNKPVTDNPVTDRLVMATGGPAAAPAAASAPAHPAEPYTTVTTQNTASQTMSAIENLRQRNTYTHKDLENSLFSKKKYIGLIDKKCELKKILDDYSILIIGILIGTNIITLIYNFIGWINYIKCYQNDDKMFYCPKDWVGYNNVCYYFSNEEKNYTNASNYCKQLNSTLANNNTNLVNLTKTLNLTKTYNHESNYWVNYSLIKNESVLLRNSGYYKKQKHVSLLYICSKIILIFLIFSNIVLSIIYWVSFNKTIILDSNITNDNNDINGVSWNTYFNNSFNTLATCGKAGNFCECSNYSTSLYNITNNCSLTIFPHNTDIFNTTYQLVYLNQKINYTIKLLTPVDSPNITYNCTNSLITCKKNNGTNTNIYLNINDTIVNYTNESILNYYWNNSNINNFTATCIINNTISSSNETELINCTNPTLKYQNYFYTFFKLFYIIIFIVSGIIISILFISIITFLSLRKRKKHVEEIESPPPSESNEEEQCQHDDTTSIHEPSPREPLLPKPYSRYQYNTPIYYMRPSTQPLNPFPLPKPCPPPKPCPPPKPCPPPKPCPSAESYSPPKPLPSIPLLPNIPPLSTQNISLIHVDRII

SEQ ID NO: 28 - protein, 2032 aa, Artificial Sequence
  PLS-ASF fusion protein no. 3'
QIFVKTLTGKTITLEVEPSDTIENVKGKIQEKEGIPPDQQRLIFAGKQLEDGRTLSDYNIQKESTLHLVLRLRGAYHDYASKLLADYRSDPPLWESDLPRHNRYSDNILNSRYCGNKNGAAPVYNEYTNSPEKAEKGLQLSDLRNFSFMLNPQHKNIGYGDAQDLEPYSSIPKNKLFNHFKNHRPAFSTHTENLIRRNVVRTEKKTFPQVASLKGTQKNCLTQPSSLPSLKNPKNSSVPSTRFSEHTKFFSYEDLPKLRTKGTIKHEQHLGDQMPGQHYNGYIPHKDVYNILCLAHNLPASVEKGIAGRGIPLGNPHVKPNIEQELIKSTSTYTDVPMLGPLPPKDSQHGREYQEFSANRHMLQVSNILHSVFANHSIKPQILEDIPVLNAQLTSIKPVSPFLNKAYQTHYMENIVTLVPRFKSIANYSSPIPNYSKRNSGQAEYFDTSKQTISRHNNYIPKYTGGIGDSKLDSTFPKDFNASSVPLTSAEKDHSLRGDNSACCISSISPSLPSNMKQFCKISVWLQQHDPDLLEIINNLCMLGNLSAAKYKHGVTFIYPKQAKIRDEIKKHAYSNDPSQAIKTLESLILPFYIPTPAEFTGEIGSYTGVKLEVEKTEANKVILKNGEAVLVPAADFKPFPDRRLAVWIMESGSMPLEGPPYKRKKEGGGNDPPVPKHISPYTPRTRIAIEVEKAFDDCMRQNWCSVNNPYLAKSVSLLSFLSLNHPTEFIKVLPLIDFDPLVTFYLLLEPYKTHGDDFLIPETILFGPTGWNGTDLYQSAMLEFKKFFTQITRQTFMDIADSATKEVDVPICYSDPETVHSYANHVRTEILHHNAVNKVTTPNLVVQAYNELEQTNTIRHYGPIFPESTINALRFWKKLWQDEQRFVIHGLHRTLMDQPTYETSEFAEIVRNLRFSRPGNNYINELNITSPAMYGDKHTTGDIAPNDRFAMLVAFINSTDFLYTAIPEEKVGGNETQTSSLTDLVPTRLHSFLNHNLSKLKILNRAQQTVRNILSNDCLNQLKHYVKHTGKNEILKLLQEYFLVADHREHHVIPFLKTDFHHMHQNPIQKKQALLEIKQLFTGDYLICKSPSTILACIERKTYKDFAASLKDGRYKNRQKMLSLREQTNCQLYFFVEGPAFPNPQKKINHVAYASIITAMTHLMVRDHIFVIQTKNEAHSSQKLVQLFYAFSKEMVCVVPTSLTPTDEELCIKLWSSLSGISGVIGKILANTCSVAHLVSGKLSSQNIDQLKTPSNRPFPKKVKRMLISISKGNKELEIKLLSGVPNIGKKLAAEILKDHALLFFLNQPVECLANIQIVQKTRTIKLGMKRAEAIHYFLNWCGSAHVTDDSQNITEASRPTMQVATQSAATQPAATQPLHEVSDDASSDASSPVGHQTLSKEMLLNTAVETQMDKLGFLLNHIGKQVTTKVLSNAHITQTMKEIILENHSVDGGAAKNVSKGKSSPKEKKHWTEFESWEQLSKSKRSFKEYWAERNEIVNTLLLNWDNVRGAIKKFLDDDREWCGRINMINGVPEIVEIIPSPYRAGENIYFGSEAMMPADIYSRVANKPAMFVFHTHPNLGSCCGGMPSICDISTTLRYLLMGWTAGHLIISSNQVGMLTVDKRIIVDLWANENPRWLMAQKILDIFMMLTSRRSLVNPWTLRDLKKILQDYGIEYIIFPSNDFFIYEDERLLMFSKKWTNFFTLHELLDDLETIETKASSTTSTKKKPTITKQELYSLVAADTQLNKALIERIFTSQQKIIQNALKHNQEVIIPPGIKFTVVTVKAKPARQGHNPATGEPIQIKAKPEHKAVKIRALKPVHDMLNVEPREQFFQDLLSAVDQQMDTVKNDIKDIMKEKTSFMVSFENFIERYDTMEKNIQDLQNKYEEMAANLMTVMTDTKIQLGAIIAQLEILMINGTPLPAKKTTIKEAMPLPSSNTNNEQTSPPASGKTSETPKKNPTNAMFFTRSEWASSNTFREKFLTPEIQAILDEQFANKTGIERLHAEGLYMWRTQFSDEQKKMVKEMMKK

SEQ ID NO: 29 - protein, 1502 aa, Artificial Sequence
  PLS-ASF fusion protein no. 4'
QIFVKTLTGKTITLEVEPSDTIENVKGKIQEKEGIPPDQQRLIFAGKQLEDGRTLSDYNIQKESTLHLVLRLRGADFILNISMKMEVIFKTDLRSSSQVVFHAGSLYNWFSVEIINSGRIVTTAIKTLLSTVKYDIVKSARIYAGQGYTEHQAQEEWNMILHVLFEEETESSASSESIHEKNDNETNECTSSFETLFEQEPSSETPKDSKLYMLAQKTVQHIEQYGKAPDFNKVIRAHNFIQTIHGTPLKEEEKEVVRLMVIKLLKKKDSEFFQPVYPRHYGECLSPVTTPSFFSTHMYTILIAIVVLVIIIIVLIYLFSSRKKKAAAAIEEEDIQFINPYQDQQWAEVTPQPGTSKPAGATTASVGKPVTGRPATNRPATNKPVTDNPVTDRLVMATGGPAAAPAAASAPAHPAEPYTTVTTQNTASQTMSAIENLRQRNTYTHKDLENSLPSNMKQFCKISVWLQQHDPDLLEIINNLCMLGNLSAAKYKHGVTFIYPKQAKIRDEIKKHAYSNDPSQAIKTLESLILPFYIPTPAEFTGEIGSYTGVKLEVEKTEANKVILKNGEAVLVPAADFKPFPDRRLAVWIMESGSMPLEGPPYKRKKEGGGNDPPVPKHISPYTPRTRIAIEVEKAFDDCMRQNWCSVNNPYLAKSVSLLSFLSLNHPTEFIKVLPLIDFDPLVTFYLLLEPYKTHGDDFLIPETILFGPTGWNGTDLYQSAMLEFKKFFTQITRQTFMDIADSATKEVDVPICYSDPETVHSYANHVRTEILHHNAVNKVTTPNLVVQAYNELEQTNTIRHYGPIFPESTINALRFWKKLWQDEQRFVIHGLHRTLMDQPTYETSEFAEIVRNLRFSRPGNNYINELNITSPAMYGDKHTTGDIAPNDRFAMLVAFINSTDFLYTAIPEEKVGGNETQTSSLTDLVPTRLHSFLNHNLSKLKILNRAQQTVRNILSNDCLNQLKHYVKHTGKNEILKLLQEFSKKKYIGLIDKKCELKKILDDYSILIIGILIGTNIITLIYNFIGWINYIKCYQNDDKMFYCPKDWVGYNNVCYYFSNEEKNYTNASNYCKQLNSTLANNNTNLVNLTKTLNLTKTYNHESNYWVNYSLIKNESVLLRNSGYYKKQKHVSLLYICSKIILIFLIFSNIVLSIIYWVSFNKTIILDSNITNDNNDINGVSWNTYFNNSFNTLATCGKAGNFCECSNYSTSLYNITNNCSLTIFPHNTDIFNTTYQLVYLNQKINYTIKLLTPVDSPNITYNCTNSLITCKKNNGTNTNIYLNINDTIVNYTNESILNYYWNNSNINNFTATCIINNTISSSNETELINCTNPTLKYQNYFYTFFKLFYIIIFIVSGIIISILFISIITFLSLRKRKKHVEEIESPPPSESNEEEQCQHDDTTSIHEPSPREPLLPKPYSRYQYNTPIYYMRPSTQPLNPFPLPKPCPPPKPCPPPKPCPPPKPCPSAESYSPPKPLPSIPLLPNIPPLSTQNISLIHVDRII

SEQ ID NO: 30 - protein, 1503 aa, Artificial Sequence
  PLS-ASF fusion protein no. 5'
QIFVKTLTGKTITLEVEPSDTIENVKGKIQEKEGIPPDQQRLIFAGKQLEDGRTLSDYNIQKESTLHLVLRLRGAYHDYASKLLADYRSDPPLWESDLPRHNRYSDNILNSRYCGNKNGAAPVYNEYTNSPEKAEKGLQLSDLRNFSFMLNPQHKNIGYGDAQDLEPYSSIPKNKLFNHFKNHRPAFSTHTENLIRRNVVRTEKKTFPQVASLKGTQKNCLTQPSSLPSLKNPKNSSVPSTRFSEHTKFFSYEDLPKLRTKGTIKHEQHLGDQMPGQHYNGYIPHKDVYNILCLAHNLPASVEKGIAGRGIPLGNPHVKPNIEQELIKSTSTYTDVPMLGPLPPKDSQHGREYQEFSANRHMLQVSNILHSVFANHSIKPQILEDIPVLNAQLTSIKPVSPFLNKAYQTHYMENIVTLVPRFKSIANYSSPIPNYSKRNSGQAEYFDTSKQTISRHNNYIPKYTGGIGDSKLDSTFPKDFNASSVPLTSAEKDHSLRGDNSACCISSISPSLYFLVADHREHHVIPFLKTDFHHMHQNPIQKKQALLEIKQLFTGDYLICKSPSTILACIERKTYKDFAASLKDGRYKNRQKMLSLREQTNCQLYFFVEGPAFPNPQKKINHVAYASIITAMTHLMVRDHIFVIQTKNEAHSSQKLVQLFYAFSKEMVCVVPTSLTPTDEELCIKLWSSLSGISGVIGKILANTCSVAHLVSGKLSSQNIDQLKTPSNRPFPKKVKRMLISISKGNKELEIKLLSGVPNIGKKLAAEILKDHALLFFLNQPVECLANIQIVQKTRTIKLGMKRAEAIHYFLNWCGSAHVTDDSQNITEASRPTMQVATQSAATQPAATQPLHEVSDDASSDASSPVGHQTLSKEMLLNTAVETQMDKLGFLLNHIGKQVTTKVLSNAHITQTMKEIILENHSVDGGAAKNVSKGKSSPKEKKHWTEFESWEQLSKSKRSFKEYWAERNEIVNTLLLNWDNVRGAIKKFLDDDREWCGRINMINGVPEIVEIIPSPYRAGENIYFGSEAMMPADIYSRVANKPAMFVFHTHPNLGSCCGGMPSICDISTTLRYLLMGWTAGHLIISSNQVGMLTVDKRIIVDLWANENPRWLMAQKILDIFMMLTSRRSLVNPWTLRDLKKILQDYGIEYIIFPSNDFFIYEDERLLMFSKKWTNFFTLHELLDDLETIETKASSTTSTKKKPTITKQELYSLVAADTQLNKALIERIFTSQQKIIQNALKHNQEVIIPPGIKFTVVTVKAKPARQGHNPATGEPIQIKAKPEHKAVKIRALKPVHDMLNVEPREQFFQDLLSAVDQQMDTVKNDIKDIMKEKTSFMVSFENFIERYDTMEKNIQDLQNKYEEMAANLMTVMTDTKIQLGAIIAQLEILMINGTPLPAKKTTIKEAMPLPSSNTNNEQTSPPASGKTSETPKKNPTNAMFFTRSEWASSNTFREKFLTPEIQAILDEQFANKTGIERLHAEGLYMWRTQFSDEQKKMVKEMMKK

SEQ ID NO: 31 - DNA, 8565 bp, Artificial Sequence
  PLS-ASF fusion protein no. 1
gattttattttaaatatatccatgaaaatggaggtcatcttcaaaacggatttaagatcatcttcacaagttgtgtttcatgcgggtagcctgtataattggttttctgttgagattatcaatagcggtagaattgttacgaccgctataaaaacattgcttagtactgttaagtatgatattgtgaaatctgctcgtatatatgcagggcaagggtatactgaacatcaggctcaagaagaatggaatatgattctgcatgtgctgtttgaagaggagacggaatcctcagcatcttcggagtcaattcatgaaaaaaatgataatgaaaccaatgaatgcacatcctcctttgaaacgttgtttgagcaagagccctcatcggagacacctaaagactccaagctgtatatgcttgcacaaaagactgtgcaacatattgaacaatatggaaaggcacctgattttaacaaggttattagagcacataattttattcaaaccattcatggaacccctctaaaggaagaagaaaaagaggtggtaagactcatggttattaaacttttaaaaaaaaaagattctgaattttttcaaccggtttatccgcggcattatggtgagtgtttgtcaccagtcactacaccaagcttcttctccacacatatgtatactattctcattgctatcgtggtcttagtcatcattatcatcgttctaatctatctattctcttcaagaaagaaaaaagctgctgctgctattgaggaggaagatatacagtttataaatccttatcaagatcagcagtgggcagaagtcactccacaaccaggtacctctaaaccagctggagcgactacagcaagtgtaggcaagccagtcacgggcagaccggcaacaaacagaccagcaacaaacaaaccagttacggacaacccagttacggacagactagtcatggcaactggcgggccggcggccgcacctgcggccgcgagtgctcctgctcatccggctgagccttacacgacagtcactactcagaacactgcttcacaaacaatgtcggctattgaaaatttacgacaaagaaacacctatacgcataaagacctagaaaactccttgttttctaagaaaaagtacatcggtcttatcgataagaagtgtgaattgaaaaaaatactagatgattatagtatattaataattggaatattaattggaactaacatcataacccttatttataattttataggatggattaattatataaaatgttaccaaaatgatgataagatgttttattgccctaaagattgggttggatataataatgtttgttattattttagtaatgaagaaaaaaattatactaatgcaagtaattattgtaagcaattaaatagtacgcttgctaataataatactaatttagtaaatcttactaaaacattaaatcttactaaaacatataatcacgaatctaattattgggttaattattctttaattaaaaatgagtcagtactattacgtaatagtggatattacaaaaaacaaaaacatgtaagtttattatatatttgtagtaaaataatacttatttttttaatattttctaacatagttttaagtattatatattgggttagttttaataaaacaataattttagatagtaatattactaatgataataatgatataaatggagtatcatggaatacttattttaataattcttttaatacactagctacatgtggaaaagcaggtaacttttgtgaatgttctaattatagtacatcactatataatataacaaataattgtagcttaactatttttcctcataatactgatatatttaatacaacatatcaactagtatatctaaatcaaaaaattaattatacaataaaattattaacacctgtagattctccaaatatcacatataattgtactaattctttaataacatgtaaaaaaaataatggaacaaacactaatatatatttaaatataaatgatactatagttaattatactaatgaaagtatacttaattattattggaataatagtaacattaacaattttacagctacatgtataattaataatacaattagttcttctaatgaaacagaacttataaattgtactaatcccacattgaaatatcaaaactatttttatactttttttaaattattttatattataatatttatcgtatctgggataataataagtattctttttatatccatcataacttttttatctttacgaaaaagaaaaaaacatgttgaagaaatagaaagtccaccaccttctgaatctaatgaagaagaacaatgtcagcatgatgacaccacttccatacatgaaccatctcccagagaaccattacttcctaagccttacagtcgttatcagtataatacacctatttactacatgcgtccctcaacacaaccactcaacccatttcccttacctaaaccgtgtcctccacccaaaccatgtccgccacccaaaccatgtcctccacctaaaccatgtccttcagctgaatcctattctccacccaaaccactacctagtatcccgctactacccaatatcccgccattatctacccaaaatatttcgcttattcacgtagatagaattatttatcatgattatgcttcaaagctgttagccgattataggtcagatccacctctttgggaaagcgatttgccgcgtcataaccggtattctgataatatactaaattcccggtactgcggcaacaaaaatggagctgcgcctgtatacaatgaatacactaatagtcctgaaaaggctgaaaagggattgcaactcagtgatctacgtaacttttcttttatgctgaaccctcagcacaaaaacattggttacggcgatgcgcaagatctggagccgtacagctccattccaaaaaataaactttttaatcattttaaaaatcatcgtcctgctttttcaacccatacggaaaacctaattaggcgcaatgttgttcgtacggaaaaaaaaacatttccgcaggtggctagcttaaagggcacacagaaaaattgtctgacccagccttcctcattgccttccttaaaaaacccaaaaaatagttcggttccttctacgaggttcagcgagcacacaaaatttttttcgtacgaggatcttcctaaactcagaacaaagggtaccattaagcatgagcagcaccttggcgatcagatgccgggccagcactataacggatatattccgcacaaagacgtgtacaatattttgtgtttagcgcacaatctacctgcgtcggtagaaaaagggattgcaggtagaggtattcctttaggaaatccacatgtcaaaccgaacatagagcaggaactcataaaatccaccagtacctacacggacgtgccgatgcttggtccccttccgcccaaagattcgcaacacggcagagaataccaggaattttccgcaaatagacatatgctacaagtatctaatatactacattctgtgtttgctaatcattctataaagccacaaatcctagaagacataccggtactcaatgcacaactaacaagcataaagccggtaagcccatttttaaacaaagcgtatcaaacccattatatggaaaatattgttaccttggtgccccggtttaagagtattgccaactactcaagccctataccgaattattctaaaagaaatagcggtcaggctgaatattttgatacctcaaagcaaacaatttctagacacaataattatatacctaaatatacgggaggaattggagattccaaactagacagcacctttcctaaagatttcaacgcctcctcggtaccgttaacaagcgcggaaaaggaccattccctgcggggagacaactcagcatgttgcatctcatctatatctccatcattgccctctaatatgaaacagttttgcaagatttctgtatggctacagcagcacgatccagatttattagaaattatcaacaacttatgtatgcttggcaatttatccgcggcaaagtacaaacacggagttaccttcatttaccccaaacaggcaaagatccgcgatgaaataaaaaaacatgcctactccaatgacccttcacaagccataaagaccttagaatcactcatccttccattttacattcccactccagcggagttcaccggggaaatcggctcctacaccggagtgaaattagaggttgaaaaaacggaggcgaataaagttattttaaaaaatggagaagcggtcctagtaccggcggccgattttaagccctttcctgatcgccgactagcggtctggatcatggagtcaggctctatgcccctggagggtcccccctataagcggaaaaaggagggtggggggaatgacccgccggttcctaagcatatctcgccgtatactccgcgcacgcgtattgccattgaggtggaaaaggcctttgatgactgtatgcgtcaaaactggtgtagtgtcaataatccctatcttgccaagtcggtctccttgctgtctttcttgtcgctcaaccatcccaccgagtttattaaggtactgccgcttatagactttgaccccttggtgaccttttatctacttcttgagccctataaaacgcatggggatgactttttaattccggaaaccattttattcggccctaccggatggaatggtacagatctgtatcaaagtgccatgctggagtttaaaaagttttttacccagattactcgccaaacctttatggacatagccgattcggctactaaggaggtagatgttcccatatgttactcggatcccgaaaccgtacattcctatgccaatcacgtgcgtactgaaattttgcatcacaatgccgtcaataaggttacaacacctaacctcgtcgtgcaggcctataatgagctcgagcaaaccaataccatacgacattacggccctattttcccggaaagtaccatcaacgcactgcgtttttggaaaaagctgtggcaggatgaacagcgatttgttatccacggcctgcaccgcacgttgatggatcaacccacctatgaaacctctgagtttgcagagatcgttagaaatttacggttttcgcgtcccggcaataactatataaacgagcttaatattacaagtcccgctatgtacggcgacaagcataccaccggagatattgcgcccaatgatagatttgccatgttggtggcctttatcaacagtactgactttttatacaccgcgattcccgaggaaaaggtaggggggaatgaaacccaaaccagtagccttacagacctagttccaacacggctacactcttttttaaatcataatctaagcaaacttaaaatcttaaaccgcgcgcagcaaacggttagaaatattctttcaaatgattgtcttaatcaactgaaacattatgttaaacacacgggaaaaaatgaaatactaaagttacttcaagaatattttctagtagcagatcatcgagaacatcatgtgattccttttcttaaaaccgatttccatcacatgcatcaaaatcctatacaaaaaaaacaagctctcctagaaatcaaacagctttttactggagattatctcatctgcaaaagcccttctaccattctggcctgtattgaacgaaaaacctacaaagactttgcggcttctttgaaagatggacgttataaaaatcgccaaaaaatgctgtcgctgcgagaacaaaccaactgtcaactttatttttttgtagaaggcccggcatttcctaaccctcaaaaaaaaattaatcacgttgcctatgcaagcattattactgctatgacgcatcttatggttagagatcatatttttgtcattcaaacgaaaaatgaggcccacagttcccaaaagcttgtgcagcttttttatgccttttctaaggaaatggtgtgcgtcgttcccacctccctcacccccacggatgaagagctatgcatcaagctatggtcttctctttctggtatttcaggcgtgataggtaaaatcttggcaaacacttgttccgtagctcatttggtttctggaaagctttcatcgcagaatattgatcagttaaaaactccctccaaccgaccattccccaaaaaagtaaaacgtatgcttataagcattagcaaaggaaataaggagttagaaataaaattgctctcgggggttcccaatatcgggaaaaaattagctgccgaaattttaaaagatcatgcgcttcttttttttctaaatcagcccgtagaatgcttggcaaatatacaaatcgttcaaaaaacccgtacgattaagttgggaatgaagcgagccgaagcgattcattattttttaaactggtgtggctctgcccatgtaaccgatgatagccaaaatatcacagaggcgtcgcggcctacaatgcaggtcgcgacgcagtccgccgcaactcagcccgctgcaacgcagccattgcacgaagtatcagatgatgcatcatcagatgcttcatcacccgtagggcatcaaacattatctaaagaaatgttattgaacacagccgttgagacacaaatggacaaacttggttttctgctaaatcacataggtaaacaggttaccactaaggtgcttagcaatgcccatataactcaaacgatgaaggagattattttggaaaatcatagtgtagatggtggagccgcaaaaaatgtttcaaaagggaagtcttccccaaaagaaaaaaaacattggactgagttcgaatcctgggaacagctcagcaagtctaaaagaagttttaaggaatactgggcggagcgtaatgagattgtgaatactctgttgcttaactgggacaatgttcggggtgccatcaaaaaatttttggacgatgaccgtgaatggtgcggccgcattaatatgataaacggtgtacccgagatagtggaaatcattccaagcccctatagggcaggagagaacatttattttggcagcgaggctatgatgcctgctgatatttatagcagggtggccaacaagcctgctatgtttgtgtttcacacgcatcctaatttgggttcatgttgtggaggaatgccttccatatgtgacatttctacaacgctgcgttatctactcatggggtggactgctgggcatctaatcatttcttcgaatcaagtaggaatgctcacggttgataagagaattattgttgatttgtgggccaatgagaatccgcgctggcttatggcgcaaaaaatattagatatttttatgatgctcacttcgcgtagaagcctggtaaatccctggaccctgagagacctaaaaaaaatattacaagactatggtattgagtatatcatttttccttcgaatgacttttttatttatgaagacgaacgtcttttaatgttttcaaaaaaatggaccaacttttttacgttacatgagttattggatgacctcgaaactattgagacaaaggcatcgtccacaacatcgacaaaaaaaaagcccacaattaccaagcaagagctttactccttagtagcggcagatacccagttaaataaagcattgattgaaagaatctttacaagtcagcaaaaaataatacaaaatgctttaaagcacaatcaagaagttattataccacccggaatcaagttcaccgtcgttacggtgaaagctaaacctgctcgccagggccataatcccgccacaggagagcctattcaaattaaagctaaacctgaacataaagccgtaaagatacgagcattgaaacctgtccatgatatgttaaacgttgagccacgcgaacagttttttcaagatctgctttcagcagtggatcaacaaatggacactgtaaaaaatgacataaaagacattatgaaagaaaaaacgtcttttatggtatcattcgaaaactttatagaacgttacgataccatggaaaaaaatattcaagaccttcagaataagtacgaagaaatggcggccaaccttatgaccgtcatgacggatacaaaaattcagcttggagccattatcgcccaacttgagattctaatgataaatggcactccacttccggcaaaaaagacaacaattaaggaggctatgcccttaccttcatcaaacacgaataatgaacaaacgagtcctcccgcctcaggcaaaacaagtgaaacacctaaaaaaaatcccacgaatgcgatgttcttcacgcgtagcgaatgggcatcctcgaatacttttcgagaaaagtttttaacaccagaaattcaagccatattggatgagcagtttgcaaacaagaccgggatcgaaagattgcatgccgagggtctttacatgtggagaacccaattctctgacgaacagaagaaaatggtcaaagagatgatgaagaag

SEQ ID NO: 32 - DNA, 2694 bp, Artificial Sequence
  PLS-ASF fusion protein no. 2
gattttattttaaatatatccatgaaaatggaggtcatcttcaaaacggatttaagatcatcttcacaagttgtgtttcatgcgggtagcctgtataattggttttctgttgagattatcaatagcggtagaattgttacgaccgctataaaaacattgcttagtactgttaagtatgatattgtgaaatctgctcgtatatatgcagggcaagggtatactgaacatcaggctcaagaagaatggaatatgattctgcatgtgctgtttgaagaggagacggaatcctcagcatcttcggagtcaattcatgaaaaaaatgataatgaaaccaatgaatgcacatcctcctttgaaacgttgtttgagcaagagccctcatcggagacacctaaagactccaagctgtatatgcttgcacaaaagactgtgcaacatattgaacaatatggaaaggcacctgattttaacaaggttattagagcacataattttattcaaaccattcatggaacccctctaaaggaagaagaaaaagaggtggtaagactcatggttattaaacttttaaaaaaaaaagattctgaattttttcaaccggtttatccgcggcattatggtgagtgtttgtcaccagtcactacaccaagcttcttctccacacatatgtatactattctcattgctatcgtggtcttagtcatcattatcatcgttctaatctatctattctcttcaagaaagaaaaaagctgctgctgctattgaggaggaagatatacagtttataaatccttatcaagatcagcagtgggcagaagtcactccacaaccaggtacctctaaaccagctggagcgactacagcaagtgtaggcaagccagtcacgggcagaccggcaacaaacagaccagcaacaaacaaaccagttacggacaacccagttacggacagactagtcatggcaactggcgggccggcggccgcacctgcggccgcgagtgctcctgctcatccggctgagccttacacgacagtcactactcagaacactgcttcacaaacaatgtcggctattgaaaatttacgacaaagaaacacctatacgcataaagacctagaaaactccttgttttctaagaaaaagtacatcggtcttatcgataagaagtgtgaattgaaaaaaatactagatgattatagtatattaataattggaatattaattggaactaacatcataacccttatttataattttataggatggattaattatataaaatgttaccaaaatgatgataagatgttttattgccctaaagattgggttggatataataatgtttgttattattttagtaatgaagaaaaaaattatactaatgcaagtaattattgtaagcaattaaatagtacgcttgctaataataatactaatttagtaaatcttactaaaacattaaatcttactaaaacatataatcacgaatctaattattgggttaattattctttaattaaaaatgagtcagtactattacgtaatagtggatattacaaaaaacaaaaacatgtaagtttattatatatttgtagtaaaataatacttatttttttaatattttctaacatagttttaagtattatatattgggttagttttaataaaacaataattttagatagtaatattactaatgataataatgatataaatggagtatcatggaatacttattttaataattcttttaatacactagctacatgtggaaaagcaggtaacttttgtgaatgttctaattatagtacatcactatataatataacaaataattgtagcttaactatttttcctcataatactgatatatttaatacaacatatcaactagtatatctaaatcaaaaaattaattatacaataaaattattaacacctgtagattctccaaatatcacatataattgtactaattctttaataacatgtaaaaaaaataatggaacaaacactaatatatatttaaatataaatgatactatagttaattatactaatgaaagtatacttaattattattggaataatagtaacattaacaattttacagctacatgtataattaataatacaattagttcttctaatgaaacagaacttataaattgtactaatcccacattgaaatatcaaaactatttttatactttttttaaattattttatattataatatttatcgtatctgggataataataagtattctttttatatccatcataacttttttatctttacgaaaaagaaaaaaacatgttgaagaaatagaaagtccaccaccttctgaatctaatgaagaagaacaatgtcagcatgatgacaccacttccatacatgaaccatctcccagagaaccattacttcctaagccttacagtcgttatcagtataatacacctatttactacatgcgtccctcaacacaaccactcaacccatttcccttacctaaaccgtgtcctccacccaaaccatgtccgccacccaaaccatgtcctccacctaaaccatgtccttcagctgaatcctattctccacccaaaccactacctagtatcccgctactacccaatatcccgccattatctacccaaaatatttcgcttattcacgtagatagaattatt

SEQ ID NO: 33 - DNA, 5871 bp, Artificial Sequence
  PLS-ASF fusion protein no. 3
tatcatgattatgcttcaaagctgttagccgattataggtcagatccacctctttgggaaagcgatttgccgcgtcataaccggtattctgataatatactaaattcccggtactgcggcaacaaaaatggagctgcgcctgtatacaatgaatacactaatagtcctgaaaaggctgaaaagggattgcaactcagtgatctacgtaacttttcttttatgctgaaccctcagcacaaaaacattggttacggcgatgcgcaagatctggagccgtacagctccattccaaaaaataaactttttaatcattttaaaaatcatcgtcctgctttttcaacccatacggaaaacctaattaggcgcaatgttgttcgtacggaaaaaaaaacatttccgcaggtggctagcttaaagggcacacagaaaaattgtctgacccagccttcctcattgccttccttaaaaaacccaaaaaatagttcggttccttctacgaggttcagcgagcacacaaaatttttttcgtacgaggatcttcctaaactcagaacaaagggtaccattaagcatgagcagcaccttggcgatcagatgccgggccagcactataacggatatattccgcacaaagacgtgtacaatattttgtgtttagcgcacaatctacctgcgtcggtagaaaaagggattgcaggtagaggtattcctttaggaaatccacatgtcaaaccgaacatagagcaggaactcataaaatccaccagtacctacacggacgtgccgatgcttggtccccttccgcccaaagattcgcaacacggcagagaataccaggaattttccgcaaatagacatatgctacaagtatctaatatactacattctgtgtttgctaatcattctataaagccacaaatcctagaagacataccggtactcaatgcacaactaacaagcataaagccggtaagcccatttttaaacaaagcgtatcaaacccattatatggaaaatattgttaccttggtgccccggtttaagagtattgccaactactcaagccctataccgaattattctaaaagaaatagcggtcaggctgaatattttgatacctcaaagcaaacaatttctagacacaataattatatacctaaatatacgggaggaattggagattccaaactagacagcacctttcctaaagatttcaacgcctcctcggtaccgttaacaagcgcggaaaaggaccattccctgcggggagacaactcagcatgttgcatctcatctatatctccatcattgccctctaatatgaaacagttttgcaagatttctgtatggctacagcagcacgatccagatttattagaaattatcaacaacttatgtatgcttggcaatttatccgcggcaaagtacaaacacggagttaccttcatttaccccaaacaggcaaagatccgcgatgaaataaaaaaacatgcctactccaatgacccttcacaagccataaagaccttagaatcactcatccttccattttacattcccactccagcggagttcaccggggaaatcggctcctacaccggagtgaaattagaggttgaaaaaacggaggcgaataaagttattttaaaaaatggagaagcggtcctagtaccggcggccgattttaagccctttcctgatcgccgactagcggtctggatcatggagtcaggctctatgcccctggagggtcccccctataagcggaaaaaggagggtggggggaatgacccgccggttcctaagcatatctcgccgtatactccgcgcacgcgtattgccattgaggtggaaaaggcctttgatgactgtatgcgtcaaaactggtgtagtgtcaataatccctatcttgccaagtcggtctccttgctgtctttcttgtcgctcaaccatcccaccgagtttattaaggtactgccgcttatagactttgaccccttggtgaccttttatctacttcttgagccctataaaacgcatggggatgactttttaattccggaaaccattttattcggccctaccggatggaatggtacagatctgtatcaaagtgccatgctggagtttaaaaagttttttacccagattactcgccaaacctttatggacatagccgattcggctactaaggaggtagatgttcccatatgttactcggatcccgaaaccgtacattcctatgccaatcacgtgcgtactgaaattttgcatcacaatgccgtcaataaggttacaacacctaacctcgtcgtgcaggcctataatgagctcgagcaaaccaataccatacgacattacggccctattttcccggaaagtaccatcaacgcactgcgtttttggaaaaagctgtggcaggatgaacagcgatttgttatccacggcctgcaccgcacgttgatggatcaacccacctatgaaacctctgagtttgcagagatcgttagaaatttacggttttcgcgtcccggcaataactatataaacgagcttaatattacaagtcccgctatgtacggcgacaagcataccaccggagatattgcgcccaatgatagatttgccatgttggtggcctttatcaacagtactgactttttatacaccgcgattcccgaggaaaaggtaggggggaatgaaacccaaaccagtagccttacagacctagttccaacacggctacactcttttttaaatcataatctaagcaaacttaaaatcttaaaccgcgcgcagcaaacggttagaaatattctttcaaatgattgtcttaatcaactgaaacattatgttaaacacacgggaaaaaatgaaatactaaagttacttcaagaatattttctagtagcagatcatcgagaacatcatgtgattccttttcttaaaaccgatttccatcacatgcatcaaaatcctatacaaaaaaaacaagctctcctagaaatcaaacagctttttactggagattatctcatctgcaaaagcccttctaccattctggcctgtattgaacgaaaaacctacaaagactttgcggcttctttgaaagatggacgttataaaaatcgccaaaaaatgctgtcgctgcgagaacaaaccaactgtcaactttatttttttgtagaaggcccggcatttcctaaccctcaaaaaaaaattaatcacgttgcctatgcaagcattattactgctatgacgcatcttatggttagagatcatatttttgtcattcaaacgaaaaatgaggcccacagttcccaaaagcttgtgcagcttttttatgccttttctaaggaaatggtgtgcgtcgttcccacctccctcacccccacggatgaagagctatgcatcaagctatggtcttctctttctggtatttcaggcgtgataggtaaaatcttggcaaacacttgttccgtagctcatttggtttctggaaagctttcatcgcagaatattgatcagttaaaaactccctccaaccgaccattccccaaaaaagtaaaacgtatgcttataagcattagcaaaggaaataaggagttagaaataaaattgctctcgggggttcccaatatcgggaaaaaattagctgccgaaattttaaaagatcatgcgcttcttttttttctaaatcagcccgtagaatgcttggcaaatatacaaatcgttcaaaaaacccgtacgattaagttgggaatgaagcgagccgaagcgattcattattttttaaactggtgtggctctgcccatgtaaccgatgatagccaaaatatcacagaggcgtcgcggcctacaatgcaggtcgcgacgcagtccgccgcaactcagcccgctgcaacgcagccattgcacgaagtatcagatgatgcatcatcagatgcttcatcacccgtagggcatcaaacattatctaaagaaatgttattgaacacagccgttgagacacaaatggacaaacttggttttctgctaaatcacataggtaaacaggttaccactaaggtgcttagcaatgcccatataactcaaacgatgaaggagattattttggaaaatcatagtgtagatggtggagccgcaaaaaatgtttcaaaagggaagtcttccccaaaagaaaaaaaacattggactgagttcgaatcctgggaacagctcagcaagtctaaaagaagttttaaggaatactgggcggagcgtaatgagattgtgaatactctgttgcttaactgggacaatgttcggggtgccatcaaaaaatttttggacgatgaccgtgaatggtgcggccgcattaatatgataaacggtgtacccgagatagtggaaatcattccaagcccctatagggcaggagagaacatttattttggcagcgaggctatgatgcctgctgatatttatagcagggtggccaacaagcctgctatgtttgtgtttcacacgcatcctaatttgggttcatgttgtggaggaatgccttccatatgtgacatttctacaacgctgcgttatctactcatggggtggactgctgggcatctaatcatttcttcgaatcaagtaggaatgctcacggttgataagagaattattgttgatttgtgggccaatgagaatccgcgctggcttatggcgcaaaaaatattagatatttttatgatgctcacttcgcgtagaagcctggtaaatccctggaccctgagagacctaaaaaaaatattacaagactatggtattgagtatatcatttttccttcgaatgacttttttatttatgaagacgaacgtcttttaatgttttcaaaaaaatggaccaacttttttacgttacatgagttattggatgacctcgaaactattgagacaaaggcatcgtccacaacatcgacaaaaaaaaagcccacaattaccaagcaagagctttactccttagtagcggcagatacccagttaaataaagcattgattgaaagaatctttacaagtcagcaaaaaataatacaaaatgctttaaagcacaatcaagaagttattataccacccggaatcaagttcaccgtcgttacggtgaaagctaaacctgctcgccagggccataatcccgccacaggagagcctattcaaattaaagctaaacctgaacataaagccgtaaagatacgagcattgaaacctgtccatgatatgttaaacgttgagccacgcgaacagttttttcaagatctgctttcagcagtggatcaacaaatggacactgtaaaaaatgacataaaagacattatgaaagaaaaaacgtcttttatggtatcattcgaaaactttatagaacgttacgataccatggaaaaaaatattcaagaccttcagaataagtacgaagaaatggcggccaaccttatgaccgtcatgacggatacaaaaattcagcttggagccattatcgcccaacttgagattctaatgataaatggcactccacttccggcaaaaaagacaacaattaaggaggctatgcccttaccttcatcaaacacgaataatgaacaaacgagtcctcccgcctcaggcaaaacaagtgaaacacctaaaaaaaatcccacgaatgcgatgttcttcacgcgtagcgaatgggcatcctcgaatacttttcgagaaaagtttttaacaccagaaattcaagccatattggatgagcagtttgcaaacaagaccgggatcgaaagattgcatgccgagggtctttacatgtggagaacccaattctctgacgaacagaagaaaatggtcaaagagatgatgaagaag

SEQ ID NO: 34 - DNA, 4281 bp, Artificial Sequence
  PLS-ASF fusion protein no. 4
gattttattttaaatatatccatgaaaatggaggtcatcttcaaaacggatttaagatcatcttcacaagttgtgtttcatgcgggtagcctgtataattggttttctgttgagattatcaatagcggtagaattgttacgaccgctataaaaacattgcttagtactgttaagtatgatattgtgaaatctgctcgtatatatgcagggcaagggtatactgaacatcaggctcaagaagaatggaatatgattctgcatgtgctgtttgaagaggagacggaatcctcagcatcttcggagtcaattcatgaaaaaaatgataatgaaaccaatgaatgcacatcctcctttgaaacgttgtttgagcaagagccctcatcggagacacctaaagactccaagctgtatatgcttgcacaaaagactgtgcaacatattgaacaatatggaaaggcacctgattttaacaaggttattagagcacataattttattcaaaccattcatggaacccctctaaaggaagaagaaaaagaggtggtaagactcatggttattaaacttttaaaaaaaaaagattctgaattttttcaaccggtttatccgcggcattatggtgagtgtttgtcaccagtcactacaccaagcttcttctccacacatatgtatactattctcattgctatcgtggtcttagtcatcattatcatcgttctaatctatctattctcttcaagaaagaaaaaagctgctgctgctattgaggaggaagatatacagtttataaatccttatcaagatcagcagtgggcagaagtcactccacaaccaggtacctctaaaccagctggagcgactacagcaagtgtaggcaagccagtcacgggcagaccggcaacaaacagaccagcaacaaacaaaccagttacggacaacccagttacggacagactagtcatggcaactggcgggccggcggccgcacctgcggccgcgagtgctcctgctcatccggctgagccttacacgacagtcactactcagaacactgcttcacaaacaatgtcggctattgaaaatttacgacaaagaaacacctatacgcataaagacctagaaaactccttgccctctaatatgaaacagttttgcaagatttctgtatggctacagcagcacgatccagatttattagaaattatcaacaacttatgtatgcttggcaatttatccgcggcaaagtacaaacacggagttaccttcatttaccccaaacaggcaaagatccgcgatgaaataaaaaaacatgcctactccaatgacccttcacaagccataaagaccttagaatcactcatccttccattttacattcccactccagcggagttcaccggggaaatcggctcctacaccggagtgaaattagaggttgaaaaaacggaggcgaataaagttattttaaaaaatggagaagcggtcctagtaccggcggccgattttaagccctttcctgatcgccgactagcggtctggatcatggagtcaggctctatgcccctggagggtcccccctataagcggaaaaaggagggtggggggaatgacccgccggttcctaagcatatctcgccgtatactccgcgcacgcgtattgccattgaggtggaaaaggcctttgatgactgtatgcgtcaaaactggtgtagtgtcaataatccctatcttgccaagtcggtctccttgctgtctttcttgtcgctcaaccatcccaccgagtttattaaggtactgccgcttatagactttgaccccttggtgaccttttatctacttcttgagccctataaaacgcatggggatgactttttaattccggaaaccattttattcggccctaccggatggaatggtacagatctgtatcaaagtgccatgctggagtttaaaaagttttttacccagattactcgccaaacctttatggacatagccgattcggctactaaggaggtagatgttcccatatgttactcggatcccgaaaccgtacattcctatgccaatcacgtgcgtactgaaattttgcatcacaatgccgtcaataaggttacaacacctaacctcgtcgtgcaggcctataatgagctcgagcaaaccaataccatacgacattacggccctattttcccggaaagtaccatcaacgcactgcgtttttggaaaaagctgtggcaggatgaacagcgatttgttatccacggcctgcaccgcacgttgatggatcaacccacctatgaaacctctgagtttgcagagatcgttagaaatttacggttttcgcgtcccggcaataactatataaacgagcttaatattacaagtcccgctatgtacggcgacaagcataccaccggagatattgcgcccaatgatagatttgccatgttggtggcctttatcaacagtactgactttttatacaccgcgattcccgaggaaaaggtaggggggaatgaaacccaaaccagtagccttacagacctagttccaacacggctacactcttttttaaatcataatctaagcaaacttaaaatcttaaaccgcgcgcagcaaacggttagaaatattctttcaaatgattgtcttaatcaactgaaacattatgttaaacacacgggaaaaaatgaaatactaaagttacttcaagaattttctaagaaaaagtacatcggtcttatcgataagaagtgtgaattgaaaaaaatactagatgattatagtatattaataattggaatattaattggaactaacatcataacccttatttataattttataggatggattaattatataaaatgttaccaaaatgatgataagatgttttattgccctaaagattgggttggatataataatgtttgttattattttagtaatgaagaaaaaaattatactaatgcaagtaattattgtaagcaattaaatagtacgcttgctaataataatactaatttagtaaatcttactaaaacattaaatcttactaaaacatataatcacgaatctaattattgggttaattattctttaattaaaaatgagtcagtactattacgtaatagtggatattacaaaaaacaaaaacatgtaagtttattatatatttgtagtaaaataatacttatttttttaatattttctaacatagttttaagtattatatattgggttagttttaataaaacaataattttagatagtaatattactaatgataataatgatataaatggagtatcatggaatacttattttaataattcttttaatacactagctacatgtggaaaagcaggtaacttttgtgaatgttctaattatagtacatcactatataatataacaaataattgtagcttaactatttttcctcataatactgatatatttaatacaacatatcaactagtatatctaaatcaaaaaattaattatacaataaaattattaacacctgtagattctccaaatatcacatataattgtactaattctttaataacatgtaaaaaaaataatggaacaaacactaatatatatttaaatataaatgatactatagttaattatactaatgaaagtatacttaattattattggaataatagtaacattaacaattttacagctacatgtataattaataatacaattagttcttctaatgaaacagaacttataaattgtactaatcccacattgaaatatcaaaactatttttatactttttttaaattattttatattataatatttatcgtatctgggataataataagtattctttttatatccatcataacttttttatctttacgaaaaagaaaaaaacatgttgaagaaatagaaagtccaccaccttctgaatctaatgaagaagaacaatgtcagcatgatgacaccacttccatacatgaaccatctcccagagaaccattacttcctaagccttacagtcgttatcagtataatacacctatttactacatgcgtccctcaacacaaccactcaacccatttcccttacctaaaccgtgtcctccacccaaaccatgtccgccacccaaaccatgtcctccacctaaaccatgtccttcagctgaatcctattctccacccaaaccactacctagtatcccgctactacccaatatcccgccattatctacccaaaatatttcgcttattcacgtagatagaattatt

SEQ ID NO: 35 - DNA, 4284 bp, Artificial Sequence
  PLS-ASF fusion protein no. 5
tatcatgattatgcttcaaagctgttagccgattataggtcagatccacctctttgggaaagcgatttgccgcgtcataaccggtattctgataatatactaaattcccggtactgcggcaacaaaaatggagctgcgcctgtatacaatgaatacactaatagtcctgaaaaggctgaaaagggattgcaactcagtgatctacgtaacttttcttttatgctgaaccctcagcacaaaaacattggttacggcgatgcgcaagatctggagccgtacagctccattccaaaaaataaactttttaatcattttaaaaatcatcgtcctgctttttcaacccatacggaaaacctaattaggcgcaatgttgttcgtacggaaaaaaaaacatttccgcaggtggctagcttaaagggcacacagaaaaattgtctgacccagccttcctcattgccttccttaaaaaacccaaaaaatagttcggttccttctacgaggttcagcgagcacacaaaatttttttcgtacgaggatcttcctaaactcagaacaaagggtaccattaagcatgagcagcaccttggcgatcagatgccgggccagcactataacggatatattccgcacaaagacgtgtacaatattttgtgtttagcgcacaatctacctgcgtcggtagaaaaagggattgcaggtagaggtattcctttaggaaatccacatgtcaaaccgaacatagagcaggaactcataaaatccaccagtacctacacggacgtgccgatgcttggtccccttccgcccaaagattcgcaacacggcagagaataccaggaattttccgcaaatagacatatgctacaagtatctaatatactacattctgtgtttgctaatcattctataaagccacaaatcctagaagacataccggtactcaatgcacaactaacaagcataaagccggtaagcccatttttaaacaaagcgtatcaaacccattatatggaaaatattgttaccttggtgccccggtttaagagtattgccaactactcaagccctataccgaattattctaaaagaaatagcggtcaggctgaatattttgatacctcaaagcaaacaatttctagacacaataattatatacctaaatatacgggaggaattggagattccaaactagacagcacctttcctaaagatttcaacgcctcctcggtaccgttaacaagcgcggaaaaggaccattccctgcggggagacaactcagcatgttgcatctcatctatatctccatcattgtattttctagtagcagatcatcgagaacatcatgtgattccttttcttaaaaccgatttccatcacatgcatcaaaatcctatacaaaaaaaacaagctctcctagaaatcaaacagctttttactggagattatctcatctgcaaaagcccttctaccattctggcctgtattgaacgaaaaacctacaaagactttgcggcttctttgaaagatggacgttataaaaatcgccaaaaaatgctgtcgctgcgagaacaaaccaactgtcaactttatttttttgtagaaggcccggcatttcctaaccctcaaaaaaaaattaatcacgttgcctatgcaagcattattactgctatgacgcatcttatggttagagatcatatttttgtcattcaaacgaaaaatgaggcccacagttcccaaaagcttgtgcagcttttttatgccttttctaaggaaatggtgtgcgtcgttcccacctccctcacccccacggatgaagagctatgcatcaagctatggtcttctctttctggtatttcaggcgtgataggtaaaatcttggcaaacacttgttccgtagctcatttggtttctggaaagctttcatcgcagaatattgatcagttaaaaactccctccaaccgaccattccccaaaaaagtaaaacgtatgcttataagcattagcaaaggaaataaggagttagaaataaaattgctctcgggggttcccaatatcgggaaaaaattagctgccgaaattttaaaagatcatgcgcttcttttttttctaaatcagcccgtagaatgcttggcaaatatacaaatcgttcaaaaaacccgtacgattaagttgggaatgaagcgagccgaagcgattcattattttttaaactggtgtggctctgcccatgtaaccgatgatagccaaaatatcacagaggcgtcgcggcctacaatgcaggtcgcgacgcagtccgccgcaactcagcccgctgcaacgcagccattgcacgaagtatcagatgatgcatcatcagatgcttcatcacccgtagggcatcaaacattatctaaagaaatgttattgaacacagccgttgagacacaaatggacaaacttggttttctgctaaatcacataggtaaacaggttaccactaaggtgcttagcaatgcccatataactcaaacgatgaaggagattattttggaaaatcatagtgtagatggtggagccgcaaaaaatgtttcaaaagggaagtcttccccaaaagaaaaaaaacattggactgagttcgaatcctgggaacagctcagcaagtctaaaagaagttttaaggaatactgggcggagcgtaatgagattgtgaatactctgttgcttaactgggacaatgttcggggtgccatcaaaaaatttttggacgatgaccgtgaatggtgcggccgcattaatatgataaacggtgtacccgagatagtggaaatcattccaagcccctatagggcaggagagaacatttattttggcagcgaggctatgatgcctgctgatatttatagcagggtggccaacaagcctgctatgtttgtgtttcacacgcatcctaatttgggttcatgttgtggaggaatgccttccatatgtgacatttctacaacgctgcgttatctactcatggggtggactgctgggcatctaatcatttcttcgaatcaagtaggaatgctcacggttgataagagaattattgttgatttgtgggccaatgagaatccgcgctggcttatggcgcaaaaaatattagatatttttatgatgctcacttcgcgtagaagcctggtaaatccctggaccctgagagacctaaaaaaaatattacaagactatggtattgagtatatcatttttccttcgaatgacttttttatttatgaagacgaacgtcttttaatgttttcaaaaaaatggaccaacttttttacgttacatgagttattggatgacctcgaaactattgagacaaaggcatcgtccacaacatcgacaaaaaaaaagcccacaattaccaagcaagagctttactccttagtagcggcagatacccagttaaataaagcattgattgaaagaatctttacaagtcagcaaaaaataatacaaaatgctttaaagcacaatcaagaagttattataccacccggaatcaagttcaccgtcgttacggtgaaagctaaacctgctcgccagggccataatcccgccacaggagagcctattcaaattaaagctaaacctgaacataaagccgtaaagatacgagcattgaaacctgtccatgatatgttaaacgttgagccacgcgaacagttttttcaagatctgctttcagcagtggatcaacaaatggacactgtaaaaaatgacataaaagacattatgaaagaaaaaacgtcttttatggtatcattcgaaaactttatagaacgttacgataccatggaaaaaaatattcaagaccttcagaataagtacgaagaaatggcggccaaccttatgaccgtcatgacggatacaaaaattcagcttggagccattatcgcccaacttgagattctaatgataaatggcactccacttccggcaaaaaagacaacaattaaggaggctatgcccttaccttcatcaaacacgaataatgaacaaacgagtcctcccgcctcaggcaaaacaagtgaaacacctaaaaaaaatcccacgaatgcgatgttcttcacgcgtagcgaatgggcatcctcgaatacttttcgagaaaagtttttaacaccagaaattcaagccatattggatgagcagtttgcaaacaagaccgggatcgaaagattgcatgccgagggtctttacatgtggagaacccaattctctgacgaacagaagaaaatggtcaaagagatgatgaagaag

SEQ ID NO: 36 - DNA, 8790 bp, Artificial Sequence
  PLS-ASF fusion protein no. 1'
cagatctttgtaaagaccttgactggtaagaccatcaccctggaagtggagcccagtgacaccattgagaatgtcaaggggaagattcaagaaaaagagggcatccccccagaccagcagaggctgatctttgccgggaagcagctggaagatgggcgcaccctgtctgactacaacatccagaaggagtccaccctgcacctggtcctccgcctcagaggtgccgattttattttaaatatatccatgaaaatggaggtcatcttcaaaacggatttaagatcatcttcacaagttgtgtttcatgcgggtagcctgtataattggttttctgttgagattatcaatagcggtagaattgttacgaccgctataaaaacattgcttagtactgttaagtatgatattgtgaaatctgctcgtatatatgcagggcaagggtatactgaacatcaggctcaagaagaatggaatatgattctgcatgtgctgtttgaagaggagacggaatcctcagcatcttcggagtcaattcatgaaaaaaatgataatgaaaccaatgaatgcacatcctcctttgaaacgttgtttgagcaagagccctcatcggagacacctaaagactccaagctgtatatgcttgcacaaaagactgtgcaacatattgaacaatatggaaaggcacctgattttaacaaggttattagagcacataattttattcaaaccattcatggaacccctctaaaggaagaagaaaaagaggtggtaagactcatggttattaaacttttaaaaaaaaaagattctgaattttttcaaccggtttatccgcggcattatggtgagtgtttgtcaccagtcactacaccaagcttcttctccacacatatgtatactattctcattgctatcgtggtcttagtcatcattatcatcgttctaatctatctattctcttcaagaaagaaaaaagctgctgctgctattgaggaggaagatatacagtttataaatccttatcaagatcagcagtgggcagaagtcactccacaaccaggtacctctaaaccagctggagcgactacagcaagtgtaggcaagccagtcacgggcagaccggcaacaaacagaccagcaacaaacaaaccagttacggacaacccagttacggacagactagtcatggcaactggcgggccggcggccgcacctgcggccgcgagtgctcctgctcatccggctgagccttacacgacagtcactactcagaacactgcttcacaaacaatgtcggctattgaaaatttacgacaaagaaacacctatacgcataaagacctagaaaactccttgttttctaagaaaaagtacatcggtcttatcgataagaagtgtgaattgaaaaaaatactagatgattatagtatattaataattggaatattaattggaactaacatcataacccttatttataattttataggatggattaattatataaaatgttaccaaaatgatgataagatgttttattgccctaaagattgggttggatataataatgtttgttattattttagtaatgaagaaaaaaattatactaatgcaagtaattattgtaagcaattaaatagtacgcttgctaataataatactaatttagtaaatcttactaaaacattaaatcttactaaaacatataatcacgaatctaattattgggttaattattctttaattaaaaatgagtcagtactattacgtaatagtggatattacaaaaaacaaaaacatgtaagtttattatatatttgtagtaaaataatacttatttttttaatattttctaacatagttttaagtattatatattgggttagttttaataaaacaataattttagatagtaatattactaatgataataatgatataaatggagtatcatggaatacttattttaataattcttttaatacactagctacatgtggaaaagcaggtaacttttgtgaatgttctaattatagtacatcactatataatataacaaataattgtagcttaactatttttcctcataatactgatatatttaatacaacatatcaactagtatatctaaatcaaaaaattaattatacaataaaattattaacacctgtagattctccaaatatcacatataattgtactaattctttaataacatgtaaaaaaaataatggaacaaacactaatatatatttaaatataaatgatactatagttaattatactaatgaaagtatacttaattattattggaataatagtaacattaacaattttacagctacatgtataattaataatacaattagttcttctaatgaaacagaacttataaattgtactaatcccacattgaaatatcaaaactatttttatactttttttaaattattttatattataatatttatcgtatctgggataataataagtattctttttatatccatcataacttttttatctttacgaaaaagaaaaaaacatgttgaagaaatagaaagtccaccaccttctgaatctaatgaagaagaacaatgtcagcatgatgacaccacttccatacatgaaccatctcccagagaaccattacttcctaagccttacagtcgttatcagtataatacacctatttactacatgcgtccctcaacacaaccactcaacccatttcccttacctaaaccgtgtcctccacccaaaccatgtccgccacccaaaccatgtcctccacctaaaccatgtccttcagctgaatcctattctccacccaaaccactacctagtatcccgctactacccaatatcccgccattatctacccaaaatatttcgcttattcacgtagatagaattatttatcatgattatgcttcaaagctgttagccgattataggtcagatccacctctttgggaaagcgatttgccgcgtcataaccggtattctgataatatactaaattcccggtactgcggcaacaaaaatggagctgcgcctgtatacaatgaatacactaatagtcctgaaaaggctgaaaagggattgcaactcagtgatctacgtaacttttcttttatgctgaaccctcagcacaaaaacattggttacggcgatgcgcaagatctggagccgtacagctccattccaaaaaataaactttttaatcattttaaaaatcatcgtcctgctttttcaacccatacggaaaacctaattaggcgcaatgttgttcgtacggaaaaaaaaacatttccgcaggtggctagcttaaagggcacacagaaaaattgtctgacccagccttcctcattgccttccttaaaaaacccaaaaaatagttcggttccttctacgaggttcagcgagcacacaaaatttttttcgtacgaggatcttcctaaactcagaacaaagggtaccattaagcatgagcagcaccttggcgatcagatgccgggccagcactataacggatatattccgcacaaagacgtgtacaatattttgtgtttagcgcacaatctacctgcgtcggtagaaaaagggattgcaggtagaggtattcctttaggaaatccacatgtcaaaccgaacatagagcaggaactcataaaatccaccagtacctacacggacgtgccgatgcttggtccccttccgcccaaagattcgcaacacggcagagaataccaggaattttccgcaaatagacatatgctacaagtatctaatatactacattctgtgtttgctaatcattctataaagccacaaatcctagaagacataccggtactcaatgcacaactaacaagcataaagccggtaagcccatttttaaacaaagcgtatcaaacccattatatggaaaatattgttaccttggtgccccggtttaagagtattgccaactactcaagccctataccgaattattctaaaagaaatagcggtcaggctgaatattttgatacctcaaagcaaacaatttctagacacaataattatatacctaaatatacgggaggaattggagattccaaactagacagcacctttcctaaagatttcaacgcctcctcggtaccgttaacaagcgcggaaaaggaccattccctgcggggagacaactcagcatgttgcatctcatctatatctccatcattgccctctaatatgaaacagttttgcaagatttctgtatggctacagcagcacgatccagatttattagaaattatcaacaacttatgtatgcttggcaatttatccgcggcaaagtacaaacacggagttaccttcatttaccccaaacaggcaaagatccgcgatgaaataaaaaaacatgcctactccaatgacccttcacaagccataaagaccttagaatcactcatccttccattttacattcccactccagcggagttcaccggggaaatcggctcctacaccggagtgaaattagaggttgaaaaaacggaggcgaataaagttattttaaaaaatggagaagcggtcctagtaccggcggccgattttaagccctttcctgatcgccgactagcggtctggatcatggagtcaggctctatgcccctggagggtcccccctataagcggaaaaaggagggtggggggaatgacccgccggttcctaagcatatctcgccgtatactccgcgcacgcgtattgccattgaggtggaaaaggcctttgatgactgtatgcgtcaaaactggtgtagtgtcaataatccctatcttgccaagtcggtctccttgctgtctttcttgtcgctcaaccatcccaccgagtttattaaggtactgccgcttatagactttgaccccttggtgaccttttatctacttcttgagccctataaaacgcatggggatgactttttaattccggaaaccattttattcggccctaccggatggaatggtacagatctgtatcaaagtgccatgctggagtttaaaaagttttttacccagattactcgccaaacctttatggacatagccgattcggctactaaggaggtagatgttcccatatgttactcggatcccgaaaccgtacattcctatgccaatcacgtgcgtactgaaattttgcatcacaatgccgtcaataaggttacaacacctaacctcgtcgtgcaggcctataatgagctcgagcaaaccaataccatacgacattacggccctattttcccggaaagtaccatcaacgcactgcgtttttggaaaaagctgtggcaggatgaacagcgatttgttatccacggcctgcaccgcacgttgatggatcaacccacctatgaaacctctgagtttgcagagatcgttagaaatttacggttttcgcgtcccggcaataactatataaacgagcttaatattacaagtcccgctatgtacggcgacaagcataccaccggagatattgcgcccaatgatagatttgccatgttggtggcctttatcaacagtactgactttttatacaccgcgattcccgaggaaaaggtaggggggaatgaaacccaaaccagtagccttacagacctagttccaacacggctacactcttttttaaatcataatctaagcaaacttaaaatcttaaaccgcgcgcagcaaacggttagaaatattctttcaaatgattgtcttaatcaactgaaacattatgttaaacacacgggaaaaaatgaaatactaaagttacttcaagaatattttctagtagcagatcatcgagaacatcatgtgattccttttcttaaaaccgatttccatcacatgcatcaaaatcctatacaaaaaaaacaagctctcctagaaatcaaacagctttttactggagattatctcatctgcaaaagcccttctaccattctggcctgtattgaacgaaaaacctacaaagactttgcggcttctttgaaagatggacgttataaaaatcgccaaaaaatgctgtcgctgcgagaacaaaccaactgtcaactttatttttttgtagaaggcccggcatttcctaaccctcaaaaaaaaattaatcacgttgcctatgcaagcattattactgctatgacgcatcttatggttagagatcatatttttgtcattcaaacgaaaaatgaggcccacagttcccaaaagcttgtgcagcttttttatgccttttctaaggaaatggtgtgcgtcgttcccacctccctcacccccacggatgaagagctatgcatcaagctatggtcttctctttctggtatttcaggcgtgataggtaaaatcttggcaaacacttgttccgtagctcatttggtttctggaaagctttcatcgcagaatattgatcagttaaaaactccctccaaccgaccattccccaaaaaagtaaaacgtatgcttataagcattagcaaaggaaataaggagttagaaataaaattgctctcgggggttcccaatatcgggaaaaaattagctgccgaaattttaaaagatcatgcgcttcttttttttctaaatcagcccgtagaatgcttggcaaatatacaaatcgttcaaaaaacccgtacgattaagttgggaatgaagcgagccgaagcgattcattattttttaaactggtgtggctctgcccatgtaaccgatgatagccaaaatatcacagaggcgtcgcggcctacaatgcaggtcgcgacgcagtccgccgcaactcagcccgctgcaacgcagccattgcacgaagtatcagatgatgcatcatcagatgcttcatcacccgtagggcatcaaacattatctaaagaaatgttattgaacacagccgttgagacacaaatggacaaacttggttttctgctaaatcacataggtaaacaggttaccactaaggtgcttagcaatgcccatataactcaaacgatgaaggagattattttggaaaatcatagtgtagatggtggagccgcaaaaaatgtttcaaaagggaagtcttccccaaaagaaaaaaaacattggactgagttcgaatcctgggaacagctcagcaagtctaaaagaagttttaaggaatactgggcggagcgtaatgagattgtgaatactctgttgcttaactgggacaatgttcggggtgccatcaaaaaatttttggacgatgaccgtgaatggtgcggccgcattaatatgataaacggtgtacccgagatagtggaaatcattccaagcccctatagggcaggagagaacatttattttggcagcgaggctatgatgcctgctgatatttatagcagggtggccaacaagcctgctatgtttgtgtttcacacgcatcctaatttgggttcatgttgtggaggaatgccttccatatgtgacatttctacaacgctgcgttatctactcatggggtggactgctgggcatctaatcatttcttcgaatcaagtaggaatgctcacggttgataagagaattattgttgatttgtgggccaatgagaatccgcgctggcttatggcgcaaaaaatattagatatttttatgatgctcacttcgcgtagaagcctggtaaatccctggaccctgagagacctaaaaaaaatattacaagactatggtattgagtatatcatttttccttcgaatgacttttttatttatgaagacgaacgtcttttaatgttttcaaaaaaatggaccaacttttttacgttacatgagttattggatgacctcgaaactattgagacaaaggcatcgtccacaacatcgacaaaaaaaaagcccacaattaccaagcaagagctttactccttagtagcggcagatacccagttaaataaagcattgattgaaagaatctttacaagtcagcaaaaaataatacaaaatgctttaaagcacaatcaagaagttattataccacccggaatcaagttcaccgtcgttacggtgaaagctaaacctgctcgccagggccataatcccgccacaggagagcctattcaaattaaagctaaacctgaacataaagccgtaaagatacgagcattgaaacctgtccatgatatgttaaacgttgagccacgcgaacagttttttcaagatctgctttcagcagtggatcaacaaatggacactgtaaaaaatgacataaaagacattatgaaagaaaaaacgtcttttatggtatcattcgaaaactttatagaacgttacgataccatggaaaaaaatattcaagaccttcagaataagtacgaagaaatggcggccaaccttatgaccgtcatgacggatacaaaaattcagcttggagccattatcgcccaacttgagattctaatgataaatggcactccacttccggcaaaaaagacaacaattaaggaggctatgcccttaccttcatcaaacacgaataatgaacaaacgagtcctcccgcctcaggcaaaacaagtgaaacacctaaaaaaaatcccacgaatgcgatgttcttcacgcgtagcgaatgggcatcctcgaatacttttcgagaaaagtttttaacaccagaaattcaagccatattggatgagcagtttgcaaacaagaccgggatcgaaagattgcatgccgagggtctttacatgtggagaacccaattctctgacgaacagaagaaaatggtcaaagagatgatgaagaag

SEQ ID NO: 37 - DNA, 2919 bp, Artificial Sequence
  PLS-ASF fusion protein no. 2'
cagatctttgtaaagaccttgactggtaagaccatcaccctggaagtggagcccagtgacaccattgagaatgtcaaggggaagattcaagaaaaagagggcatccccccagaccagcagaggctgatctttgccgggaagcagctggaagatgggcgcaccctgtctgactacaacatccagaaggagtccaccctgcacctggtcctccgcctcagaggtgccgattttattttaaatatatccatgaaaatggaggtcatcttcaaaacggatttaagatcatcttcacaagttgtgtttcatgcgggtagcctgtataattggttttctgttgagattatcaatagcggtagaattgttacgaccgctataaaaacattgcttagtactgttaagtatgatattgtgaaatctgctcgtatatatgcagggcaagggtatactgaacatcaggctcaagaagaatggaatatgattctgcatgtgctgtttgaagaggagacggaatcctcagcatcttcggagtcaattcatgaaaaaaatgataatgaaaccaatgaatgcacatcctcctttgaaacgttgtttgagcaagagccctcatcggagacacctaaagactccaagctgtatatgcttgcacaaaagactgtgcaacatattgaacaatatggaaaggcacctgattttaacaaggttattagagcacataattttattcaaaccattcatggaacccctctaaaggaagaagaaaaagaggtggtaagactcatggttattaaacttttaaaaaaaaaagattctgaattttttcaaccggtttatccgcggcattatggtgagtgtttgtcaccagtcactacaccaagcttcttctccacacatatgtatactattctcattgctatcgtggtcttagtcatcattatcatcgttctaatctatctattctcttcaagaaagaaaaaagctgctgctgctattgaggaggaagatatacagtttataaatccttatcaagatcagcagtgggcagaagtcactccacaaccaggtacctctaaaccagctggagcgactacagcaagtgtaggcaagccagtcacgggcagaccggcaacaaacagaccagcaacaaacaaaccagttacggacaacccagttacggacagactagtcatggcaactggcgggccggcggccgcacctgcggccgcgagtgctcctgctcatccggctgagccttacacgacagtcactactcagaacactgcttcacaaacaatgtcggctattgaaaatttacgacaaagaaacacctatacgcataaagacctagaaaactccttgttttctaagaaaaagtacatcggtcttatcgataagaagtgtgaattgaaaaaaatactagatgattatagtatattaataattggaatattaattggaactaacatcataacccttatttataattttataggatggattaattatataaaatgttaccaaaatgatgataagatgttttattgccctaaagattgggttggatataataatgtttgttattattttagtaatgaagaaaaaaattatactaatgcaagtaattattgtaagcaattaaatagtacgcttgctaataataatactaatttagtaaatcttactaaaacattaaatcttactaaaacatataatcacgaatctaattattgggttaattattctttaattaaaaatgagtcagtactattacgtaatagtggatattacaaaaaacaaaaacatgtaagtttattatatatttgtagtaaaataatacttatttttttaatattttctaacatagttttaagtattatatattgggttagttttaataaaacaataattttagatagtaatattactaatgataataatgatataaatggagtatcatggaatacttattttaataattcttttaatacactagctacatgtggaaaagcaggtaacttttgtgaatgttctaattatagtacatcactatataatataacaaataattgtagcttaactatttttcctcataatactgatatatttaatacaacatatcaactagtatatctaaatcaaaaaattaattatacaataaaattattaacacctgtagattctccaaatatcacatataattgtactaattctttaataacatgtaaaaaaaataatggaacaaacactaatatatatttaaatataaatgatactatagttaattatactaatgaaagtatacttaattattattggaataatagtaacattaacaattttacagctacatgtataattaataatacaattagttcttctaatgaaacagaacttataaattgtactaatcccacattgaaatatcaaaactatttttatactttttttaaattattttatattataatatttatcgtatctgggataataataagtattctttttatatccatcataacttttttatctttacgaaaaagaaaaaaacatgttgaagaaatagaaagtccaccaccttctgaatctaatgaagaagaacaatgtcagcatgatgacaccacttccatacatgaaccatctcccagagaaccattacttcctaagccttacagtcgttatcagtataatacacctatttactacatgcgtccctcaacacaaccactcaacccatttcccttacctaaaccgtgtcctccacccaaaccatgtccgccacccaaaccatgtcctccacctaaaccatgtccttcagctgaatcctattctccacccaaaccactacctagtatcccgctactacccaatatcccgccattatctacccaaaatatttcgcttattcacgtagatagaattatt

SEQ ID NO: 38 - DNA, 6096 bp, Artificial Sequence
  PLS-ASF fusion protein no. 3'
cagatctttgtaaagaccttgactggtaagaccatcaccctggaagtggagcccagtgacaccattgagaatgtcaaggggaagattcaagaaaaagagggcatccccccagaccagcagaggctgatctttgccgggaagcagctggaagatgggcgcaccctgtctgactacaacatccagaaggagtccaccctgcacctggtcctccgcctcagaggtgcctatcatgattatgcttcaaagctgttagccgattataggtcagatccacctctttgggaaagcgatttgccgcgtcataaccggtattctgataatatactaaattcccggtactgcggcaacaaaaatggagctgcgcctgtatacaatgaatacactaatagtcctgaaaaggctgaaaagggattgcaactcagtgatctacgtaacttttcttttatgctgaaccctcagcacaaaaacattggttacggcgatgcgcaagatctggagccgtacagctccattccaaaaaataaactttttaatcattttaaaaatcatcgtcctgctttttcaacccatacggaaaacctaattaggcgcaatgttgttcgtacggaaaaaaaaacatttccgcaggtggctagcttaaagggcacacagaaaaattgtctgacccagccttcctcattgccttccttaaaaaacccaaaaaatagttcggttccttctacgaggttcagcgagcacacaaaatttttttcgtacgaggatcttcctaaactcagaacaaagggtaccattaagcatgagcagcaccttggcgatcagatgccgggccagcactataacggatatattccgcacaaagacgtgtacaatattttgtgtttagcgcacaatctacctgcgtcggtagaaaaagggattgcaggtagaggtattcctttaggaaatccacatgtcaaaccgaacatagagcaggaactcataaaatccaccagtacctacacggacgtgccgatgcttggtccccttccgcccaaagattcgcaacacggcagagaataccaggaattttccgcaaatagacatatgctacaagtatctaatatactacattctgtgtttgctaatcattctataaagccacaaatcctagaagacataccggtactcaatgcacaactaacaagcataaagccggtaagcccatttttaaacaaagcgtatcaaacccattatatggaaaatattgttaccttggtgccccggtttaagagtattgccaactactcaagccctataccgaattattctaaaagaaatagcggtcaggctgaatattttgatacctcaaagcaaacaatttctagacacaataattatatacctaaatatacgggaggaattggagattccaaactagacagcacctttcctaaagatttcaacgcctcctcggtaccgttaacaagcgcggaaaaggaccattccctgcggggagacaactcagcatgttgcatctcatctatatctccatcattgccctctaatatgaaacagttttgcaagatttctgtatggctacagcagcacgatccagatttattagaaattatcaacaacttatgtatgcttggcaatttatccgcggcaaagtacaaacacggagttaccttcatttaccccaaacaggcaaagatccgcgatgaaataaaaaaacatgcctactccaatgacccttcacaagccataaagaccttagaatcactcatccttccattttacattcccactccagcggagttcaccggggaaatcggctcctacaccggagtgaaattagaggttgaaaaaacggaggcgaataaagttattttaaaaaatggagaagcggtcctagtaccggcggccgattttaagccctttcctgatcgccgactagcggtctggatcatggagtcaggctctatgcccctggagggtcccccctataagcggaaaaaggagggtggggggaatgacccgccggttcctaagcatatctcgccgtatactccgcgcacgcgtattgccattgaggtggaaaaggcctttgatgactgtatgcgtcaaaactggtgtagtgtcaataatccctatcttgccaagtcggtctccttgctgtctttcttgtcgctcaaccatcccaccgagtttattaaggtactgccgcttatagactttgaccccttggtgaccttttatctacttcttgagccctataaaacgcatggggatgactttttaattccggaaaccattttattcggccctaccggatggaatggtacagatctgtatcaaagtgccatgctggagtttaaaaagttttttacccagattactcgccaaacctttatggacatagccgattcggctactaaggaggtagatgttcccatatgttactcggatcccgaaaccgtacattcctatgccaatcacgtgcgtactgaaattttgcatcacaatgccgtcaataaggttacaacacctaacctcgtcgtgcaggcctataatgagctcgagcaaaccaataccatacgacattacggccctattttcccggaaagtaccatcaacgcactgcgtttttggaaaaagctgtggcaggatgaacagcgatttgttatccacggcctgcaccgcacgttgatggatcaacccacctatgaaacctctgagtttgcagagatcgttagaaatttacggttttcgcgtcccggcaataactatataaacgagcttaatattacaagtcccgctatgtacggcgacaagcataccaccggagatattgcgcccaatgatagatttgccatgttggtggcctttatcaacagtactgactttttatacaccgcgattcccgaggaaaaggtaggggggaatgaaacccaaaccagtagccttacagacctagttccaacacggctacactcttttttaaatcataatctaagcaaacttaaaatcttaaaccgcgcgcagcaaacggttagaaatattctttcaaatgattgtcttaatcaactgaaacattatgttaaacacacgggaaaaaatgaaatactaaagttacttcaagaatattttctagtagcagatcatcgagaacatcatgtgattccttttcttaaaaccgatttccatcacatgcatcaaaatcctatacaaaaaaaacaagctctcctagaaatcaaacagctttttactggagattatctcatctgcaaaagcccttctaccattctggcctgtattgaacgaaaaacctacaaagactttgcggcttctttgaaagatggacgttataaaaatcgccaaaaaatgctgtcgctgcgagaacaaaccaactgtcaactttatttttttgtagaaggcccggcatttcctaaccctcaaaaaaaaattaatcacgttgcctatgcaagcattattactgctatgacgcatcttatggttagagatcatatttttgtcattcaaacgaaaaatgaggcccacagttcccaaaagcttgtgcagcttttttatgccttttctaaggaaatggtgtgcgtcgttcccacctccctcacccccacggatgaagagctatgcatcaagctatggtcttctctttctggtatttcaggcgtgataggtaaaatcttggcaaacacttgttccgtagctcatttggtttctggaaagctttcatcgcagaatattgatcagttaaaaactccctccaaccgaccattccccaaaaaagtaaaacgtatgcttataagcattagcaaaggaaataaggagttagaaataaaattgctctcgggggttcccaatatcgggaaaaaattagctgccgaaattttaaaagatcatgcgcttcttttttttctaaatcagcccgtagaatgcttggcaaatatacaaatcgttcaaaaaacccgtacgattaagttgggaatgaagcgagccgaagcgattcattattttttaaactggtgtggctctgcccatgtaaccgatgatagccaaaatatcacagaggcgtcgcggcctacaatgcaggtcgcgacgcagtccgccgcaactcagcccgctgcaacgcagccattgcacgaagtatcagatgatgcatcatcagatgcttcatcacccgtagggcatcaaacattatctaaagaaatgttattgaacacagccgttgagacacaaatggacaaacttggttttctgctaaatcacataggtaaacaggttaccactaaggtgcttagcaatgcccatataactcaaacgatgaaggagattattttggaaaatcatagtgtagatggtggagccgcaaaaaatgtttcaaaagggaagtcttccccaaaagaaaaaaaacattggactgagttcgaatcctgggaacagctcagcaagtctaaaagaagttttaaggaatactgggcggagcgtaatgagattgtgaatactctgttgcttaactgggacaatgttcggggtgccatcaaaaaatttttggacgatgaccgtgaatggtgcggccgcattaatatgataaacggtgtacccgagatagtggaaatcattccaagcccctatagggcaggagagaacatttattttggcagcgaggctatgatgcctgctgatatttatagcagggtggccaacaagcctgctatgtttgtgtttcacacgcatcctaatttgggttcatgttgtggaggaatgccttccatatgtgacatttctacaacgctgcgttatctactcatggggtggactgctgggcatctaatcatttcttcgaatcaagtaggaatgctcacggttgataagagaattattgttgatttgtgggccaatgagaatccgcgctggcttatggcgcaaaaaatattagatatttttatgatgctcacttcgcgtagaagcctggtaaatccctggaccctgagagacctaaaaaaaatattacaagactatggtattgagtatatcatttttccttcgaatgacttttttatttatgaagacgaacgtcttttaatgttttcaaaaaaatggaccaacttttttacgttacatgagttattggatgacctcgaaactattgagacaaaggcatcgtccacaacatcgacaaaaaaaaagcccacaattaccaagcaagagctttactccttagtagcggcagatacccagttaaataaagcattgattgaaagaatctttacaagtcagcaaaaaataatacaaaatgctttaaagcacaatcaagaagttattataccacccggaatcaagttcaccgtcgttacggtgaaagctaaacctgctcgccagggccataatcccgccacaggagagcctattcaaattaaagctaaacctgaacataaagccgtaaagatacgagcattgaaacctgtccatgatatgttaaacgttgagccacgcgaacagttttttcaagatctgctttcagcagtggatcaacaaatggacactgtaaaaaatgacataaaagacattatgaaagaaaaaacgtcttttatggtatcattcgaaaactttatagaacgttacgataccatggaaaaaaatattcaagaccttcagaataagtacgaagaaatggcggccaaccttatgaccgtcatgacggatacaaaaattcagcttggagccattatcgcccaacttgagattctaatgataaatggcactccacttccggcaaaaaagacaacaattaaggaggctatgcccttaccttcatcaaacacgaataatgaacaaacgagtcctcccgcctcaggcaaaacaagtgaaacacctaaaaaaaatcccacgaatgcgatgttcttcacgcgtagcgaatgggcatcctcgaatacttttcgagaaaagtttttaacaccagaaattcaagccatattggatgagcagtttgcaaacaagaccgggatcgaaagattgcatgccgagggtctttacatgtggagaacccaattctctgacgaacagaagaaaatggtcaaagagatgatgaagaag

SEQ ID NO: 39 - DNA, 4506 bp, Artificial Sequence
  PLS-ASF fusion protein no. 4'
cagatctttgtaaagaccttgactggtaagaccatcaccctggaagtggagcccagtgacaccattgagaatgtcaaggggaagattcaagaaaaagagggcatccccccagaccagcagaggctgatctttgccgggaagcagctggaagatgggcgcaccctgtctgactacaacatccagaaggagtccaccctgcacctggtcctccgcctcagaggtgccgattttattttaaatatatccatgaaaatggaggtcatcttcaaaacggatttaagatcatcttcacaagttgtgtttcatgcgggtagcctgtataattggttttctgttgagattatcaatagcggtagaattgttacgaccgctataaaaacattgcttagtactgttaagtatgatattgtgaaatctgctcgtatatatgcagggcaagggtatactgaacatcaggctcaagaagaatggaatatgattctgcatgtgctgtttgaagaggagacggaatcctcagcatcttcggagtcaattcatgaaaaaaatgataatgaaaccaatgaatgcacatcctcctttgaaacgttgtttgagcaagagccctcatcggagacacctaaagactccaagctgtatatgcttgcacaaaagactgtgcaacatattgaacaatatggaaaggcacctgattttaacaaggttattagagcacataattttattcaaaccattcatggaacccctctaaaggaagaagaaaaagaggtggtaagactcatggttattaaacttttaaaaaaaaaagattctgaattttttcaaccggtttatccgcggcattatggtgagtgtttgtcaccagtcactacaccaagcttcttctccacacatatgtatactattctcattgctatcgtggtcttagtcatcattatcatcgttctaatctatctattctcttcaagaaagaaaaaagctgctgctgctattgaggaggaagatatacagtttataaatccttatcaagatcagcagtgggcagaagtcactccacaaccaggtacctctaaaccagctggagcgactacagcaagtgtaggcaagccagtcacgggcagaccggcaacaaacagaccagcaacaaacaaaccagttacggacaacccagttacggacagactagtcatggcaactggcgggccggcggccgcacctgcggccgcgagtgctcctgctcatccggctgagccttacacgacagtcactactcagaacactgcttcacaaacaatgtcggctattgaaaatttacgacaaagaaacacctatacgcataaagacctagaaaactccttgccctctaatatgaaacagttttgcaagatttctgtatggctacagcagcacgatccagatttattagaaattatcaacaacttatgtatgcttggcaatttatccgcggcaaagtacaaacacggagttaccttcatttaccccaaacaggcaaagatccgcgatgaaataaaaaaacatgcctactccaatgacccttcacaagccataaagaccttagaatcactcatccttccattttacattcccactccagcggagttcaccggggaaatcggctcctacaccggagtgaaattagaggttgaaaaaacggaggcgaataaagttattttaaaaaatggagaagcggtcctagtaccggcggccgattttaagccctttcctgatcgccgactagcggtctggatcatggagtcaggctctatgcccctggagggtcccccctataagcggaaaaaggagggtggggggaatgacccgccggttcctaagcatatctcgccgtatactccgcgcacgcgtattgccattgaggtggaaaaggcctttgatgactgtatgcgtcaaaactggtgtagtgtcaataatccctatcttgccaagtcggtctccttgctgtctttcttgtcgctcaaccatcccaccgagtttattaaggtactgccgcttatagactttgaccccttggtgaccttttatctacttcttgagccctataaaacgcatggggatgactttttaattccggaaaccattttattcggccctaccggatggaatggtacagatctgtatcaaagtgccatgctggagtttaaaaagttttttacccagattactcgccaaacctttatggacatagccgattcggctactaaggaggtagatgttcccatatgttactcggatcccgaaaccgtacattcctatgccaatcacgtgcgtactgaaattttgcatcacaatgccgtcaataaggttacaacacctaacctcgtcgtgcaggcctataatgagctcgagcaaaccaataccatacgacattacggccctattttcccggaaagtaccatcaacgcactgcgtttttggaaaaagctgtggcaggatgaacagcgatttgttatccacggcctgcaccgcacgttgatggatcaacccacctatgaaacctctgagtttgcagagatcgttagaaatttacggttttcgcgtcccggcaataactatataaacgagcttaatattacaagtcccgctatgtacggcgacaagcataccaccggagatattgcgcccaatgatagatttgccatgttggtggcctttatcaacagtactgactttttatacaccgcgattcccgaggaaaaggtaggggggaatgaaacccaaaccagtagccttacagacctagttccaacacggctacactcttttttaaatcataatctaagcaaacttaaaatcttaaaccgcgcgcagcaaacggttagaaatattctttcaaatgattgtcttaatcaactgaaacattatgttaaacacacgggaaaaaatgaaatactaaagttacttcaagaattttctaagaaaaagtacatcggtcttatcgataagaagtgtgaattgaaaaaaatactagatgattatagtatattaataattggaatattaattggaactaacatcataacccttatttataattttataggatggattaattatataaaatgttaccaaaatgatgataagatgttttattgccctaaagattgggttggatataataatgtttgttattattttagtaatgaagaaaaaaattatactaatgcaagtaattattgtaagcaattaaatagtacgcttgctaataataatactaatttagtaaatcttactaaaacattaaatcttactaaaacatataatcacgaatctaattattgggttaattattctttaattaaaaatgagtcagtactattacgtaatagtggatattacaaaaaacaaaaacatgtaagtttattatatatttgtagtaaaataatacttatttttttaatattttctaacatagttttaagtattatatattgggttagttttaataaaacaataattttagatagtaatattactaatgataataatgatataaatggagtatcatggaatacttattttaataattcttttaatacactagctacatgtggaaaagcaggtaacttttgtgaatgttctaattatagtacatcactatataatataacaaataattgtagcttaactatttttcctcataatactgatatatttaatacaacatatcaactagtatatctaaatcaaaaaattaattatacaataaaattattaacacctgtagattctccaaatatcacatataattgtactaattctttaataacatgtaaaaaaaataatggaacaaacactaatatatatttaaatataaatgatactatagttaattatactaatgaaagtatacttaattattattggaataatagtaacattaacaattttacagctacatgtataattaataatacaattagttcttctaatgaaacagaacttataaattgtactaatcccacattgaaatatcaaaactatttttatactttttttaaattattttatattataatatttatcgtatctgggataataataagtattctttttatatccatcataacttttttatctttacgaaaaagaaaaaaacatgttgaagaaatagaaagtccaccaccttctgaatctaatgaagaagaacaatgtcagcatgatgacaccacttccatacatgaaccatctcccagagaaccattacttcctaagccttacagtcgttatcagtataatacacctatttactacatgcgtccctcaacacaaccactcaacccatttcccttacctaaaccgtgtcctccacccaaaccatgtccgccacccaaaccatgtcctccacctaaaccatgtccttcagctgaatcctattctccacccaaaccactacctagtatcccgctactacccaatatcccgccattatctacccaaaatatttcgcttattcacgtagatagaattatt

SEQ ID NO: 40 - DNA, 4509 bp, Artificial Sequence
  PLS-ASF fusion protein no. 5'
cagatctttgtaaagaccttgactggtaagaccatcaccctggaagtggagcccagtgacaccattgagaatgtcaaggggaagattcaagaaaaagagggcatccccccagaccagcagaggctgatctttgccgggaagcagctggaagatgggcgcaccctgtctgactacaacatccagaaggagtccaccctgcacctggtcctccgcctcagaggtgcctatcatgattatgcttcaaagctgttagccgattataggtcagatccacctctttgggaaagcgatttgccgcgtcataaccggtattctgataatatactaaattcccggtactgcggcaacaaaaatggagctgcgcctgtatacaatgaatacactaatagtcctgaaaaggctgaaaagggattgcaactcagtgatctacgtaacttttcttttatgctgaaccctcagcacaaaaacattggttacggcgatgcgcaagatctggagccgtacagctccattccaaaaaataaactttttaatcattttaaaaatcatcgtcctgctttttcaacccatacggaaaacctaattaggcgcaatgttgttcgtacggaaaaaaaaacatttccgcaggtggctagcttaaagggcacacagaaaaattgtctgacccagccttcctcattgccttccttaaaaaacccaaaaaatagttcggttccttctacgaggttcagcgagcacacaaaatttttttcgtacgaggatcttcctaaactcagaacaaagggtaccattaagcatgagcagcaccttggcgatcagatgccgggccagcactataacggatatattccgcacaaagacgtgtacaatattttgtgtttagcgcacaatctacctgcgtcggtagaaaaagggattgcaggtagaggtattcctttaggaaatccacatgtcaaaccgaacatagagcaggaactcataaaatccaccagtacctacacggacgtgccgatgcttggtccccttccgcccaaagattcgcaacacggcagagaataccaggaattttccgcaaatagacatatgctacaagtatctaatatactacattctgtgtttgctaatcattctataaagccacaaatcctagaagacataccggtactcaatgcacaactaacaagcataaagccggtaagcccatttttaaacaaagcgtatcaaacccattatatggaaaatattgttaccttggtgccccggtttaagagtattgccaactactcaagccctataccgaattattctaaaagaaatagcggtcaggctgaatattttgatacctcaaagcaaacaatttctagacacaataattatatacctaaatatacgggaggaattggagattccaaactagacagcacctttcctaaagatttcaacgcctcctcggtaccgttaacaagcgcggaaaaggaccattccctgcggggagacaactcagcatgttgcatctcatctatatctccatcattgtattttctagtagcagatcatcgagaacatcatgtgattccttttcttaaaaccgatttccatcacatgcatcaaaatcctatacaaaaaaaacaagctctcctagaaatcaaacagctttttactggagattatctcatctgcaaaagcccttctaccattctggcctgtattgaacgaaaaacctacaaagactttgcggcttctttgaaagatggacgttataaaaatcgccaaaaaatgctgtcgctgcgagaacaaaccaactgtcaactttatttttttgtagaaggcccggcatttcctaaccctcaaaaaaaaattaatcacgttgcctatgcaagcattattactgctatgacgcatcttatggttagagatcatatttttgtcattcaaacgaaaaatgaggcccacagttcccaaaagcttgtgcagcttttttatgccttttctaaggaaatggtgtgcgtcgttcccacctccctcacccccacggatgaagagctatgcatcaagctatggtcttctctttctggtatttcaggcgtgataggtaaaatcttggcaaacacttgttccgtagctcatttggtttctggaaagctttcatcgcagaatattgatcagttaaaaactccctccaaccgaccattccccaaaaaagtaaaacgtatgcttataagcattagcaaaggaaataaggagttagaaataaaattgctctcgggggttcccaatatcgggaaaaaattagctgccgaaattttaaaagatcatgcgcttcttttttttctaaatcagcccgtagaatgcttggcaaatatacaaatcgttcaaaaaacccgtacgattaagttgggaatgaagcgagccgaagcgattcattattttttaaactggtgtggctctgcccatgtaaccgatgatagccaaaatatcacagaggcgtcgcggcctacaatgcaggtcgcgacgcagtccgccgcaactcagcccgctgcaacgcagccattgcacgaagtatcagatgatgcatcatcagatgcttcatcacccgtagggcatcaaacattatctaaagaaatgttattgaacacagccgttgagacacaaatggacaaacttggttttctgctaaatcacataggtaaacaggttaccactaaggtgcttagcaatgcccatataactcaaacgatgaaggagattattttggaaaatcatagtgtagatggtggagccgcaaaaaatgtttcaaaagggaagtcttccccaaaagaaaaaaaacattggactgagttcgaatcctgggaacagctcagcaagtctaaaagaagttttaaggaatactgggcggagcgtaatgagattgtgaatactctgttgcttaactgggacaatgttcggggtgccatcaaaaaatttttggacgatgaccgtgaatggtgcggccgcattaatatgataaacggtgtacccgagatagtggaaatcattccaagcccctatagggcaggagagaacatttattttggcagcgaggctatgatgcctgctgatatttatagcagggtggccaacaagcctgctatgtttgtgtttcacacgcatcctaatttgggttcatgttgtggaggaatgccttccatatgtgacatttctacaacgctgcgttatctactcatggggtggactgctgggcatctaatcatttcttcgaatcaagtaggaatgctcacggttgataagagaattattgttgatttgtgggccaatgagaatccgcgctggcttatggcgcaaaaaatattagatatttttatgatgctcacttcgcgtagaagcctggtaaatccctggaccctgagagacctaaaaaaaatattacaagactatggtattgagtatatcatttttccttcgaatgacttttttatttatgaagacgaacgtcttttaatgttttcaaaaaaatggaccaacttttttacgttacatgagttattggatgacctcgaaactattgagacaaaggcatcgtccacaacatcgacaaaaaaaaagcccacaattaccaagcaagagctttactccttagtagcggcagatacccagttaaataaagcattgattgaaagaatctttacaagtcagcaaaaaataatacaaaatgctttaaagcacaatcaagaagttattataccacccggaatcaagttcaccgtcgttacggtgaaagctaaacctgctcgccagggccataatcccgccacaggagagcctattcaaattaaagctaaacctgaacataaagccgtaaagatacgagcattgaaacctgtccatgatatgttaaacgttgagccacgcgaacagttttttcaagatctgctttcagcagtggatcaacaaatggacactgtaaaaaatgacataaaagacattatgaaagaaaaaacgtcttttatggtatcattcgaaaactttatagaacgttacgataccatggaaaaaaatattcaagaccttcagaataagtacgaagaaatggcggccaaccttatgaccgtcatgacggatacaaaaattcagcttggagccattatcgcccaacttgagattctaatgataaatggcactccacttccggcaaaaaagacaacaattaaggaggctatgcccttaccttcatcaaacacgaataatgaacaaacgagtcctcccgcctcaggcaaaacaagtgaaacacctaaaaaaaatcccacgaatgcgatgttcttcacgcgtagcgaatgggcatcctcgaatacttttcgagaaaagtttttaacaccagaaattcaagccatattggatgagcagtttgcaaacaagaccgggatcgaaagattgcatgccgagggtctttacatgtggagaacccaattctctgacgaacagaagaaaatggtcaaagagatgatgaagaag

SEQ ID NO: 41 - protein, 75 aa, Artificial Sequence
  PLS-ASF ubiquitin
QIFVKTLTGKTITLEVEPSDTIENVKGKIQEKEGIPPDQQRLIFAGKQLEDGRTLSDYNIQKESTLHLVLRLRGA

SEQ ID NO: 42 - DNA, 225 bp, Artificial Sequence
  PLS-ASF ubiquitin
cagatctttgtaaagaccttgactggtaagaccatcaccctggaagtggagcccagtgacaccattgagaatgtcaaggggaagattcaagaaaaagagggcatccccccagaccagcagaggctgatctttgccgggaagcagctggaagatgggcgcaccctgtctgactacaacatccagaaggagtccaccctgcacctggtcctccgcctcagaggtgcc

SEQ ID NO: 43 - protein, 7 aa, Artificial Sequence
  Furin cleavage site
RGRKRRS

SEQ ID NO: 44 - DNA, 21 bp, Artificial Sequence
  Furin cleavage site
agaggaagaaagagaagatca

SEQ ID NO: 45 - protein, 2994 aa, Artificial Sequence
  PLS-ASF fusion protein no. 1''
MQIFVKTLTGKTITLEVEPSDTIENVKGKIQEKEGIPPDQQRLIFAGKQLEDGRTLSDYNIQKESTLHLVLRLRGADFILNISMKMEVIFKTDLRSSSQVVFHAGSLYNWFSVEIINSGRIVTTAIKTLLSTVKYDIVKSARIYAGQGYTEHQAQEEWNMILHVLFEEETESSASSESIHEKNDNETNECTSSFETLFEQEPSSETPKDSKLYMLAQKTVQHIEQYGKAPDFNKVIRAHNFIQTIHGTPLKEEEKEVVRLMVIKLLKKKRGRKRRSDSEFFQPVYPRHYGECLSPVTTPSFFSTHMYTILIAIVVLVIIIIVLIYLFSSRKKKAAAAIEEEDIQFINPYQDQQWAEVTPQPGTSKPAGATTASVGKPVTGRPATNRPATNKPVTDNPVTDRLVMATGGPAAAPAAASAPAHPAEPYTTVTTQNTASQTMSAIENLRQRNTYTHKDLENSLRGRKRRSFSKKKYIGLIDKKCELKKILDDYSILIIGILIGTNIITLIYNFIGWINYIKCYQNDDKMFYCPKDWVGYNNVCYYFSNEEKNYTNASNYCKQLNSTLANNNTNLVNLTKTLNLTKTYNHESNYWVNYSLIKNESVLLRNSGYYKKQKHVSLLYICSKRGRKRRSIILIFLIFSNIVLSIIYWVSFNKTIILDSNITNDNNDINGVSWNTYFNNSFNTLATCGKAGNFCECSNYSTSLYNITNNCSLTIFPHNTDIFNTTYQLVYLNQKINYTIKLLTPVDSPNITYNCTNSLITCKKNNGTNTNIYLNINDTIVNYTNESILNYYWNNSNINNFTATCIINNTISSSNETELINCTNPTLKYQNYFYTFFKLFYIIIFIVSGIIISILFISIITFLSLRKRKKHVEEIESPPPSESNEEEQCQHDDTTSIHEPSPREPLLPKPYSRYQYNTPIYYMRPSTQPLNPFPLPKPCPPPKPCPPPKPCPPPKPCPSAESYSPPKPLPSIPLLPNIPPLSTQNISLIHVDRIIRGRKRRSYHDYASKLLADYRSDPPLWESDLPRHNRYSDNILNSRYCGNKNGAAPVYNEYTNSPEKAEKGLQLSDLRNFSFMLNPQHKNIGYGDAQDLEPYSSIPKNKLFNHFKNHRPAFSTHTENLIRRNVVRTEKKTFPQVASLKGTQKNCLTQPSSLPSLKNPKNSSVPSTRFSEHTKFFSYEDLPKLRTKGTIKHEQHLGDQMPGQHYNGYIPHKDVYNILCLAHNLPASVEKGIAGRGIPLGNPHVKPNIEQELIKSTSTYTDVPMLGPLPPKDSQHGREYQEFSANRHMLQVSNILHSVFANHSIKPQILEDIPVLNAQLTSIKPVSPFLNKAYQTHYMENIVTLVPRFKSIANYSSPIPNYSKRNSGQAEYFDTSKQTISRHNNYIPKYTGGIGDSKLDSTFPKDFNASSVPLTSAEKDHSLRGDNSACCISSISPSLRGRKRRSPSNMKQFCKISVWLQQHDPDLLEIINNLCMLGNLSAAKYKHGVTFIYPKQAKIRDEIKKHAYSNDPSQAIKTLESLILPFYIPTPAEFTGEIGSYTGVKLEVEKTEANKVILKNGEAVLVPAADFKPFPDRRLAVWIMESGSMPLEGPPYKRKKEGGGNDPPVPKHISPYTPRTRIAIEVEKAFDDCMRQNWCSVNNPYLAKSVSLLSFLSLNHPTEFIKVLPLIDFDPLVTFYLLLEPYKTHGDDFLIPETILFGPTGWNGTDLYQSAMLEFKKFFTQITRQTFMDIADSATKEVDVPICYSDPETVHSYANHVRTEILHHNAVNKVTTPNLVVQAYNELEQTNTIRHYGPIFPESTINALRFWKKLWQDEQRFVIHGLHRTLMDQPTYETSEFAEIVRNLRFSRPGNNYINELNITSPAMYGDKHTTGDIAPNDRFAMLVAFINSTDFLYTAIPEEKVGGNETQTSSLTDLVPTRLHSFLNHNLSKLKILNRAQQTVRNILSNDCLNQLKHYVKHTGKNEILKLLQERGRKRRSYFLVADHREHHVIPFLKTDFHHMHQNPIQKKQALLEIKQLFTGDYLICKSPSTILACIERKTYKDFAASLKDGRYKNRQKMLSLREQTNCQLYFFVEGPAFPNPQKKINHVAYASIITAMTHLMVRDHIFVIQTKNEAHSSQKLVQLFYAFSKEMVCVVPTSLTPTDEELCIKLWSSLSGISGVIGKILANTCSVAHLVSGKLSSQNIDQLKTPSNRPFPKKVKRMLISISKGNKELEIKLLSGVPNIGKKLAAEILKDHALLFFLNQPVECLANIQIVQKTRTIKLGMKRAEAIHYFLNWCGSAHVTDDSQNITEASRPTMQVATQSAATQPAATQPLHEVSDDASSDASSPVGHQTLSKEMLLNTARGRKRRSVETQMDKLGFLLNHIGKQVTTKVLSNAHITQTMKEIILENHSVDGGAAKNVSKGKSSPKEKKHWTEFESWEQLSKSKRSFKEYWAERNEIVNTLLLNWDNVRGAIKKFLDDDREWCGRINMINGVPEIVEIIPSPYRAGENIYFGSEAMMPADIYSRVANKPAMFVFHTHPNLGSCCGGMPSICDISTTLRYLLMGWTAGHLIISSNQVGMLTVDKRIIVDLWANENPRWLMAQKILDIFMMLTSRRSLVNPWTLRDLKKILQDYGIEYIIFPSNDFFIYEDERLLMFSKKWTNFFTLHELLDDLETIETKASSTTRGRKRRSSTKKKPTITKQELYSLVAADTQLNKALIERIFTSQQKIIQNALKHNQEVIIPPGIKFTVVTVKAKPARQGHNPATGEPIQIKAKPEHKAVKIRALKPVHDMLNRGRKRRSVEPREQFFQDLLSAVDQQMDTVKNDIKDIMKEKTSFMVSFENFIERYDTMEKNIQDLQNKYEEMAANLMTVMTDTKIQLGAIIAQLEILMINGTPLPAKKTTIKEAMPLPSSNTNNEQTSPPASGKTSETPKKNPTNAMFFTRSEWASSNTFREKFLTPEIQAILDEQFANKTGIERLHAEGLYMWRTQFSDEQKKMVKEMMKK

SEQ ID NO: 46 - protein, 995 aa, Artificial Sequence
  PLS-ASF fusion protein no. 2''
MQIFVKTLTGKTITLEVEPSDTIENVKGKIQEKEGIPPDQQRLIFAGKQLEDGRTLSDYNIQKESTLHLVLRLRGADFILNISMKMEVIFKTDLRSSSQVVFHAGSLYNWFSVEIINSGRIVTTAIKTLLSTVKYDIVKSARIYAGQGYTEHQAQEEWNMILHVLFEEETESSASSESIHEKNDNETNECTSSFETLFEQEPSSETPKDSKLYMLAQKTVQHIEQYGKAPDFNKVIRAHNFIQTIHGTPLKEEEKEVVRLMVIKLLKKKRGRKRRSDSEFFQPVYPRHYGECLSPVTTPSFFSTHMYTILIAIVVLVIIIIVLIYLFSSRKKKAAAAIEEEDIQFINPYQDQQWAEVTPQPGTSKPAGATTASVGKPVTGRPATNRPATNKPVTDNPVTDRLVMATGGPAAAPAAASAPAHPAEPYTTVTTQNTASQTMSAIENLRQRNTYTHKDLENSLRGRKRRSFSKKKYIGLIDKKCELKKILDDYSILIIGILIGTNIITLIYNFIGWINYIKCYQNDDKMFYCPKDWVGYNNVCYYFSNEEKNYTNASNYCKQLNSTLANNNTNLVNLTKTLNLTKTYNHESNYWVNYSLIKNESVLLRNSGYYKKQKHVSLLYICSKRGRKRRSIILIFLIFSNIVLSIIYWVSFNKTIILDSNITNDNNDINGVSWNTYFNNSFNTLATCGKAGNFCECSNYSTSLYNITNNCSLTIFPHNTDIFNTTYQLVYLNQKINYTIKLLTPVDSPNITYNCTNSLITCKKNNGTNTNIYLNINDTIVNYTNESILNYYWNNSNINNFTATCIINNTISSSNETELINCTNPTLKYQNYFYTFFKLFYIIIFIVSGIIISILFISIITFLSLRKRKKHVEEIESPPPSESNEEEQCQHDDTTSIHEPSPREPLLPKPYSRYQYNTPIYYMRPSTQPLNPFPLPKPCPPPKPCPPPKPCPPPKPCPSAESYSPPKPLPSIPLLPNIPPLSTQNISLIHVDRII

SEQ ID NO: 47 - protein, 2068 aa, Artificial Sequence
  PLS-ASF fusion protein no. 3''
MQIFVKTLTGKTITLEVEPSDTIENVKGKIQEKEGIPPDQQRLIFAGKQLEDGRTLSDYNIQKESTLHLVLRLRGAYHDYASKLLADYRSDPPLWESDLPRHNRYSDNILNSRYCGNKNGAAPVYNEYTNSPEKAEKGLQLSDLRNFSFMLNPQHKNIGYGDAQDLEPYSSIPKNKLFNHFKNHRPAFSTHTENLIRRNVVRTEKKTFPQVASLKGTQKNCLTQPSSLPSLKNPKNSSVPSTRFSEHTKFFSYEDLPKLRTKGTIKHEQHLGDQMPGQHYNGYIPHKDVYNILCLAHNLPASVEKGIAGRGIPLGNPHVKPNIEQELIKSTSTYTDVPMLGPLPPKDSQHGREYQEFSANRHMLQVSNILHSVFANHSIKPQILEDIPVLNAQLTSIKPVSPFLNKAYQTHYMENIVTLVPRFKSIANYSSPIPNYSKRNSGQAEYFDTSKQTISRHNNYIPKYTGGIGDSKLDSTFPKDFNASSVPLTSAEKDHSLRGDNSACCISSISPSLRGRKRRSPSNMKQFCKISVWLQQHDPDLLEIINNLCMLGNLSAAKYKHGVTFIYPKQAKIRDEIKKHAYSNDPSQAIKTLESLILPFYIPTPAEFTGEIGSYTGVKLEVEKTEANKVILKNGEAVLVPAADFKPFPDRRLAVWIMESGSMPLEGPPYKRKKEGGGNDPPVPKHISPYTPRTRIAIEVEKAFDDCMRQNWCSVNNPYLAKSVSLLSFLSLNHPTEFIKVLPLIDFDPLVTFYLLLEPYKTHGDDFLIPETILFGPTGWNGTDLYQSAMLEFKKFFTQITRQTFMDIADSATKEVDVPICYSDPETVHSYANHVRTEILHHNAVNKVTTPNLVVQAYNELEQTNTIRHYGPIFPESTINALRFWKKLWQDEQRFVIHGLHRTLMDQPTYETSEFAEIVRNLRFSRPGNNYINELNITSPAMYGDKHTTGDIAPNDRFAMLVAFINSTDFLYTAIPEEKVGGNETQTSSLTDLVPTRLHSFLNHNLSKLKILNRAQQTVRNILSNDCLNQLKHYVKHTGKNEILKLLQERGRKRRSYFLVADHREHHVIPFLKTDFHHMHQNPIQKKQALLEIKQLFTGDYLICKSPSTILACIERKTYKDFAASLKDGRYKNRQKMLSLREQTNCQLYFFVEGPAFPNPQKKINHVAYASIITAMTHLMVRDHIFVIQTKNEAHSSQKLVQLFYAFSKEMVCVVPTSLTPTDEELCIKLWSSLSGISGVIGKILANTCSVAHLVSGKLSSQNIDQLKTPSNRPFPKKVKRMLISISKGNKELEIKLLSGVPNIGKKLAAEILKDHALLFFLNQPVECLANIQIVQKTRTIKLGMKRAEAIHYFLNWCGSAHVTDDSQNITEASRPTMQVATQSAATQPAATQPLHEVSDDASSDASSPVGHQTLSKEMLLNTARGRKRRSVETQMDKLGFLLNHIGKQVTTKVLSNAHITQTMKEIILENHSVDGGAAKNVSKGKSSPKEKKHWTEFESWEQLSKSKRSFKEYWAERNEIVNTLLLNWDNVRGAIKKFLDDDREWCGRINMINGVPEIVEIIPSPYRAGENIYFGSEAMMPADIYSRVANKPAMFVFHTHPNLGSCCGGMPSICDISTTLRYLLMGWTAGHLIISSNQVGMLTVDKRIIVDLWANENPRWLMAQKILDIFMMLTSRRSLVNPWTLRDLKKILQDYGIEYIIFPSNDFFIYEDERLLMFSKKWTNFFTLHELLDDLETIETKASSTTRGRKRRSSTKKKPTITKQELYSLVAADTQLNKALIERIFTSQQKIIQNALKHNQEVIIPPGIKFTVVTVKAKPARQGHNPATGEPIQIKAKPEHKAVKIRALKPVHDMLNRGRKRRSVEPREQFFQDLLSAVDQQMDTVKNDIKDIMKEKTSFMVSFENFIERYDTMEKNIQDLQNKYEEMAANLMTVMTDTKIQLGAIIAQLEILMINGTPLPAKKTTIKEAMPLPSSNTNNEQTSPPASGKTSETPKKNPTNAMFFTRSEWASSNTFREKFLTPEIQAILDEQFANKTGIERLHAEGLYMWRTQFSDEQKKMVKEMMKK

SEQ ID NO: 48 - protein, 1531 aa, Artificial Sequence
  PLS-ASF fusion protein no. 4''
MQIFVKTLTGKTITLEVEPSDTIENVKGKIQEKEGIPPDQQRLIFAGKQLEDGRTLSDYNIQKESTLHLVLRLRGADFILNISMKMEVIFKTDLRSSSQVVFHAGSLYNWFSVEIINSGRIVTTAIKTLLSTVKYDIVKSARIYAGQGYTEHQAQEEWNMILHVLFEEETESSASSESIHEKNDNETNECTSSFETLFEQEPSSETPKDSKLYMLAQKTVQHIEQYGKAPDFNKVIRAHNFIQTIHGTPLKEEEKEVVRLMVIKLLKKKRGRKRRSDSEFFQPVYPRHYGECLSPVTTPSFFSTHMYTILIAIVVLVIIIIVLIYLFSSRKKKAAAAIEEEDIQFINPYQDQQWAEVTPQPGTSKPAGATTASVGKPVTGRPATNRPATNKPVTDNPVTDRLVMATGGPAAAPAAASAPAHPAEPYTTVTTQNTASQTMSAIENLRQRNTYTHKDLENSLRGRKRRSPSNMKQFCKISVWLQQHDPDLLEIINNLCMLGNLSAAKYKHGVTFIYPKQAKIRDEIKKHAYSNDPSQAIKTLESLILPFYIPTPAEFTGEIGSYTGVKLEVEKTEANKVILKNGEAVLVPAADFKPFPDRRLAVWIMESGSMPLEGPPYKRKKEGGGNDPPVPKHISPYTPRTRIAIEVEKAFDDCMRQNWCSVNNPYLAKSVSLLSFLSLNHPTEFIKVLPLIDFDPLVTFYLLLEPYKTHGDDFLIPETILFGPTGWNGTDLYQSAMLEFKKFFTQITRQTFMDIADSATKEVDVPICYSDPETVHSYANHVRTEILHHNAVNKVTTPNLVVQAYNELEQTNTIRHYGPIFPESTINALRFWKKLWQDEQRFVIHGLHRTLMDQPTYETSEFAEIVRNLRFSRPGNNYINELNITSPAMYGDKHTTGDIAPNDRFAMLVAFINSTDFLYTAIPEEKVGGNETQTSSLTDLVPTRLHSFLNHNLSKLKILNRAQQTVRNILSNDCLNQLKHYVKHTGKNEILKLLQERGRKRRSFSKKKYIGLIDKKCELKKILDDYSILIIGILIGTNIITLIYNFIGWINYIKCYQNDDKMFYCPKDWVGYNNVCYYFSNEEKNYTNASNYCKQLNSTLANNNTNLVNLTKTLNLTKTYNHESNYWVNYSLIKNESVLLRNSGYYKKQKHVSLLYICSKRGRKRRSIILIFLIFSNIVLSIIYWVSFNKTIILDSNITNDNNDINGVSWNTYFNNSFNTLATCGKAGNFCECSNYSTSLYNITNNCSLTIFPHNTDIFNTTYQLVYLNQKINYTIKLLTPVDSPNITYNCTNSLITCKKNNGTNTNIYLNINDTIVNYTNESILNYYWNNSNINNFTATCIINNTISSSNETELINCTNPTLKYQNYFYTFFKLFYIIIFIVSGIIISILFISIITFLSLRKRKKHVEEIESPPPSESNEEEQCQHDDTTSIHEPSPREPLLPKPYSRYQYNTPIYYMRPSTQPLNPFPLPKPCPPPKPCPPPKPCPPPKPCPSAESYSPPKPLPSIPLLPNIPPLSTQNISLIHVDRII

SEQ ID NO: 49 - protein, 1532 aa, Artificial Sequence
  PLS-ASF fusion protein no. 5''
MQIFVKTLTGKTITLEVEPSDTIENVKGKIQEKEGIPPDQQRLIFAGKQLEDGRTLSDYNIQKESTLHLVLRLRGAYHDYASKLLADYRSDPPLWESDLPRHNRYSDNILNSRYCGNKNGAAPVYNEYTNSPEKAEKGLQLSDLRNFSFMLNPQHKNIGYGDAQDLEPYSSIPKNKLFNHFKNHRPAFSTHTENLIRRNVVRTEKKTFPQVASLKGTQKNCLTQPSSLPSLKNPKNSSVPSTRFSEHTKFFSYEDLPKLRTKGTIKHEQHLGDQMPGQHYNGYIPHKDVYNILCLAHNLPASVEKGIAGRGIPLGNPHVKPNIEQELIKSTSTYTDVPMLGPLPPKDSQHGREYQEFSANRHMLQVSNILHSVFANHSIKPQILEDIPVLNAQLTSIKPVSPFLNKAYQTHYMENIVTLVPRFKSIANYSSPIPNYSKRNSGQAEYFDTSKQTISRHNNYIPKYTGGIGDSKLDSTFPKDFNASSVPLTSAEKDHSLRGDNSACCISSISPSLRGRKRRSYFLVADHREHHVIPFLKTDFHHMHQNPIQKKQALLEIKQLFTGDYLICKSPSTILACIERKTYKDFAASLKDGRYKNRQKMLSLREQTNCQLYFFVEGPAFPNPQKKINHVAYASIITAMTHLMVRDHIFVIQTKNEAHSSQKLVQLFYAFSKEMVCVVPTSLTPTDEELCIKLWSSLSGISGVIGKILANTCSVAHLVSGKLSSQNIDQLKTPSNRPFPKKVKRMLISISKGNKELEIKLLSGVPNIGKKLAAEILKDHALLFFLNQPVECLANIQIVQKTRTIKLGMKRAEAIHYFLNWCGSAHVTDDSQNITEASRPTMQVATQSAATQPAATQPLHEVSDDASSDASSPVGHQTLSKEMLLNTARGRKRRSVETQMDKLGFLLNHIGKQVTTKVLSNAHITQTMKEIILENHSVDGGAAKNVSKGKSSPKEKKHWTEFESWEQLSKSKRSFKEYWAERNEIVNTLLLNWDNVRGAIKKFLDDDREWCGRINMINGVPEIVEIIPSPYRAGENIYFGSEAMMPADIYSRVANKPAMFVFHTHPNLGSCCGGMPSICDISTTLRYLLMGWTAGHLIISSNQVGMLTVDKRIIVDLWANENPRWLMAQKILDIFMMLTSRRSLVNPWTLRDLKKILQDYGIEYIIFPSNDFFIYEDERLLMFSKKWTNFFTLHELLDDLETIETKASSTTRGRKRRSSTKKKPTITKQELYSLVAADTQLNKALIERIFTSQQKIIQNALKHNQEVIIPPGIKFTVVTVKAKPARQGHNPATGEPIQIKAKPEHKAVKIRALKPVHDMLNRGRKRRSVEPREQFFQDLLSAVDQQMDTVKNDIKDIMKEKTSFMVSFENFIERYDTMEKNIQDLQNKYEEMAANLMTVMTDTKIQLGAIIAQLEILMINGTPLPAKKTTIKEAMPLPSSNTNNEQTSPPASGKTSETPKKNPTNAMFFTRSEWASSNTFREKFLTPEIQAILDEQFANKTGIERLHAEGLYMWRTQFSDEQKKMVKEMMKK

SEQ ID NO: 50 - DNA, 8985 bp, Artificial Sequence
  PLS-ASF fusion protein no. 1''
atgcagatctttgtaaagaccttgactggtaagaccatcaccctggaagtggagcccagtgacaccattgagaatgtcaaggggaagattcaagaaaaagagggcatccccccagaccagcagaggctgatctttgccgggaagcagctggaagatgggcgcaccctgtctgactacaacatccagaaggagtccaccctgcacctggtcctccgcctcagaggtgccgattttattttaaatatatccatgaaaatggaggtcatcttcaaaacggatttaagatcatcttcacaagttgtgtttcatgcgggtagcctgtataattggttttctgttgagattatcaatagcggtagaattgttacgaccgctataaaaacattgcttagtactgttaagtatgatattgtgaaatctgctcgtatatatgcagggcaagggtatactgaacatcaggctcaagaagaatggaatatgattctgcatgtgctgtttgaagaggagacggaatcctcagcatcttcggagtcaattcatgaaaaaaatgataatgaaaccaatgaatgcacatcctcctttgaaacgttgtttgagcaagagccctcatcggagacacctaaagactccaagctgtatatgcttgcacaaaagactgtgcaacatattgaacaatatggaaaggcacctgattttaacaaggttattagagcacataattttattcaaaccattcatggaacccctctaaaggaagaagaaaaagaggtggtaagactcatggttattaaacttttaaaaaaaaaaagaggaagaaagagaagatcagattctgaattttttcaaccggtttatccgcggcattatggtgagtgtttgtcaccagtcactacaccaagcttcttctccacacatatgtatactattctcattgctatcgtggtcttagtcatcattatcatcgttctaatctatctattctcttcaagaaagaaaaaagctgctgctgctattgaggaggaagatatacagtttataaatccttatcaagatcagcagtgggcagaagtcactccacaaccaggtacctctaaaccagctggagcgactacagcaagtgtaggcaagccagtcacgggcagaccggcaacaaacagaccagcaacaaacaaaccagttacggacaacccagttacggacagactagtcatggcaactggcgggccggcggccgcacctgcggccgcgagtgctcctgctcatccggctgagccttacacgacagtcactactcagaacactgcttcacaaacaatgtcggctattgaaaatttacgacaaagaaacacctatacgcataaagacctagaaaactccttgagaggaagaaagagaagatcattttctaagaaaaagtacatcggtcttatcgataagaagtgtgaattgaaaaaaatactagatgattatagtatattaataattggaatattaattggaactaacatcataacccttatttataattttataggatggattaattatataaaatgttaccaaaatgatgataagatgttttattgccctaaagattgggttggatataataatgtttgttattattttagtaatgaagaaaaaaattatactaatgcaagtaattattgtaagcaattaaatagtacgcttgctaataataatactaatttagtaaatcttactaaaacattaaatcttactaaaacatataatcacgaatctaattattgggttaattattctttaattaaaaatgagtcagtactattacgtaatagtggatattacaaaaaacaaaaacatgtaagtttattatatatttgtagtaaaagaggaagaaagagaagatcaataatacttatttttttaatattttctaacatagttttaagtattatatattgggttagttttaataaaacaataattttagatagtaatattactaatgataataatgatataaatggagtatcatggaatacttattttaataattcttttaatacactagctacatgtggaaaagcaggtaacttttgtgaatgttctaattatagtacatcactatataatataacaaataattgtagcttaactatttttcctcataatactgatatatttaatacaacatatcaactagtatatctaaatcaaaaaattaattatacaataaaattattaacacctgtagattctccaaatatcacatataattgtactaattctttaataacatgtaaaaaaaataatggaacaaacactaatatatatttaaatataaatgatactatagttaattatactaatgaaagtatacttaattattattggaataatagtaacattaacaattttacagctacatgtataattaataatacaattagttcttctaatgaaacagaacttataaattgtactaatcccacattgaaatatcaaaactatttttatactttttttaaattattttatattataatatttatcgtatctgggataataataagtattctttttatatccatcataacttttttatctttacgaaaaagaaaaaaacatgttgaagaaatagaaagtccaccaccttctgaatctaatgaagaagaacaatgtcagcatgatgacaccacttccatacatgaaccatctcccagagaaccattacttcctaagccttacagtcgttatcagtataatacacctatttactacatgcgtccctcaacacaaccactcaacccatttcccttacctaaaccgtgtcctccacccaaaccatgtccgccacccaaaccatgtcctccacctaaaccatgtccttcagctgaatcctattctccacccaaaccactacctagtatcccgctactacccaatatcccgccattatctacccaaaatatttcgcttattcacgtagatagaattattagaggaagaaagagaagatcatatcatgattatgcttcaaagctgttagccgattataggtcagatccacctctttgggaaagcgatttgccgcgtcataaccggtattctgataatatactaaattcccggtactgcggcaacaaaaatggagctgcgcctgtatacaatgaatacactaatagtcctgaaaaggctgaaaagggattgcaactcagtgatctacgtaacttttcttttatgctgaaccctcagcacaaaaacattggttacggcgatgcgcaagatctggagccgtacagctccattccaaaaaataaactttttaatcattttaaaaatcatcgtcctgctttttcaacccatacggaaaacctaattaggcgcaatgttgttcgtacggaaaaaaaaacatttccgcaggtggctagcttaaagggcacacagaaaaattgtctgacccagccttcctcattgccttccttaaaaaacccaaaaaatagttcggttccttctacgaggttcagcgagcacacaaaatttttttcgtacgaggatcttcctaaactcagaacaaagggtaccattaagcatgagcagcaccttggcgatcagatgccgggccagcactataacggatatattccgcacaaagacgtgtacaatattttgtgtttagcgcacaatctacctgcgtcggtagaaaaagggattgcaggtagaggtattcctttaggaaatccacatgtcaaaccgaacatagagcaggaactcataaaatccaccagtacctacacggacgtgccgatgcttggtccccttccgcccaaagattcgcaacacggcagagaataccaggaattttccgcaaatagacatatgctacaagtatctaatatactacattctgtgtttgctaatcattctataaagccacaaatcctagaagacataccggtactcaatgcacaactaacaagcataaagccggtaagcccatttttaaacaaagcgtatcaaacccattatatggaaaatattgttaccttggtgccccggtttaagagtattgccaactactcaagccctataccgaattattctaaaagaaatagcggtcaggctgaatattttgatacctcaaagcaaacaatttctagacacaataattatatacctaaatatacgggaggaattggagattccaaactagacagcacctttcctaaagatttcaacgcctcctcggtaccgttaacaagcgcggaaaaggaccattccctgcggggagacaactcagcatgttgcatctcatctatatctccatcattgagaggaagaaagagaagatcaccctctaatatgaaacagttttgcaagatttctgtatggctacagcagcacgatccagatttattagaaattatcaacaacttatgtatgcttggcaatttatccgcggcaaagtacaaacacggagttaccttcatttaccccaaacaggcaaagatccgcgatgaaataaaaaaacatgcctactccaatgacccttcacaagccataaagaccttagaatcactcatccttccattttacattcccactccagcggagttcaccggggaaatcggctcctacaccggagtgaaattagaggttgaaaaaacggaggcgaataaagttattttaaaaaatggagaagcggtcctagtaccggcggccgattttaagccctttcctgatcgccgactagcggtctggatcatggagtcaggctctatgcccctggagggtcccccctataagcggaaaaaggagggtggggggaatgacccgccggttcctaagcatatctcgccgtatactccgcgcacgcgtattgccattgaggtggaaaaggcctttgatgactgtatgcgtcaaaactggtgtagtgtcaataatccctatcttgccaagtcggtctccttgctgtctttcttgtcgctcaaccatcccaccgagtttattaaggtactgccgcttatagactttgaccccttggtgaccttttatctacttcttgagccctataaaacgcatggggatgactttttaattccggaaaccattttattcggccctaccggatggaatggtacagatctgtatcaaagtgccatgctggagtttaaaaagttttttacccagattactcgccaaacctttatggacatagccgattcggctactaaggaggtagatgttcccatatgttactcggatcccgaaaccgtacattcctatgccaatcacgtgcgtactgaaattttgcatcacaatgccgtcaataaggttacaacacctaacctcgtcgtgcaggcctataatgagctcgagcaaaccaataccatacgacattacggccctattttcccggaaagtaccatcaacgcactgcgtttttggaaaaagctgtggcaggatgaacagcgatttgttatccacggcctgcaccgcacgttgatggatcaacccacctatgaaacctctgagtttgcagagatcgttagaaatttacggttttcgcgtcccggcaataactatataaacgagcttaatattacaagtcccgctatgtacggcgacaagcataccaccggagatattgcgcccaatgatagatttgccatgttggtggcctttatcaacagtactgactttttatacaccgcgattcccgaggaaaaggtaggggggaatgaaacccaaaccagtagccttacagacctagttccaacacggctacactcttttttaaatcataatctaagcaaacttaaaatcttaaaccgcgcgcagcaaacggttagaaatattctttcaaatgattgtcttaatcaactgaaacattatgttaaacacacgggaaaaaatgaaatactaaagttacttcaagaaagaggaagaaagagaagatcatattttctagtagcagatcatcgagaacatcatgtgattccttttcttaaaaccgatttccatcacatgcatcaaaatcctatacaaaaaaaacaagctctcctagaaatcaaacagctttttactggagattatctcatctgcaaaagcccttctaccattctggcctgtattgaacgaaaaacctacaaagactttgcggcttctttgaaagatggacgttataaaaatcgccaaaaaatgctgtcgctgcgagaacaaaccaactgtcaactttatttttttgtagaaggcccggcatttcctaaccctcaaaaaaaaattaatcacgttgcctatgcaagcattattactgctatgacgcatcttatggttagagatcatatttttgtcattcaaacgaaaaatgaggcccacagttcccaaaagcttgtgcagcttttttatgccttttctaaggaaatggtgtgcgtcgttcccacctccctcacccccacggatgaagagctatgcatcaagctatggtcttctctttctggtatttcaggcgtgataggtaaaatcttggcaaacacttgttccgtagctcatttggtttctggaaagctttcatcgcagaatattgatcagttaaaaactccctccaaccgaccattccccaaaaaagtaaaacgtatgcttataagcattagcaaaggaaataaggagttagaaataaaattgctctcgggggttcccaatatcgggaaaaaattagctgccgaaattttaaaagatcatgcgcttcttttttttctaaatcagcccgtagaatgcttggcaaatatacaaatcgttcaaaaaacccgtacgattaagttgggaatgaagcgagccgaagcgattcattattttttaaactggtgtggctctgcccatgtaaccgatgatagccaaaatatcacagaggcgtcgcggcctacaatgcaggtcgcgacgcagtccgccgcaactcagcccgctgcaacgcagccattgcacgaagtatcagatgatgcatcatcagatgcttcatcacccgtagggcatcaaacattatctaaagaaatgttattgaacacagccagaggaagaaagagaagatcagttgagacacaaatggacaaacttggttttctgctaaatcacataggtaaacaggttaccactaaggtgcttagcaatgcccatataactcaaacgatgaaggagattattttggaaaatcatagtgtagatggtggagccgcaaaaaatgtttcaaaagggaagtcttccccaaaagaaaaaaaacattggactgagttcgaatcctgggaacagctcagcaagtctaaaagaagttttaaggaatactgggcggagcgtaatgagattgtgaatactctgttgcttaactgggacaatgttcggggtgccatcaaaaaatttttggacgatgaccgtgaatggtgcggccgcattaatatgataaacggtgtacccgagatagtggaaatcattccaagcccctatagggcaggagagaacatttattttggcagcgaggctatgatgcctgctgatatttatagcagggtggccaacaagcctgctatgtttgtgtttcacacgcatcctaatttgggttcatgttgtggaggaatgccttccatatgtgacatttctacaacgctgcgttatctactcatggggtggactgctgggcatctaatcatttcttcgaatcaagtaggaatgctcacggttgataagagaattattgttgatttgtgggccaatgagaatccgcgctggcttatggcgcaaaaaatattagatatttttatgatgctcacttcgcgtagaagcctggtaaatccctggaccctgagagacctaaaaaaaatattacaagactatggtattgagtatatcatttttccttcgaatgacttttttatttatgaagacgaacgtcttttaatgttttcaaaaaaatggaccaacttttttacgttacatgagttattggatgacctcgaaactattgagacaaaggcatcgtccacaacaagaggaagaaagagaagatcatcgacaaaaaaaaagcccacaattaccaagcaagagctttactccttagtagcggcagatacccagttaaataaagcattgattgaaagaatctttacaagtcagcaaaaaataatacaaaatgctttaaagcacaatcaagaagttattataccacccggaatcaagttcaccgtcgttacggtgaaagctaaacctgctcgccagggccataatcccgccacaggagagcctattcaaattaaagctaaacctgaacataaagccgtaaagatacgagcattgaaacctgtccatgatatgttaaacagaggaagaaagagaagatcagttgagccacgcgaacagttttttcaagatctgctttcagcagtggatcaacaaatggacactgtaaaaaatgacataaaagacattatgaaagaaaaaacgtcttttatggtatcattcgaaaactttatagaacgttacgataccatggaaaaaaatattcaagaccttcagaataagtacgaagaaatggcggccaaccttatgaccgtcatgacggatacaaaaattcagcttggagccattatcgcccaacttgagattctaatgataaatggcactccacttccggcaaaaaagacaacaattaaggaggctatgcccttaccttcatcaaacacgaataatgaacaaacgagtcctcccgcctcaggcaaaacaagtgaaacacctaaaaaaaatcccacgaatgcgatgttcttcacgcgtagcgaatgggcatcctcgaatacttttcgagaaaagtttttaacaccagaaattcaagccatattggatgagcagtttgcaaacaagaccgggatcgaaagattgcatgccgagggtctttacatgtggagaacccaattctctgacgaacagaagaaaatggtcaaagagatgatgaagaagtaa

SEQ ID NO: 51 - DNA, 2988 bp, Artificial Sequence
  PLS-ASF fusion protein no. 2''
atgcagatctttgtaaagaccttgactggtaagaccatcaccctggaagtggagcccagtgacaccattgagaatgtcaaggggaagattcaagaaaaagagggcatccccccagaccagcagaggctgatctttgccgggaagcagctggaagatgggcgcaccctgtctgactacaacatccagaaggagtccaccctgcacctggtcctccgcctcagaggtgccgattttattttaaatatatccatgaaaatggaggtcatcttcaaaacggatttaagatcatcttcacaagttgtgtttcatgcgggtagcctgtataattggttttctgttgagattatcaatagcggtagaattgttacgaccgctataaaaacattgcttagtactgttaagtatgatattgtgaaatctgctcgtatatatgcagggcaagggtatactgaacatcaggctcaagaagaatggaatatgattctgcatgtgctgtttgaagaggagacggaatcctcagcatcttcggagtcaattcatgaaaaaaatgataatgaaaccaatgaatgcacatcctcctttgaaacgttgtttgagcaagagccctcatcggagacacctaaagactccaagctgtatatgcttgcacaaaagactgtgcaacatattgaacaatatggaaaggcacctgattttaacaaggttattagagcacataattttattcaaaccattcatggaacccctctaaaggaagaagaaaaagaggtggtaagactcatggttattaaacttttaaaaaaaaaaagaggaagaaagagaagatcagattctgaattttttcaaccggtttatccgcggcattatggtgagtgtttgtcaccagtcactacaccaagcttcttctccacacatatgtatactattctcattgctatcgtggtcttagtcatcattatcatcgttctaatctatctattctcttcaagaaagaaaaaagctgctgctgctattgaggaggaagatatacagtttataaatccttatcaagatcagcagtgggcagaagtcactccacaaccaggtacctctaaaccagctggagcgactacagcaagtgtaggcaagccagtcacgggcagaccggcaacaaacagaccagcaacaaacaaaccagttacggacaacccagttacggacagactagtcatggcaactggcgggccggcggccgcacctgcggccgcgagtgctcctgctcatccggctgagccttacacgacagtcactactcagaacactgcttcacaaacaatgtcggctattgaaaatttacgacaaagaaacacctatacgcataaagacctagaaaactccttgagaggaagaaagagaagatcattttctaagaaaaagtacatcggtcttatcgataagaagtgtgaattgaaaaaaatactagatgattatagtatattaataattggaatattaattggaactaacatcataacccttatttataattttataggatggattaattatataaaatgttaccaaaatgatgataagatgttttattgccctaaagattgggttggatataataatgtttgttattattttagtaatgaagaaaaaaattatactaatgcaagtaattattgtaagcaattaaatagtacgcttgctaataataatactaatttagtaaatcttactaaaacattaaatcttactaaaacatataatcacgaatctaattattgggttaattattctttaattaaaaatgagtcagtactattacgtaatagtggatattacaaaaaacaaaaacatgtaagtttattatatatttgtagtaaaagaggaagaaagagaagatcaataatacttatttttttaatattttctaacatagttttaagtattatatattgggttagttttaataaaacaataattttagatagtaatattactaatgataataatgatataaatggagtatcatggaatacttattttaataattcttttaatacactagctacatgtggaaaagcaggtaacttttgtgaatgttctaattatagtacatcactatataatataacaaataattgtagcttaactatttttcctcataatactgatatatttaatacaacatatcaactagtatatctaaatcaaaaaattaattatacaataaaattattaacacctgtagattctccaaatatcacatataattgtactaattctttaataacatgtaaaaaaaataatggaacaaacactaatatatatttaaatataaatgatactatagttaattatactaatgaaagtatacttaattattattggaataatagtaacattaacaattttacagctacatgtataattaataatacaattagttcttctaatgaaacagaacttataaattgtactaatcccacattgaaatatcaaaactatttttatactttttttaaattattttatattataatatttatcgtatctgggataataataagtattctttttatatccatcataacttttttatctttacgaaaaagaaaaaaacatgttgaagaaatagaaagtccaccaccttctgaatctaatgaagaagaacaatgtcagcatgatgacaccacttccatacatgaaccatctcccagagaaccattacttcctaagccttacagtcgttatcagtataatacacctatttactacatgcgtccctcaacacaaccactcaacccatttcccttacctaaaccgtgtcctccacccaaaccatgtccgccacccaaaccatgtcctccacctaaaccatgtccttcagctgaatcctattctccacccaaaccactacctagtatcccgctactacccaatatcccgccattatctacccaaaatatttcgcttattcacgtagatagaattatttaa

SEQ ID NO: 52 - DNA, 6207 bp, Artificial Sequence
  PLS-ASF fusion protein no. 3''
atgcagatctttgtaaagaccttgactggtaagaccatcaccctggaagtggagcccagtgacaccattgagaatgtcaaggggaagattcaagaaaaagagggcatccccccagaccagcagaggctgatctttgccgggaagcagctggaagatgggcgcaccctgtctgactacaacatccagaaggagtccaccctgcacctggtcctccgcctcagaggtgcctatcatgattatgcttcaaagctgttagccgattataggtcagatccacctctttgggaaagcgatttgccgcgtcataaccggtattctgataatatactaaattcccggtactgcggcaacaaaaatggagctgcgcctgtatacaatgaatacactaatagtcctgaaaaggctgaaaagggattgcaactcagtgatctacgtaacttttcttttatgctgaaccctcagcacaaaaacattggttacggcgatgcgcaagatctggagccgtacagctccattccaaaaaataaactttttaatcattttaaaaatcatcgtcctgctttttcaacccatacggaaaacctaattaggcgcaatgttgttcgtacggaaaaaaaaacatttccgcaggtggctagcttaaagggcacacagaaaaattgtctgacccagccttcctcattgccttccttaaaaaacccaaaaaatagttcggttccttctacgaggttcagcgagcacacaaaatttttttcgtacgaggatcttcctaaactcagaacaaagggtaccattaagcatgagcagcaccttggcgatcagatgccgggccagcactataacggatatattccgcacaaagacgtgtacaatattttgtgtttagcgcacaatctacctgcgtcggtagaaaaagggattgcaggtagaggtattcctttaggaaatccacatgtcaaaccgaacatagagcaggaactcataaaatccaccagtacctacacggacgtgccgatgcttggtccccttccgcccaaagattcgcaacacggcagagaataccaggaattttccgcaaatagacatatgctacaagtatctaatatactacattctgtgtttgctaatcattctataaagccacaaatcctagaagacataccggtactcaatgcacaactaacaagcataaagccggtaagcccatttttaaacaaagcgtatcaaacccattatatggaaaatattgttaccttggtgccccggtttaagagtattgccaactactcaagccctataccgaattattctaaaagaaatagcggtcaggctgaatattttgatacctcaaagcaaacaatttctagacacaataattatatacctaaatatacgggaggaattggagattccaaactagacagcacctttcctaaagatttcaacgcctcctcggtaccgttaacaagcgcggaaaaggaccattccctgcggggagacaactcagcatgttgcatctcatctatatctccatcattgagaggaagaaagagaagatcaccctctaatatgaaacagttttgcaagatttctgtatggctacagcagcacgatccagatttattagaaattatcaacaacttatgtatgcttggcaatttatccgcggcaaagtacaaacacggagttaccttcatttaccccaaacaggcaaagatccgcgatgaaataaaaaaacatgcctactccaatgacccttcacaagccataaagaccttagaatcactcatccttccattttacattcccactccagcggagttcaccggggaaatcggctcctacaccggagtgaaattagaggttgaaaaaacggaggcgaataaagttattttaaaaaatggagaagcggtcctagtaccggcggccgattttaagccctttcctgatcgccgactagcggtctggatcatggagtcaggctctatgcccctggagggtcccccctataagcggaaaaaggagggtggggggaatgacccgccggttcctaagcatatctcgccgtatactccgcgcacgcgtattgccattgaggtggaaaaggcctttgatgactgtatgcgtcaaaactggtgtagtgtcaataatccctatcttgccaagtcggtctccttgctgtctttcttgtcgctcaaccatcccaccgagtttattaaggtactgccgcttatagactttgaccccttggtgaccttttatctacttcttgagccctataaaacgcatggggatgactttttaattccggaaaccattttattcggccctaccggatggaatggtacagatctgtatcaaagtgccatgctggagtttaaaaagttttttacccagattactcgccaaacctttatggacatagccgattcggctactaaggaggtagatgttcccatatgttactcggatcccgaaaccgtacattcctatgccaatcacgtgcgtactgaaattttgcatcacaatgccgtcaataaggttacaacacctaacctcgtcgtgcaggcctataatgagctcgagcaaaccaataccatacgacattacggccctattttcccggaaagtaccatcaacgcactgcgtttttggaaaaagctgtggcaggatgaacagcgatttgttatccacggcctgcaccgcacgttgatggatcaacccacctatgaaacctctgagtttgcagagatcgttagaaatttacggttttcgcgtcccggcaataactatataaacgagcttaatattacaagtcccgctatgtacggcgacaagcataccaccggagatattgcgcccaatgatagatttgccatgttggtggcctttatcaacagtactgactttttatacaccgcgattcccgaggaaaaggtaggggggaatgaaacccaaaccagtagccttacagacctagttccaacacggctacactcttttttaaatcataatctaagcaaacttaaaatcttaaaccgcgcgcagcaaacggttagaaatattctttcaaatgattgtcttaatcaactgaaacattatgttaaacacacgggaaaaaatgaaatactaaagttacttcaagaaagaggaagaaagagaagatcatattttctagtagcagatcatcgagaacatcatgtgattccttttcttaaaaccgatttccatcacatgcatcaaaatcctatacaaaaaaaacaagctctcctagaaatcaaacagctttttactggagattatctcatctgcaaaagcccttctaccattctggcctgtattgaacgaaaaacctacaaagactttgcggcttctttgaaagatggacgttataaaaatcgccaaaaaatgctgtcgctgcgagaacaaaccaactgtcaactttatttttttgtagaaggcccggcatttcctaaccctcaaaaaaaaattaatcacgttgcctatgcaagcattattactgctatgacgcatcttatggttagagatcatatttttgtcattcaaacgaaaaatgaggcccacagttcccaaaagcttgtgcagcttttttatgccttttctaaggaaatggtgtgcgtcgttcccacctccctcacccccacggatgaagagctatgcatcaagctatggtcttctctttctggtatttcaggcgtgataggtaaaatcttggcaaacacttgttccgtagctcatttggtttctggaaagctttcatcgcagaatattgatcagttaaaaactccctccaaccgaccattccccaaaaaagtaaaacgtatgcttataagcattagcaaaggaaataaggagttagaaataaaattgctctcgggggttcccaatatcgggaaaaaattagctgccgaaattttaaaagatcatgcgcttcttttttttctaaatcagcccgtagaatgcttggcaaatatacaaatcgttcaaaaaacccgtacgattaagttgggaatgaagcgagccgaagcgattcattattttttaaactggtgtggctctgcccatgtaaccgatgatagccaaaatatcacagaggcgtcgcggcctacaatgcaggtcgcgacgcagtccgccgcaactcagcccgctgcaacgcagccattgcacgaagtatcagatgatgcatcatcagatgcttcatcacccgtagggcatcaaacattatctaaagaaatgttattgaacacagccagaggaagaaagagaagatcagttgagacacaaatggacaaacttggttttctgctaaatcacataggtaaacaggttaccactaaggtgcttagcaatgcccatataactcaaacgatgaaggagattattttggaaaatcatagtgtagatggtggagccgcaaaaaatgtttcaaaagggaagtcttccccaaaagaaaaaaaacattggactgagttcgaatcctgggaacagctcagcaagtctaaaagaagttttaaggaatactgggcggagcgtaatgagattgtgaatactctgttgcttaactgggacaatgttcggggtgccatcaaaaaatttttggacgatgaccgtgaatggtgcggccgcattaatatgataaacggtgtacccgagatagtggaaatcattccaagcccctatagggcaggagagaacatttattttggcagcgaggctatgatgcctgctgatatttatagcagggtggccaacaagcctgctatgtttgtgtttcacacgcatcctaatttgggttcatgttgtggaggaatgccttccatatgtgacatttctacaacgctgcgttatctactcatggggtggactgctgggcatctaatcatttcttcgaatcaagtaggaatgctcacggttgataagagaattattgttgatttgtgggccaatgagaatccgcgctggcttatggcgcaaaaaatattagatatttttatgatgctcacttcgcgtagaagcctggtaaatccctggaccctgagagacctaaaaaaaatattacaagactatggtattgagtatatcatttttccttcgaatgacttttttatttatgaagacgaacgtcttttaatgttttcaaaaaaatggaccaacttttttacgttacatgagttattggatgacctcgaaactattgagacaaaggcatcgtccacaacaagaggaagaaagagaagatcatcgacaaaaaaaaagcccacaattaccaagcaagagctttactccttagtagcggcagatacccagttaaataaagcattgattgaaagaatctttacaagtcagcaaaaaataatacaaaatgctttaaagcacaatcaagaagttattataccacccggaatcaagttcaccgtcgttacggtgaaagctaaacctgctcgccagggccataatcccgccacaggagagcctattcaaattaaagctaaacctgaacataaagccgtaaagatacgagcattgaaacctgtccatgatatgttaaacagaggaagaaagagaagatcagttgagccacgcgaacagttttttcaagatctgctttcagcagtggatcaacaaatggacactgtaaaaaatgacataaaagacattatgaaagaaaaaacgtcttttatggtatcattcgaaaactttatagaacgttacgataccatggaaaaaaatattcaagaccttcagaataagtacgaagaaatggcggccaaccttatgaccgtcatgacggatacaaaaattcagcttggagccattatcgcccaacttgagattctaatgataaatggcactccacttccggcaaaaaagacaacaattaaggaggctatgcccttaccttcatcaaacacgaataatgaacaaacgagtcctcccgcctcaggcaaaacaagtgaaacacctaaaaaaaatcccacgaatgcgatgttcttcacgcgtagcgaatgggcatcctcgaatacttttcgagaaaagtttttaacaccagaaattcaagccatattggatgagcagtttgcaaacaagaccgggatcgaaagattgcatgccgagggtctttacatgtggagaacccaattctctgacgaacagaagaaaatggtcaaagagatgatgaagaagtaa

SEQ ID NO: 53 - DNA, 4596 bp, Artificial Sequence
  PLS-ASF fusion protein no. 4''
atgcagatctttgtaaagaccttgactggtaagaccatcaccctggaagtggagcccagtgacaccattgagaatgtcaaggggaagattcaagaaaaagagggcatccccccagaccagcagaggctgatctttgccgggaagcagctggaagatgggcgcaccctgtctgactacaacatccagaaggagtccaccctgcacctggtcctccgcctcagaggtgccgattttattttaaatatatccatgaaaatggaggtcatcttcaaaacggatttaagatcatcttcacaagttgtgtttcatgcgggtagcctgtataattggttttctgttgagattatcaatagcggtagaattgttacgaccgctataaaaacattgcttagtactgttaagtatgatattgtgaaatctgctcgtatatatgcagggcaagggtatactgaacatcaggctcaagaagaatggaatatgattctgcatgtgctgtttgaagaggagacggaatcctcagcatcttcggagtcaattcatgaaaaaaatgataatgaaaccaatgaatgcacatcctcctttgaaacgttgtttgagcaagagccctcatcggagacacctaaagactccaagctgtatatgcttgcacaaaagactgtgcaacatattgaacaatatggaaaggcacctgattttaacaaggttattagagcacataattttattcaaaccattcatggaacccctctaaaggaagaagaaaaagaggtggtaagactcatggttattaaacttttaaaaaaaaaaagaggaagaaagagaagatcagattctgaattttttcaaccggtttatccgcggcattatggtgagtgtttgtcaccagtcactacaccaagcttcttctccacacatatgtatactattctcattgctatcgtggtcttagtcatcattatcatcgttctaatctatctattctcttcaagaaagaaaaaagctgctgctgctattgaggaggaagatatacagtttataaatccttatcaagatcagcagtgggcagaagtcactccacaaccaggtacctctaaaccagctggagcgactacagcaagtgtaggcaagccagtcacgggcagaccggcaacaaacagaccagcaacaaacaaaccagttacggacaacccagttacggacagactagtcatggcaactggcgggccggcggccgcacctgcggccgcgagtgctcctgctcatccggctgagccttacacgacagtcactactcagaacactgcttcacaaacaatgtcggctattgaaaatttacgacaaagaaacacctatacgcataaagacctagaaaactccttgagaggaagaaagagaagatcaccctctaatatgaaacagttttgcaagatttctgtatggctacagcagcacgatccagatttattagaaattatcaacaacttatgtatgcttggcaatttatccgcggcaaagtacaaacacggagttaccttcatttaccccaaacaggcaaagatccgcgatgaaataaaaaaacatgcctactccaatgacccttcacaagccataaagaccttagaatcactcatccttccattttacattcccactccagcggagttcaccggggaaatcggctcctacaccggagtgaaattagaggttgaaaaaacggaggcgaataaagttattttaaaaaatggagaagcggtcctagtaccggcggccgattttaagccctttcctgatcgccgactagcggtctggatcatggagtcaggctctatgcccctggagggtcccccctataagcggaaaaaggagggtggggggaatgacccgccggttcctaagcatatctcgccgtatactccgcgcacgcgtattgccattgaggtggaaaaggcctttgatgactgtatgcgtcaaaactggtgtagtgtcaataatccctatcttgccaagtcggtctccttgctgtctttcttgtcgctcaaccatcccaccgagtttattaaggtactgccgcttatagactttgaccccttggtgaccttttatctacttcttgagccctataaaacgcatggggatgactttttaattccggaaaccattttattcggccctaccggatggaatggtacagatctgtatcaaagtgccatgctggagtttaaaaagttttttacccagattactcgccaaacctttatggacatagccgattcggctactaaggaggtagatgttcccatatgttactcggatcccgaaaccgtacattcctatgccaatcacgtgcgtactgaaattttgcatcacaatgccgtcaataaggttacaacacctaacctcgtcgtgcaggcctataatgagctcgagcaaaccaataccatacgacattacggccctattttcccggaaagtaccatcaacgcactgcgtttttggaaaaagctgtggcaggatgaacagcgatttgttatccacggcctgcaccgcacgttgatggatcaacccacctatgaaacctctgagtttgcagagatcgttagaaatttacggttttcgcgtcccggcaataactatataaacgagcttaatattacaagtcccgctatgtacggcgacaagcataccaccggagatattgcgcccaatgatagatttgccatgttggtggcctttatcaacagtactgactttttatacaccgcgattcccgaggaaaaggtaggggggaatgaaacccaaaccagtagccttacagacctagttccaacacggctacactcttttttaaatcataatctaagcaaacttaaaatcttaaaccgcgcgcagcaaacggttagaaatattctttcaaatgattgtcttaatcaactgaaacattatgttaaacacacgggaaaaaatgaaatactaaagttacttcaagaaagaggaagaaagagaagatcattttctaagaaaaagtacatcggtcttatcgataagaagtgtgaattgaaaaaaatactagatgattatagtatattaataattggaatattaattggaactaacatcataacccttatttataattttataggatggattaattatataaaatgttaccaaaatgatgataagatgttttattgccctaaagattgggttggatataataatgtttgttattattttagtaatgaagaaaaaaattatactaatgcaagtaattattgtaagcaattaaatagtacgcttgctaataataatactaatttagtaaatcttactaaaacattaaatcttactaaaacatataatcacgaatctaattattgggttaattattctttaattaaaaatgagtcagtactattacgtaatagtggatattacaaaaaacaaaaacatgtaagtttattatatatttgtagtaaaagaggaagaaagagaagatcaataatacttatttttttaatattttctaacatagttttaagtattatatattgggttagttttaataaaacaataattttagatagtaatattactaatgataataatgatataaatggagtatcatggaatacttattttaataattcttttaatacactagctacatgtggaaaagcaggtaacttttgtgaatgttctaattatagtacatcactatataatataacaaataattgtagcttaactatttttcctcataatactgatatatttaatacaacatatcaactagtatatctaaatcaaaaaattaattatacaataaaattattaacacctgtagattctccaaatatcacatataattgtactaattctttaataacatgtaaaaaaaataatggaacaaacactaatatatatttaaatataaatgatactatagttaattatactaatgaaagtatacttaattattattggaataatagtaacattaacaattttacagctacatgtataattaataatacaattagttcttctaatgaaacagaacttataaattgtactaatcccacattgaaatatcaaaactatttttatactttttttaaattattttatattataatatttatcgtatctgggataataataagtattctttttatatccatcataacttttttatctttacgaaaaagaaaaaaacatgttgaagaaatagaaagtccaccaccttctgaatctaatgaagaagaacaatgtcagcatgatgacaccacttccatacatgaaccatctcccagagaaccattacttcctaagccttacagtcgttatcagtataatacacctatttactacatgcgtccctcaacacaaccactcaacccatttcccttacctaaaccgtgtcctccacccaaaccatgtccgccacccaaaccatgtcctccacctaaaccatgtccttcagctgaatcctattctccacccaaaccactacctagtatcccgctactacccaatatcccgccattatctacccaaaatatttcgcttattcacgtagatagaattatttaa

SEQ ID NO: 54 - DNA, 4599 bp, Artificial Sequence
  PLS-ASF fusion protein no. 5''
atgcagatctttgtaaagaccttgactggtaagaccatcaccctggaagtggagcccagtgacaccattgagaatgtcaaggggaagattcaagaaaaagagggcatccccccagaccagcagaggctgatctttgccgggaagcagctggaagatgggcgcaccctgtctgactacaacatccagaaggagtccaccctgcacctggtcctccgcctcagaggtgcctatcatgattatgcttcaaagctgttagccgattataggtcagatccacctctttgggaaagcgatttgccgcgtcataaccggtattctgataatatactaaattcccggtactgcggcaacaaaaatggagctgcgcctgtatacaatgaatacactaatagtcctgaaaaggctgaaaagggattgcaactcagtgatctacgtaacttttcttttatgctgaaccctcagcacaaaaacattggttacggcgatgcgcaagatctggagccgtacagctccattccaaaaaataaactttttaatcattttaaaaatcatcgtcctgctttttcaacccatacggaaaacctaattaggcgcaatgttgttcgtacggaaaaaaaaacatttccgcaggtggctagcttaaagggcacacagaaaaattgtctgacccagccttcctcattgccttccttaaaaaacccaaaaaatagttcggttccttctacgaggttcagcgagcacacaaaatttttttcgtacgaggatcttcctaaactcagaacaaagggtaccattaagcatgagcagcaccttggcgatcagatgccgggccagcactataacggatatattccgcacaaagacgtgtacaatattttgtgtttagcgcacaatctacctgcgtcggtagaaaaagggattgcaggtagaggtattcctttaggaaatccacatgtcaaaccgaacatagagcaggaactcataaaatccaccagtacctacacggacgtgccgatgcttggtccccttccgcccaaagattcgcaacacggcagagaataccaggaattttccgcaaatagacatatgctacaagtatctaatatactacattctgtgtttgctaatcattctataaagccacaaatcctagaagacataccggtactcaatgcacaactaacaagcataaagccggtaagcccatttttaaacaaagcgtatcaaacccattatatggaaaatattgttaccttggtgccccggtttaagagtattgccaactactcaagccctataccgaattattctaaaagaaatagcggtcaggctgaatattttgatacctcaaagcaaacaatttctagacacaataattatatacctaaatatacgggaggaattggagattccaaactagacagcacctttcctaaagatttcaacgcctcctcggtaccgttaacaagcgcggaaaaggaccattccctgcggggagacaactcagcatgttgcatctcatctatatctccatcattgagaggaagaaagagaagatcatattttctagtagcagatcatcgagaacatcatgtgattccttttcttaaaaccgatttccatcacatgcatcaaaatcctatacaaaaaaaacaagctctcctagaaatcaaacagctttttactggagattatctcatctgcaaaagcccttctaccattctggcctgtattgaacgaaaaacctacaaagactttgcggcttctttgaaagatggacgttataaaaatcgccaaaaaatgctgtcgctgcgagaacaaaccaactgtcaactttatttttttgtagaaggcccggcatttcctaaccctcaaaaaaaaattaatcacgttgcctatgcaagcattattactgctatgacgcatcttatggttagagatcatatttttgtcattcaaacgaaaaatgaggcccacagttcccaaaagcttgtgcagcttttttatgccttttctaaggaaatggtgtgcgtcgttcccacctccctcacccccacggatgaagagctatgcatcaagctatggtcttctctttctggtatttcaggcgtgataggtaaaatcttggcaaacacttgttccgtagctcatttggtttctggaaagctttcatcgcagaatattgatcagttaaaaactccctccaaccgaccattccccaaaaaagtaaaacgtatgcttataagcattagcaaaggaaataaggagttagaaataaaattgctctcgggggttcccaatatcgggaaaaaattagctgccgaaattttaaaagatcatgcgcttcttttttttctaaatcagcccgtagaatgcttggcaaatatacaaatcgttcaaaaaacccgtacgattaagttgggaatgaagcgagccgaagcgattcattattttttaaactggtgtggctctgcccatgtaaccgatgatagccaaaatatcacagaggcgtcgcggcctacaatgcaggtcgcgacgcagtccgccgcaactcagcccgctgcaacgcagccattgcacgaagtatcagatgatgcatcatcagatgcttcatcacccgtagggcatcaaacattatctaaagaaatgttattgaacacagccagaggaagaaagagaagatcagttgagacacaaatggacaaacttggttttctgctaaatcacataggtaaacaggttaccactaaggtgcttagcaatgcccatataactcaaacgatgaaggagattattttggaaaatcatagtgtagatggtggagccgcaaaaaatgtttcaaaagggaagtcttccccaaaagaaaaaaaacattggactgagttcgaatcctgggaacagctcagcaagtctaaaagaagttttaaggaatactgggcggagcgtaatgagattgtgaatactctgttgcttaactgggacaatgttcggggtgccatcaaaaaatttttggacgatgaccgtgaatggtgcggccgcattaatatgataaacggtgtacccgagatagtggaaatcattccaagcccctatagggcaggagagaacatttattttggcagcgaggctatgatgcctgctgatatttatagcagggtggccaacaagcctgctatgtttgtgtttcacacgcatcctaatttgggttcatgttgtggaggaatgccttccatatgtgacatttctacaacgctgcgttatctactcatggggtggactgctgggcatctaatcatttcttcgaatcaagtaggaatgctcacggttgataagagaattattgttgatttgtgggccaatgagaatccgcgctggcttatggcgcaaaaaatattagatatttttatgatgctcacttcgcgtagaagcctggtaaatccctggaccctgagagacctaaaaaaaatattacaagactatggtattgagtatatcatttttccttcgaatgacttttttatttatgaagacgaacgtcttttaatgttttcaaaaaaatggaccaacttttttacgttacatgagttattggatgacctcgaaactattgagacaaaggcatcgtccacaacaagaggaagaaagagaagatcatcgacaaaaaaaaagcccacaattaccaagcaagagctttactccttagtagcggcagatacccagttaaataaagcattgattgaaagaatctttacaagtcagcaaaaaataatacaaaatgctttaaagcacaatcaagaagttattataccacccggaatcaagttcaccgtcgttacggtgaaagctaaacctgctcgccagggccataatcccgccacaggagagcctattcaaattaaagctaaacctgaacataaagccgtaaagatacgagcattgaaacctgtccatgatatgttaaacagaggaagaaagagaagatcagttgagccacgcgaacagttttttcaagatctgctttcagcagtggatcaacaaatggacactgtaaaaaatgacataaaagacattatgaaagaaaaaacgtcttttatggtatcattcgaaaactttatagaacgttacgataccatggaaaaaaatattcaagaccttcagaataagtacgaagaaatggcggccaaccttatgaccgtcatgacggatacaaaaattcagcttggagccattatcgcccaacttgagattctaatgataaatggcactccacttccggcaaaaaagacaacaattaaggaggctatgcccttaccttcatcaaacacgaataatgaacaaacgagtcctcccgcctcaggcaaaacaagtgaaacacctaaaaaaaatcccacgaatgcgatgttcttcacgcgtagcgaatgggcatcctcgaatacttttcgagaaaagtttttaacaccagaaattcaagccatattggatgagcagtttgcaaacaagaccgggatcgaaagattgcatgccgagggtctttacatgtggagaacccaattctctgacgaacagaagaaaatggtcaaagagatgatgaagaagtaa